European Patent Application EP 4 434 551 A1, published September 25, 2024. Title: Method for diagnosing and treating NIS-expressing carcinomas and metastases. Applicant: Andreas Nuske. Application EP. The sequence listing filed with the application follows.

SEQUENCE LISTING (3 sequences)

SEQ ID NO: 1 - DNA, 153507 bp, Homo sapiens
  source 1..153507: mol_type = genomic DNA
agaagatcaagcaattttaagttagaagaaaaggctgtaaatctggctttggtccttaagaccttgtaagagatgagcaagttattttgtgaagggcaacatcggaggaggcagaataaacagaggaggagaaaaggaccttaatgaaattcaaagtaaaattgggaggttgtgggtaaaatttcataactagacataaaaatcacaagtgggaacatgtcagagtcattcaaaaagtagatacatttgtggaagtgtgtgtgtgtgcatatgtgtatgtttaacctgcctggcatgttcaactggttatgatttttgaaattttaaattaagatcttctaaacctcctgggaatttataaggcttagagattgataaatggtgtctcagataaagagaaggagcaaatgtcagcgctatgatgatacacagctgctataaatgagtggcttgattgcttgacttcaaatacagcacactaactttcctaaactcagtctgcaaaatggtttacatgtcactattctcaatgcccagttttgccgaacactcggatgataatgaaaaagttttgctacaattttaaatttttcctttaagaagtagcataacactactataaaatatctgaggtctgtccagtgagaccagtttaaatatagctggagtaaaatggaaaacaattcagttatggtaaacttctatttctagacttgcactctcttcttaatataataaacatagtatgtaattataaacctgggaacaaagtcctctttattgaaagaaaagcaaatatgtatgcaaatctcaaatgagataatcaactaagcattaattgcaaaaaaaaaaaaaaaaaaagaagtcccatgggaccatgggaccatgggaccaaacaccaatatttggaaggagtccttgtggtttggaaaaattgaaacgggcatagtctttcgtctctaggaaccccatatggatggcactgcctatgtgcaaagttgcagggtggggaccatgtgctgtttatcattttattccccgcacttagcagagggcctggcacaaaataagcactcaataaaatgtttgtggaaagaaagaattctacagctatagtttatacagtgtttttccaactttaaaagatatggcccacagtaaaaaccacattttataccaactcctggtacactcagatacacacacacatgcattacacaaaagttacgaagcagcactttctttaatacagtaggcatgttctgattatttctgtcctttttgcttgactaaaaaatactgattatgactgaataaattgatttcataacctactaaatcaagccttgcaatttgaaaaacagacatattatttcagtttacattacttaacctcttacatttatacacttcactacccataagtctccttaaaaaaaaaaatcacaaaatttttgatccagagggaatttagaaaatattcagctcaactctaaagttttgcaccacttacgaattcactgttgtggggttccccttagtcactgttgttgaattatgggaattttccgaccaaaaaaacagattggcccccatctcacatcatatacaaaatttaactcaacatgaatttaaaacctaaaggtaagaactaaacctataaaactcttaaaataaacattaggagcaaatttcatgactttgggttagtcactgacacgacaccaaaagaaaaaacaggtaaactggacttcatcaaaattaaaaactcaaatgacaacatcaagaaagtaaaaagaaccaagcatggtggcatctgcctgtaattccagctattcagaaggctgaggcaggaggatcacttgagccctaaagttcaagaccagcctaggcaacatagcaagacctcgtctttaaataaataaataaataataaataaataaataaataaataattattttaaaatgtaaaaagacaacttacagcctggaataatatattggcaaatcatgtatctgataagagactcggatatagactatataaataaataactctcacaactcaacaatagaaagaaaaataatccaatttaaaaacagggaaaggatttaagcagactttcttcaaaaaagataaatggccaatgaacacatgaaaagatgctcaacgggatagtcaccaaggcaatgcaaatcaaaaccatgagacaccggctcgggcaacatagtgagatcccatctctacaaaagaatacaaaaattagctggtgtggtggcatgcacctgttgtcccagccacttgggaggctgaggtgggaggattgctttagcccaggaattcgaggctgcagtgaactatgattgcaccactgcactccagcctgggtgagagagcaataccttgtctcaaaacaaacaaacaaacaaaaccccatgagatatcacttcataccctttaggttggctaaaataaaaaagactataacaagtgttgacaaggatgtggaaaaactggaaccctgacacattgctggtgggattgtaaaatggtgtgcccactttggaaaacagactggcagttcctcaaaaacaccgagttaccttatgatcctgcagttctgtccctaggtatatactcaagagaaataaaaatatatgtccacaagtaaccttgtacatgaatgctcacagcagcattattcataatagcccataaaagtagaaacaacctaaatattcatcaattcatgggatgaataaacaaaatgtggtatatgtgtataatggaatattgaccataaaaaggaatgaaatattaatataagctataacatggatgagcctcacaaatactatgctaagtgaaagaagaaagtcacaaaggacttcatattctatgattctatttatatgaattgtccagaataggtaaatctatagagaaagaatatctctatctagagttggtggaatgactgttaatggagagggggttcctttttggagtgatgaaaatgttctaagggtagatttggtgatgatggcacaactctgtcaataaactaaaactcattgaactgtacattttatttatttatttttgagatggagtcttgctctggggctgaagtgcagtggcgcaatctcggcttgtaacctctgcctcccagggtcaagcgattctactgcctcagccccccgagtagctgagattacaggcacgtgccaccacgcccagctaatttttgtatttcttagtagagatggagtttcaccatgttggccaggctggtcttgaactcccggcctcaagtgatccacctgcctcggcctcccaaagtgctgggattacaggcgtgagctgccatacccggcctgaattgtacattttacttctatggtatttacattttagattatattaattattcctcaataaagctgtgattttaaaaagcaggctaggcgcagtggctggtgcctataatcccagcactttggaaagctgaggcaggaggatcacttgagcccaggagtttcagactagtctaggcaacatgtcaagacacagtctctactaaacaattaaaattaaaaaaaaaaattagccaggcatggtggtgtgcacctgtagtcccagctacttgggagcctggggtgggaggattccttgagcccgggaagtcgaggctgaagtgagccgtgattgcgccacagcactccagcctgggcgacacagcaacaccctgtctcatggaagaaagaaagaaaagaaaggaagaaagaaaaaaaaaaagcagattggaactctggaattaacaagaagtaggacgcacggagcacttccgcctgagtggagactgtggatccgggtcaacctgactacctaaatcacaggccaataaatggtctttcagtggtcagtccctgtaagatccgtggctctcagcttcttatcttaggggctgtggaggaaggacatgattatgttgatttaagcgctgaatattttcccttgtgatacccatcctcgcaaaactttgcttcaaccacaaacgaggaccttctgtaccagaggggcaataaccacaatgaagctaggaagaaatgcagagcaccccagcatacagtccataagcttcctgaagtggggggcctcaggcatcgctgcctccccaaagaggatcaggcccagaacagtatgctccagaaataagactggaaaaagggaaagaggggcctcaagtccaggagaccagcggctttctgaacgcgcacctgccaacccactttggacaggtcacgatggacagcgtggcaggaaaagaaaaggtcactgtctacccaacacatgagaaactgtttctcgtgcctcacgtccccactccgtccccacccatgttgtctgagtccctcggtgtcagaaacactgctaagaaatttaagaaattctgttaatgagtttaagaaatgtttttaatgattaaaagtcagtgacttgtgaataaccatgtaacttacaaacgcaaggaactctgaaagtgtgcagcaccaccgatcagaagagaaaaccaagggacccgaaatatgctttaattaaattttcttttaaaatgtcactggaaagaacatcttgggaagacggcctggccgatcgccgtgtgaagggcaagccactctggccgagagggagccccacacctcggtctccccagaccggccctggccgggggcatccccctaaacttcggatccctcctcggaaatgggaccctctctgggccgcctcccagcggtggtggcgaggagcaaacgacaccaggtagcctgccgcggggcagagagtggacgcgggaaagccggtggctcccgccgtgggccctactgtgcgcgggcggcggccgagcccgggccgctccctcccagtcgcgcgccgccgcccccgcccccgcccccgcccccgcccccacccccacccccacccccacccccagccggcgcccgcgcccgcccccgcgccgggcccggctcggcccgacccggctccgccgcgggcaggcggggcccagcgcactcggagcccgagcccgagccgcagccgccgcctggggcgcttgggtcggcctcgaggacaccggagaggggcgccacgccgccgtggccgcaggtcagagtacgggtgcccgcggcgctcgggaaccggctgctggctgggcggggagtgctcagggagggggcgcggagggctggggccgagggtctgggggctagggccgaggaaacgggaactgacggggtcccagacggatgagagctggggagaagggggtctcggctgaggggtccggggctgaggcagggtcatggtccggcaggacccggactgacgggtcgcgggcgggcggctcacgggtgaccgggtgaaggggtcttgggctgagggcacccgggctgagggtcgcgtctaccggagcgcgcactaggggcggagggcgcgggcacagagagccgcggccggtgccgactcgagtggacgcgagccggtgcgtcccggcttccaggacagcccccctcgggagagcgccgggtgggcgcggagccggggacacggggacctccgcgtccccggcggaggtgcgcaagcgtcgggagccgctccgggggaactttggagcagggtgtctggacccggggaagcgaagatccgcgtgcgtccgtcctgaggccgcgcggcacccctgctgaggaggaggtcccgttcgctgtccagagcccaggggcgaccgccgcttggggaccgggggaccgttcagcgaggggcgcgcttgtagctggccaggccctgtgccctgacgcgttgtgctggccctacgcccggcggaggggctggggacggggactgggtgcctccgtgcctccgcggatggagcgcgcagccaggacccccagccgcaccccggggggctggaaaggcgaagtcgctgctttgtgggctcctgcaagtgccaggcgctgaccactcctcctgggagcctaactgaggggggtagaggcagcagaggttaacagaaatctcaggtcccttggtggaaggtgggtgtgtagtcgtggtactttacgcctcggtgtttagggaggagcctaaggtaaggagtcagaaacggggagtaaccgagctgcggcttttatataaggtcagtggtaggtaaggaaggggccttaacctctgctggtgaccagaagcctgcatttctgcattctgcttaattccctttccttaggtgagttggctcactctcattgcattttgttggaatgtgttggtgataggtccgaaatttgcaaaattattgtattatccttatatcatttttttttgcagtgctcttgttttataagaagaatccaattcacttgggtcataggctaacggttgtaaaaatagtgtcattgttataaaagaaatcaagtcaaaaatagtcgtctgccatgaagaaactaaaatttttcttcttttccttgcaagattagggacaaaatgtaaagtttatttgtgtaaattatcatttggatataaaaccagacaatgataaactgagttgtataatacctattcctggaaaacctctgattttgaagtacattattttaaccccaactgtttctgtcattcgtgagacaaattgttaactggatttattaagagaacaatgaataacttaactctttaaaaggacctgggcaaatcttcgacaggtttcaggtattttatggcagtctttctgtctattgctaagtgatcgattgctgactgagaacagaaccaactgatggtgctagatgatttagaaaacctttctggtatagggactggcatggacattcactgtggcttttctcttaaagaaatacctttcactcctaggggagtttgacagaagacactcatagatgctaccagttagcatttggagtaatatatcaaaacattctgttcaagttttaaagtaagttttgtgtagtatattttcaatcagattcactttggaatcaaatacactttatttgattccaaataaagtgtatttgaatattcactttaatatacgaaactttaaaggtaatgtctcagccaaaaagtgaagtgtattacaaaactgtccatttttgtcttcttgtgtacttcacataatttttctccctgatttaaattatatgatatttgatagttaacttgctaataattatgtcttaagagatctttgaatcaactggtggccatctcagtcttttaaaactcacttgaaggaaaagagaaacactaatgatggttttttttaaaatcaaaaacttttttcatatttacaagtttgtttctagttcttaaacaataactgctgtaaaaccatggcatcagtgaggtataaagttttgtagaatcccaggctgaagactttttggatgtcgttttctcatttctttacattaaaaagaatataatttctttttaaaattaaaactaaaatgtccaccggcctcatattctttattgaacttaagtgctttgaaaatatttttgcgattgatatttttaatgataaaatataatattttctttgaaggactagtttcctaaatgttcatttttttgtatgtttcagaactacttttaaaaaaattctagattatgctttaaattgcaatatttctaaattcctatgacatttaaaatgtgtacaagagaaaaggtgtgacatgaggaatatgaattagaagtggattactaatggtcgtagtgaattgtttttaatcagtgttatataaatataaacaaatacttttttcttctgtaattttctgacaataaggatgttagccactaaccttaattatcaagataattatgtgcatgaaagctgtgtaaaaggcacaaccgtggaacatatacaagtattaataatacatttcatttagttttcaggttataaaatcgttattaataacaagaggctttcatgaagtaggaaaatatgttaaaatgacattttctgaatgtttcacacattctggcccacactttcacttctttcctagcatctatatattcccaatgcataggacagagttggtcattctaattgtgggtgtctttctgctggattcgttgtcacttggacttggaaatacagtatgtcattaggtgtggcaaatgtactggaagaagtttttggtctcataggattccactaaataaatattagctgtagaggatttttaaaaactcactaatagagaaaacttggtgaagtcactagtgtgtaagcgtaaacatatgcaccccccacaactgaatttctaatttgcttatttttcctggtagatctccactttgcttactctctcttaatatcccaaagcaacaaaaagcgcagtgattttaattgcttacaaaggtcctttgaaacggatctaatttgactccacaaaagaatagtaagagttgtgaacaaccatcttgcaagtgtagatatccccagcgtatcaacttcagttagtttcatagcgttctaaatcaaaaatttagatttaagattatttgaaatcttcttggaagttcttacttactgtttgcgttttctcaaaatacagaggtagattgggggagtaatatagtatatgttttaaagctgttatttaactaaaatgtcatgttttaaattttatttaatgcacttaaagtaggttcttgggataaaatctattcagatgcaataggccatgttttggggaaaacttttgtagatgtttagataatatctgtcatcaataatagtatatgtttaaattattttgtaaaaacagatttacatatttttaaaatttctcttcaacaataagtacacatcaatattttaatgccgagaatttcattcagagtatgactgtttacattttcaactgtttcaattattatggcttaggcaagtaccttatcctttctctcaattttgtcatctttgaaacggagaaagtgttgcagttattattgcttgctcttttgctatgattttaaggctttatgagcaaacccatgtactttaaatgatgtgaccatgaccctgaatttaattgagctgatattctgaaaagaaccttcatgaatatctatgtcatagctaactcttttaccaatgttaatagttcactgtagttcaaacctcaataactttgagattgttaagattgaagatgatgcttctcatgtggtgatcaatttataaactgtttctgggaatattttattatcattcaatttaaaattgtattttccattccctgatgactttggacaaaaatcagcatagtaattatttttattccagctttgcgagtcctgtgtagcccctcttatgttaatattatacatccgatgcatctagaaggcacagattgtgcgctttgatttgataaagctctagtctttgcatatctttatggcacaccttgtgaattcttaacgtatattccccaggagcaagttcgttttataatgaggcctaggatccatcagatcagaagacagtttagtgtcacaacttaaaagactaaatagtgacttgtgcttgtcattaaaaatgggtctctttcaacaagcactcaccaaaaaatagtgttttagtggcttgaaaggttcagatatctcctaataacccacctatttgctagtagggagtaagtggaaaaacatataattaactgtgcaccatccaaataataaattttaaattcttcgcgtgaattgttgatacatattgttgtgaagtgtctcctgcttaagaaagtaagggacttggactgaatatgccaaagaggaggcctctgcaagcggtgtcttggtgatgggaagttactggtaacagcacacggggtgatggggtgaagaggcttgtgtgcgtgggccccgggggctgaggattgttggagaggacttctcccaccttctctgggccccaaactgcacactggactggcaagccactctgcccactgcagtgtggagctataaagcccaagtagggacttcactaaaaggatgcagaggcgaaggcaaagaaaggctcatgctggtgcgtgtaggtgggctgagtgtccctgtccgggagtggggagccgtgttatcttccactgccttaatcctacagcgtaggctttctcagagtcattgccataccttcaactgttccagtggccaggctgttctcaacttgaaaatcttttgtgggacagtgccatgaattttttttcctactgcgattttttagatataaaggaattgaatccattaagtggagattttaaaccctccagtcaggatttaaactagattgtgtaagttcagttcagttggattcaatatctgtttaggaagcatttttattccacttcattgattttagaaaataaattcattgcttggttttaactatgtcactattaaaaaaaaaccactttaatttgtggactcatctgggaggattatgtgtggatatgacatattgagtcagattatctgaccttctgagaagagttcagattagcaaaaacgtggggtgagaagtccttcgcagtttgccacaggtaaggagaaggtagatatgagggaggtagagaaatagggaaataccctgagtaggaatgtaccaggtctgtatatgctcaactcccacagtcagcaggttgcatgattactgtgtatagtcttaaaatataaggttgatttctaagaatttaccctgcttcttggtgacattgtaggacatctcagtttgccacttagcactgttattctttctggctctatactaaaggagataatttgggcaagggaatggaaagaggttactttttcatcctgtatgtttaaggaataaattttccttcatatcgagggcagtggagaaatataactgtcaaactgttcgagtgcaatgatgaagttccggaaggaacttcctaaccttgaccacacccctctggctgtcatacacctcttaaaatgtctttgaatttgaatgtctttgaattgaaatttaaaatgtctttgaatttgaaagctttgggtctacttttaaaatgccaaagttcctggcagggttagttcactaaaccactatcagcaaaaatgtgaaaggctagttgcttgtttccttgctacctgaaaacaaggcctttaaggagtagaaaacagatttggagtttgaaagagggggttaggagagggaaaaataaagttaatgcatgtcccagtttcctcataagccagaaactttgaaacaaaataggaaaataaccatttggaatagcagtgataggaaaagatatatttacccatcattttttttctcttagtcaagacaagtcgcagatcttccttgaaccatttttgacctcaaaacagttattctgaaacatcaattaaactaagaaatgtaatcacagttcaagttatgagctagtattatcttaatgtaattaaatatctgaatattatcacttcattatatcttgtatttcctctgtgatgttagacaaattatgtggtctcttcatgagtcaactcttccaggctttaaaagtagcttcctaatagattgaaatgagaggaacttttcaatcacttcagaaaatgatgtgccaaggtagtataaataatgcttaatcctttggcagatccacagatcataaaatatcatacatgcggccagtcgcagtggctcacgcctgtaatcccagcactttgggagacagaggcagaaggatcacctgaggtcaggagtttgagaccaacctaaccaacatggagaaaccccacctctactaaaaatacaaattagctcggcatggtggcacgtgcctttaatcccagctactcaggtggctgaggcaggagaatcggttgaacccgggaggcagaggttgcagtgagccgagatcacgctattgcactccagcctgggcaacaagagtgaaactctgtctcgaaataataataattattattatacatacttaattttatttttgctgaaaatagtatggcaagccagtgcatctctgttagaaatagaaacttagtagccacctcaaaagcaaggtcataattctgtgaatcagctaataggtggtatttagcagttaggtatgggctaccctcgtgcctcatgactaatcacattgcttactcgtcatgcattttttacaaagtcttgctaaagtctgtgaatctaaaacagagaatctcaaagtgttccttactgaatgttatcctttccgtcagttgataattacctgtgtaaacaagcttttgactgcatctagaaaagcacctatataaattcttctgttttatatggtggataaagtttataaaggagaacaaacataagaatgatgtcaatataaatgaagtagaaacttcaaaaatcatttgcatatgtcaagtataatccagaagagtgaagaaaatacccaggcatttggcaatataggattactacatgttttcctaaagaatttggaactgattagaaacatcctgattttatttaaaagcaatataatgtatttttacagtttgttttcaagaaggttcaaaaaaaaattttttttttttttttgagatggagtttcgctcttgttgcccaggttggagtgcaatggcgccatcttggctcactgcaacctccgcctcccaggttcaagtgattctcctgcctcagcctcccgagtagctgggattacaggcgcccaccaccacacctggctaattttttgcatttttattagagacggggtttcaccatgttggccagtctggtctcgaactcctgacctcaggagatccacctgcctcggcctcccaaagtgctgggattataggtgtgagccaccgtgcctggcaaagaaggctcaaatttggtgacttttaggactagagcagtttgatgtctgcaaaaatctagacaccaatttcttgaaggcaggtactgactgaattctattccagcatatagcacaattcttagtaggcacttaaatgttttagaaagaagaaagagctggtcatggtggcacacacctgtaatcccagcactttgggcagctgaggtaggcagatcacttgaggccaggagtttgagaccagcctggccaacgtggcagaaccccgtctctacaataaatacaaaaattaactgggcgtggtggcacacacctgtaatcccagctactcgggtgactgagacaggagaatcacttgaacccggtaggtggaggttgcagtgagccgagaagattgtgccactgcactctagcctgggcaacagagcaacactttgtctcaaaaaaaaaaaaaaaaaaaaaaaaagaataaagaattagtctaaggcagtggttcttaaaatgtggtcctgggatcgtgagcatcctctggcagcttgttagaaatgcagtttcttggacctcatcccagacctgtggtgggcctagcaatctgtgttttagggactctgctttatacgctgtttgggaactcttggtccaagatgattcttgcaccccacctgatagagtggggcccatttgtcagtgtgctttggatgatttctagtaagccttacccttgcttatggttaagttctttgccctatctctctccactcataggatctcttggaaccatcctataaaactacccccattgacctatcatttattacttagaaaagctcagtagtggtgtcaataagcttttgtcaagaggctagccggctcactaattagaccttgcaacactggttctttttagcttagcatggctgcttaggaatccctagtctccgcgtcaaagactacaacttcaaagactggattttataaaatcacagaagatgatcggccctagaggactggttcatgttaaacagatttacaagatatggatttgtaaacctcaattccagtttaataatagtagaaaatattcccttcctagtgattgttgataatagttttttttattttaaaattctataatttcaaggattgaagagatttacactcatatatatctgatgtcactaagatttagttcaggttacttagaaagcattgggcaatgttttgtaacttttgggactttttccaaagggctggagaatataggaaaagccgtatacacgaagagtttcataaaagcattgttataagaacccatatttggaagtaacttaaatatccaacagtagggagatgtttaaataaattatggtataatcaatagttaaaatattgtacagttataatgacaatttagaaactactcacaactctgaagaatatttaaaaagtaggataaaaaatgtgtgtgaactattgattggaaccttacaaaaatgtatgtatatgaaaaagtctggaagagaatatacaaaagtgataatagttatgttacagtagtgagatatggagggctttttgtttgtttttatatttttctctctttcccaaagtttattcagtagtataaaattacttctataatcaaaagcatacatttatagcttttttttctttttggtgtgtctgtgcttctgatagtaaagatcaaggcaatatatgatttttttcctattatacccaaaatttattttatactaaattttatttcacatattggacttccctgtacattttacttgcctagtctctatttggcatggggaaagaaacccatctctgttatggcctcttaatgttctcagccatacgtaaggtttaattttgttgatttgtttgggtccgtgatctacttgatctttagcatatgctggcaaatagagcttttaaaaaatagtttccagagttactttcttttaaagcccttctctctttatttttttctaatttttttctattatgttcctttttttctaaaattgaatgacctcatgatagagttacccagttttcctgctgctgacagaatgttgcacttataaatagcagctgatgcagatgcacagaaaggtaaatttctgttacaaatgttcattatgagcccttcatataatttgtgataataattttaaaaataaaaagaaatgggccgggcgcggtggctcacgcctgtaatcccagcactttgggaggccgaggcgggcggatcacgaggtcaggagatcgagaccatcccggctaaaacggtgaaaccccgtctctactaaaaatacaaaaaattagccgggcgtagtggcgggcgcctgtagtcccagctacttgggaggctgaggcaggagaatggcgtgaacccgggaggcagagcttgcagtgagccgagatcccgccactgcactccagcctgggcgacagagcgagactctgtctcaaaaaaaaaaaaaaaaaaaaaaaaaaaaagaaatgtaaaatagcaagcgagtagaggtttcccaaaatcagtgtgaacattgtgaaagttatatatatgtatagacacacacacacacacacacacagtaatagcctttgaatgaattcttttttcatcttttctgttgcattgtcctagaaatcccaaaggagaaagttaagtggttttgcctttgacagcggttacagattacatttttcttgtcactttctttgggacttcttttgtgaaacttgtggcatgtcctagaataatctttatcttaaagttttaaaaactttttagaaatttcatatcagtgttataaatatttattctgtatgcctccccagtttgggatgatttcatccttaatgataagccaagacaaacttcagctaacaatatttagtttatagatcttagaatgtgtttatgggtaaaagaacctcgatgtgatgataccttagagaatagatctactgagactgatgcgttttattttcatttttgtattttatttatttatttattgagacagggtctcactctgtcacccaggctggagtgcagtggtgccatcatggctcactgcagcctcaacttcttgggtttaagtgatcctcccacctcagcctcccaagtagctgggactacaggtgtgagccactacacccagctaatttttatattttttgtagaaacaggggttcgccgtattgccaggctggtcttgaactcgtaggcccaagcagtcctctggcctctgcctcccaaagtgctgggattataggtgtgagccacgcgcccagcctgaagctttttttaaatgaagatttattcaacaaatgtctattgagccacttatttgtgccacaagctgtttcagataaggaggataaagcaatgaacagacaaattccattcctccttgagtttacaattattgttatctagatttaacgagaacatttttcaatgggaatgacggtgactaagagggggtgaatgggcctgtgtcttgtaactagatggcattgctaggcaccgtggactcagggggctctctctgagattggtatagtgtatgggaaagaaaatctgtatccttgaatattttttcccagctctcttactatcctattatcttaggttatgttgcatgtattctatattgtatattatgcataatatatttataatttctgtctcagtaatgaagtgatttcagaggaggtaagaatgaatcctttgctaataagttattactttccttgaaaatccaaatgacaagaggattattcactttgcaaaaggattatttatttttataatgttttcacagtagatttaagtggttaactattcaagtgaatttaatttataaataaatcaattaatttaaaaaaattatttaaccctaagaaaatgtaaaacaaagttcatggagactgtcccattaacatcaaaaaaactttttttcttgggagataaagttggctactttctctttaaaaggccattacaaacttttacaagcttagaatataatatttgcgtaaaaggagacccagatcctattttaaacgaccaaattattttgatcaaattacttactatagctattttcaatgtctgtattcacaaactgtttactatttcagttctgttttcaagttgacagaaaatatcatattgaccacttagaaataaattctgaaccacatgaattttttgggaaaaaatgataaggaaaatcaattttgatggactttatataaagttaaatagaattaattctttcatatatacagggccgtgaaatgttacagtgtaactcaatacagatgtaaccaaaaccttcaaattttgcaaatttcaccagagttaatttgtttggttctacaaacatttaccaaatgaccactcattaaacctgcccacctatgaacatgaccttataaaatggtgagacatagcagtatctggcactgggcacacagattaccacagctcaataaaagctgagaaaatgactcagtgattgaacacagcgcattgccatggttgtgtctttaagccattcatgtaattcatgctgtgtattcgacttagcctgctgtatgatctttgatcctaaccaagcacaatacagccacagttaatttctttttatcgtgaacattaaatttttaaatgtcaggttgactttctttgtcctataacttgtgtatgaaatatttatcctggtcccagcttttttttttttcattctcaaaggaggtgaaaccagcttttgaattcagaaaatgcagactaatattaatatcagccaaagtaaaacataattagaaggcagatctactctgaaatggaatctgatatattccatgttctgtgttacacatatttgctgattatttgatgtcatgtctgataattttcatgggaaaattccatgtaccaagcaaaattgttagttcctagagggtaagaatgtgtatagtagttctcattctctttaccttgctgtgcactgtataccttccctaattcccagccaaactgggtgcactatatacactttttaatacttttcaacttgattttattttgaggacaagtgtgtgctttttcagtatcacttgtataggattctccacaatcttagggaatttcctaaactactctttaaaatattaattcctattttatgtattgtttttgtgatacataatgatatgaaactaatgccaggagaaatttccattttgttattctaaagcagacaaaatgggatatgaaagggaaaaatgttaattatagacttcaacattctatgttggacctcgtagttgttctggtcagaagaacaggttttttaatggcctaagggccagagcattgttttgcattcttgtttggagactttcaatggcaactgtaacaaactctgcttagtaccacagttggagaaaggtttacaataatgcccagtacaaaatgttattcagacttactactcatgcataaaataaaactggttctcttcttaaacttcgttacatattagataaaacactatcaagttttggcctcatttgttcataatatgtaatttaattcagttgctcagctagttcatatatgaatcacaagtattatcatcacaattatttaacagttaatctccttttatagggtagatatgtgttaataagcaacttcaaaataccaaagaaactgctttacatatacaagcaaagcaaatagatggaccttgtgacatctctggacaaccagtcttcttggtaggccttcatctgtgggtgtagaacgaaggtaggagtctgctcactaaagatcaatgcaaggaacttccatgctctccactgctgggcaacctgccattctcctcctgccaccacacctgttcagctactagggcaaagaagtgccctgctagacacaagcagatgcttctcttaccaagagaagataatataaggaaggataaagaactgaaacaggtttgaggctttctcttattcatcatctagacttcagttttcttgatttattattccttcatgtcttgccagacacaacagttgcacatgtgttcaagttggttctaggcacaaagggagataccagagcttctgtagctacgagattatcatctgcgtgagccaagaaggggtagtgttgaaacaggtaactaacaattcacagcagtatgtgattaagggctaaaataagtaaagggagagaacaaatgctacagaaattcagagaaggctaagatcagtgtggagtggagggtacagccaggtaaagccttgtagagaaagtgggaattgaactaaactttggaagctcagggattgacaggatagcctcacgaaaaatactaaaaacaatacagaagaagaaacaagaagggaattaaaggatgattccatttgtacaaaatatcccgagtaggtacatccatagagataggaagcagatgagttgccaggggctgaagagaaaggaaagggggagtgactgcttaatgggtacaggatttcctttggaggtgatgaacatgttttggaactacacagaagtgatgattgcacagctttaagaattactaaataccattggattgtacacacttcataaatacattttaaattgtgaattttacctcaaattaagaaaaaaaaagttcctggtttgaggtaaccaaaagagaaaataatttccagtataagaaaacaaagcctggaatagcaaataagcatagagttaagggaaggtttgcagagattaaccagtttgaagtggagagtgcgtggatgtgagtagtgagaaacatggttggaagtgtagattttaggccagatgataaaaggtctggaatgcaggagaaggagtgtgggttttatctcaggagcggggagattccatatcgtaagaagaggggtgagatgattgaatcagaagattaatttggcagtagcatgcagggaaagcagtcaggaggctgctgcaaaatccggacataccatgaggagggcctgtaagagtgaagtggaagggcagatgtggacgatgctctgaagcagagaatgatgctcaaagtgtggtccgtggcttgatgctgccccacaagtgttagttacagacctggcacacagtaagggtagatttgagggtaagtctttaaaactttaatattattatgatattcaagcgcatgattttgcatttcatagcaatatccacagtaggtgtaagagacaagaaaacttccttcatgccagagttagaagaccgctgccctaaaggatgaatgagtggagttgatgactgactcctgtagggcagtctttttttttttggagatggagtctcactctgtcacccaggctagagtgcagtggcacgatcttgactcactgaaacctccgcttcctgggttcaagcgattctcctgccttaccctcctgagtagctgggattacaggcatgcaccaccacacccggctagtttttaaaagtatttttagtagagatggggtttcgccatattagctaggctggtttcgaactcctgacctcaagtgatctgcccgcctcagcctcccaaagtgctgggattacaggtgtgagccactgtgcctggccaggcagtcatgttttatggctcctttacagtgttccaccccttgtgctagacactgggaccagagcagtaggcaagatggactggcactttcccttgtggagctcgctgtcacataaatagtccttctttgtcaaaggattgctaggaattaaagggaggtctggttcagctcagcataaggaaagcattctaataactacagctgtcccatagtgggaaaggatgatttgtgagaaagtgagtgcttcgtcattggacatattcatgcagagtctgaatcatctctcaagaagtcttgctttggtgggagaaatggagtgggtgacttatcaggtcttgtgtaactaaggtgccatgattccctattctctaatgtgaacttagtagaacatattttcttcataactggctgtattggaacaccagtacatatactaagtttctgtctgtttctattagcacttggaattacagttacctaaatttacatgtagattcaattttgaacttatctgtacagttagttccacaattctttttaaagcaagtactattctctaatgccttctcagacattcacttatttccaactttaatatttatagtaagttcctctttcacgtgatgtgtgtcacaagtcacgcaaatttctgcagaagtgagttacataaattgcagtcaagctgctgacctgtaaatcattcattcttgcccccgtgatgtcatattggggttgaataagaccaggcgtgactacccacttgaggatgtctttgggatgccattttaattgggtgaaataacttttattattcaacttatgtgaccagttactgcaaacgtcaaactgttacgtttaacagctagaatgatcataggttaattgcactttagaggatgtggaggacgtagactcctataggagtgatagccttactatattttgggggaaattctagaatgtttttaactcaaaggacattattttcatgaggatgattttaatgcttatggtatcaggtgaagaaaaatgttagctgcagaagaaaaaaatttgtttcacttcaagtctagtagaatattttgttaaaatagccaattttcattatgtattattaaaacaggttatacttttcattaagatgtatgtaaaaatttcacatgtgcctggtattacacagtatttacccaataaatatttattgaatattgttgaatgaatgtgaggtgagggcggagaaaatatttcaaatggaaaaatagtatgagcaaaggaaaacgtgaatacagaaagaagcaaagatagtttctttaaagtcgcatttatatgtaataacaatgggaaaactttttggctgagtaattttggtggctccttaatttcttaatatttaacaactaatgacgactctctctgatactgatatccaaagcaaatagctgaccttgaacatggaaaagttactgcctctgactaattggaatgtctgagcctttcttgtcttctatcttctttccttcctttcttcctctctttcctcctcttttcccctcaattgtagcactagctcttgttcttgttccctctacccttctcccctttttcgttcctggtgttccctatgttttcttctttccttcttttctgtctctgtttctctccctctgaatttctgcttcctttcctctctttcccaattgctactgtctctgcctttggttgtctctgagtgtaatatggaagtgaagtatatttttatctactaaacacatgatcaaatagggattttttattctgaatttaacattaacagaaatgttatgttgctctttatgagacgaaataaagttggatgtcacttataaatggattttgattgatttttttaaagtattgactcactaatcttcaaattggtagaaggaggtcagtagactttgactcataaatttttgtaagcgtaatggcttgttgaataactcctaattgtctttaacaaccttggtttctgtcctcttttttccaaatgcagatatagcagatgtcttcagcatctaattttttattacactttcatatgtgcagtcatacaagagctggagtatttgttttgttaattctgtatctttattgtctagaacactgctaacaaatagcagatgctcaacaaataattgttgcttaatatttcaaatctgtagtgtcattctacctcctaatcccaaatagccatcataactttttagactaacattactcattaaggtaacttagtatacaatgaatttataaatgtaaccatacaatttcatgcttagagaacgttttctctccattctctctacctttagaccattctgcagtttaaatcttgaaccaaaatgtcatttaaccatccttctgaacgataactccataattaactcaagcaccaaataagtcatctagctcttgatggtaataattaatatttgttgaatgcttattctatatcaggctctgttttaagcacattatatacattatctcattttattctttcagcagctatgtacaccagcagtcccccacctttttggcaccagggactggtttcatggaagacagtttttcaacagactggtggcaggtggaaatggtttcaggatgaaactgttccaccttagatcatcaggcattagttagattctcataagaagcatgcaacatagatccctcacatgcacagttcacaatagggtttgcactcctttgagaatctaaggctgctactgatctgacaggaggcggagctcaggcaataatgttcgctcgcccaccactcatctcctgccacgtggcccagttcctaacaggccatggactgctactgcttcacggccttggggtgggggactcctaatatacagtattaaagtcagatgaagaaacaggaacagagaggtaaaataacctgccaggtgataaaaactaggatttgaacccagacaatctgaacccagccaccctgtcatgcacaggagcctactttgcaagtatttggccttccagggaatgagatgtccacatcccatcaccaccgccaccactattccacatttaacaattagacctatacaggtgtaaccatattcacatgtaacagtggattaaatttaaacttttagttgtgttaattcactgcaaatcagcttatgtgtcttgtaagtagtaagcaacttgaaagtacctgttgttgcttatgacaagataaattagatcaccaaatctttatatttagtaacttcatcatcacttagaaatcaaccgctgggccgggcgcggtggctcacgcctgtaatcccccagcactttgggaggccgaggctggtggatcacgaggtcaggagatcgagaccatcctggctaacacggtgtaaccccatctctactaaaaatacaaaaaattagccgggcgtggtggtgggcgcctgtagtcccagccattagggaggctgaggcaggagaatggcgtgaacccgggaggcagagattgcagtgagccgagatcgcgccactgcactccagcctgggcgacagtgcaagactccgtctcaaaaaaaaaaaaaaaaaaaatcaaccgctgttaggaaattctttttttttttttgtctctcttaaattcctcttaatctaaataaagacattttattttgtctcaggatacagaggtcaattgaatatagcaaattttgtcagtgttgtaaaaaatctggagaggaatgtaaacggctcatcttgtgtctggcctctaattgaatcagtcagctatggtggggttaggggacagatccgtgtatttacttgcataggacaaaaattagtcatttgtgagtgttcacatacttccacctctcccaacccaccaaagagaattgtaatttgacagtacaataatcccttcccctactcttaaaaaagttgatcttacaaggtcagtcctatgtttttatgaaaaagaattagagaatgagtagaaaggaactagtcaagaaaagcagaagatttgggttgatagacataaagtgctgggaatgagaggaagagagagagatcgtgaaattcctgggctgggaataaagactgtgtgtaggtaggacagcctttggtgaaggagacactttggagagcatggtgtgtgaaaacacttaaaggaaaattaaagggaattaagaggaaattgaagggaaggagtatatgagaagggttgctttgtggttataagctgaattttctttaatgtattttgaaagaccccggtaaagaaaggaatttcttttaattttgcagagaatgaggagttgtccaattaggtgttgaattgttcttccttggaactctcaagagaggagttgtgtttagagatagatttgggagctgtaagcaagtagatgtgttatgagtcacagtgctgagggcaagaatataaagaagagatgaaggccaagaggaaacttagagaacacaaaatagaaaagctcagaaagcaggggtaccaggaaaagggactaaaatagtcatcataaggtaggataataggaggccgtgcacagtgactcacacctgtaatcccagcactttgggaggccaaggcgggttagagatcagcatggacaacataaggagatctcgcctctacaaaaaaatgaaaaattagccaggtgtgatggcgcacacatgtagtcccagctacttgggaggccgaggtgagagcatcacttgagcctgggtggttgaggctacagtgaaccatgatcacaccactgtactctaacctggatgacagagcaagaccctgtctcaaaaaaaaaaaaaaaaaaaaaaaaaaagggagaaactgatttcaaggagccaagaaaagagacagattcaatagtggaggatgggcaaaatatcaaatgctgcagaggcagagaccgtggtgtgctggagccacattgttaaattttcacaattttattgagccaatcgttatgcatgctattattaaaacttaaattgaatacagttaaacaaattatattaaaaataaaagtaataaatacacaaagcataccacttccttattactttacattgctgagatgattcatgcccatggtatctgagtagtggaaatacactgtaatatttgtgctgcttttaaatcagtcatggtgggagtatttacaccacaaaaattggcaaacactaccaatcagggcatttttctctgcaaagagagccagttaaatatttaccagcatgccactgagaaaatagaattgaagtcaagaaaagtctaatggatttagcaagaaggagatgacatatacttaagtttcagtagaaaggtaggtgacaaaaaccacagtaaagtgggttgaggagtgaaataataaaaaattaaaaacatgtgttcaagtaagtttgagaaccattgaattaaaccgagaagcagattgttattgttgatgatggttttgttttttaaattacaaggtttgcagagtacatactatgctaatgtactttattaatctccaaaaatgaagaccatatgcaaatttattttatggtagaaccttttctgttggaaaatcttagggaacaagttatctatagaatacattttgggaaatgctgctcttgtatttcacaattaagatgatactgattgtaaagtttgagattaatattcttgtttttaaagtttcatgctttttaaaagaaattttgtcaagaatggatgttgaattttactgagtactgtttttgtcgtttttgtagtaatcatacggttttttgacctagtgctgtgacacattttaatagattttcaaatattaaatcctctttgcctttctgagataaatgtaacttgattatggtggttcattattttaatagaggatttaatttgttaattaacattttatttattatttaaaatcaatattgataagtgggactgatatttttctctgttgtcaggttttaatatcagtgttatgacactccagaaaagttaattatgtcactatattttttcctactgagaaacagcttatgtagtaagaaaatcatctcttccttgaaagctttaaaaaatcaactataaaactaatagcttttggaggaagtaattctttgataagttttcaattatttccattgttaattatttttctgtatcttaagtcaacttcaccatttatttcatttcagacaagttagtctgagtaaactgcccttggcctgccttattatttacttaggttctggtaaaaatcccatcccagatgtaaaatcattgtgtgagtagagatgaacagcccctgtctaacgtgggctgtgtttaagtgtgaggcaattgtctgctgtcttcacagcccagttctctggcttctagggatgatgggtagggtgtttataatcgaatgaatataaactaatcttgagttaaatgaccagatggcagaggtgaaagaacggcaatccttggtgtctactccccccagaatggatcttgtctctgccctactgtgtttcacatctggggacgattccttctaagatacagtgcagttctgaatgggttcagaaggaagaggactggtagcaggagggggtctgggggaaaggttacctaaatctgcctgactctgacagtagtaagaaccagccaagtgttctgtttgatccgacacttggggctacacactaagaatagataccagtttctagaaatctttactttttgcccatctacttctgaagaaatacctatgtatttcaaaggaaaattggcacaagtatcaaggaaagctggtacaacttaatcttaacctggaatcaactcctttaatttttacatacagatttggttccgttttttagattaaaatttttacctttgttttcacgtatttgagccctttttttttttttttttttttttgagacagagtctcgctctgtcgcccaggctggagtgcagtggcgggatctcggctcactgcaagctccgcctcctgggttcacgccattctcctgcctcagcctcccaagtagctgggactacaggcgcccgccactacgcccggctaattttttgtatttttagtagagacggggtttcaccattttagccgggatggtctcgatctccagacctcgtgatccgcccgcctcggcctcccaaagtgctgggattacaggcgtgagccaccgtgcccggccgagccctttttaatagttgccttaaatgtaaaaaaaaaaaaaaaaaaaaaaaaaaaaaaaaacccaagtggtaatctgtcatagataaagtgtttctcatctctcatgtgttttgcctgttgtgtgtaatgagcggtttcgctgtgggtgctcctttcatttctggctaacacattagagtgtgtttatgtaaattgctgtgatactggtcagcagtcacagccagaaaacataaaacatgtgggcattacacactgacacattagctctttctaaagaagaacatgtcccattctgaaaagaaaattattgctttgtttttgatattgagtctgtattaaaattttttttttatttttgagacagggtctcactctgttgcccaggctggagtgcagtggtgtgatcatagctcactgcagccttgaactctgggactcaagagttcctcctgcctcagcctcttgagtagctgggactacaggcacatgccaccatgcccagctaatttttctgttttttgtagagacaggatttcgctgtggtgctcaggctggtctccaactcctgggctcaagcaatccgcctgcctcagccttccaaagtgaaaaggttttctctcatttttcaaatagaagtactaaacaatgccagagaaataaataaacaggcaaaatacgttggctatagtttatattatttcctgctacagttaacaaaatgggaaaacattttatcttcatggtctactacatttatgccatgtgttaagtaataaaatagcttttgtaaattataaattaaaaggtacagatttaaaagagaaaatactgtagagtttcatgtaggtaagactgtgtagaatgtcgggtctcgatgttggcgctattcaagccctgatgataaggcttttggcattagatgctgttttgtcttcatggaaaatacagctattctaggatccttgagcctttcataagagataaggttgtgaatcctaagaccctaggaccatttacttagatgatctgctctctggttcgtcctctgaaaagtctgcttcgtgaggggtgtgctgcatttgccttgcctaagtggtgtggcacacaactgtactgtcaccttaggcttaataaccatgtgtcatctagaatgaagttatattttactaaggatcgtttttgccatgtataacttctcaaacattaactttcagggttattaatccttttaaggtctagtttttcttaagtctgtgcagtaatagaggtatcgtcattcatgtgacataaaagatggaaaggggcttcattcatgttagtgatggaaataggaaagtaggtgaagtgattctaatagatgtttcttttatgaaataatttttaaaagattctccagccctgcatgatttatgatgaatcattttgtggtctgttagttacttctagagaatagaaagcattgtaggctcagggaaagcaaacattcagaatgaaatccaatagagaaggtaaatttatttgggcatgtacattttggcagcctaggctgtgtacatgtgtacacattctgaacatgtgtgtatattgaaaatcttgtctcttttttattgttaagatttgaaagaagccaacactaaaccacaaatatacaacaaggccattttctcaaacgagagtcagcctttaacggtaagtaaaatcagaatttatactgcatttgtattgaaaagtatcccttttaaagaatatgtaaattatacattgtattttattgtaaaatttcctagagagtgatttttgactattataatactttctgctatataattttccagtcagttggactatgcagtgtaacatatttgtctaacacaaaacaaaggtaagataggaaaatgacctagaagttgagaaataactcaaatccttaaaaatgaatctctaattaaagtcttttatattcatgttatttttctacttaagtaataattacattattttagattcttatgatacttttaattaaattgagataaaaattaagatttctttcatggttccctattggccatgcagtcataatctgtggtcacaaaggagaaagtagcttcgtataagccaaatgtgctccattctaggaggaagaattgctaagttatacccggcattaaaactacttccttcctggaactgactagatgggggtaggatttcagaggctccaggggctcccaaagtttcgggatatccaccatggataatttatccttccgaggcctaactatagggttccaagacagttcttagtccccaacttttttgggaaggaaaaggagacctgtcactttaaggttttatgtagttttaggactattgattttggtaaatcatgagctatcacagaatagctcattttcctgaaatctgcaaataaatgaaatccacaacattgaataaagaatcatcagatagatagatacagaaattaatatagagatgtgtatatatgtgggttattatacatatatatgtttgctaactctgtctgcttctagaggacctagaagcagtgactccccagtagcaaactagatcgtggtttccaaatacaggctgagcatcccaaatctgaaaatctgaacttcaaaatgctttcagattccaaactttttgggcatataggtgatgctcaaataaaatactcttggagcattttggattttggatttttggatttgggatgctcaacaagtaagtgttaagcaaatattccaaaatccaaaaaaattcaaaatccgagatatttctggtcccaaacattttggataagagatactcaatctataccatttttccttaaaggaaaccagagctctttggagaagtggttaattctaaggctggggcagggaaaatacaggctgagcctggaggatgttgtggtcagcctgaaagagctcccagtggccaaagctggaacaatttcatcaataaaataactacgtataatattgaattataatctgatttataaataaaatgtatacacatgagtccaaattgatatacataaatgactgaataagtaaataaatggggggagaagaactctttcttgtagaagactttaataaatgtaaaaggaatgagggaaatagaaaattgttgtcacaaagccacagcagtaattgctgcatgcaacttccactaatactaaaattagtgaggtgggccaggcatggtggctcacgcctgtaatcccagaactttgggatgctgaggtgggcggatcatttgaggtcaggagttcgagaccagactggccaacatggtgaaaccccatctctactaaaaatataaaaattagctgggtgtgatggcggatgcccataatcccagctacttgggaggctgaggcatgagaatcagttgaacccaagaggtggaggttgcagtgagctgagatcgcaccactgtactacagcctgagcaacagcaagactccctctcaaaaaattaattaattaattaattaattaattgagtgaaagtttaaggtgaaacagaatatttgcataacctcaaagtatctgcccccacttactcagtaattacaaaaggaaaaatagtaactttacagtggagaatcctgatggacaccaccttaaccacatgatcaaggtcaatatcaaggatagtaagacatagtgagctcatatgcccctgatagaatgtcctgaaaaggacagatcatgcctttcgaattcttcccaaacatccttaatctcatttgactatgagaaagctttaacctaaatacaaacacattcttcaaaatatctgaccctcgccgttcaacagtgtcagaggcataaaagacacatctttgctaaggaatcactacagattaggaggagaatattgcatgacaattaaatgcaatgtgggatcctggattggatcctagagctgaaaagggacgttagtaggaaaactggtgaaatccaaatagttatagtattgtgccattctcaatttattaggtctttttttgcttttattattatttttaattaacatataattgtacatatttatgtggtacagtgtgacatttcaatacgtgcatacaatgtgtaatgatcaaatcagggtaagtagcatatccatcacctcagacacttatcatttttttgtattgggagcattcaaaatctgctcttctagctattggaaaatatacgataggttgctgttaattatatttaccccacagtgctatagatcattagaactattccttgtatctaactgtagttttgtgtctggtaaccaatctcttgctatccccagcccttcccagcctctagtagcaactattctactgtccacttttatgagatcaactttttaaacttcgcatatgagtgagaacatgtggtatctgtctgcttatttcacttaacataatcaccaccaagctcatccatgttgtcatgaatgacaggatttcattctgttttatggctgaatggtattccatcgtgtatgtgagccacattttctttatccattcatctgttgctggaactcaggtggatgctgtatgttggcttcagtgtatcaacactgataattgtgctgggactgcactgtggtaactggggggaagctggctgaaaggtatgtaggaactccctccactatctttgcaacctttctgtaagcctcagattatttcaagttaagtagttttttaaggtcacaatggagtcactaaataatcattctcattagattttcgctaatttatagaggaagattctgcatttgcaaatcttagaacagagtaatgcaggggcattcttttcatcaagactatttcttgagctattttctaatccttctcatacacactcccatccctacctctacaagtctggtctctatttagtgtacttaatactttagccagttgcttacagccctctagaaacctgtgagtgggaataactccacaaagctctgcctcctcgggaaccacatcttagcagtgttttttgttggtgacagtgagggtctaatttgaatgttcacaccagaactgtcaaagtatttcatgcaatactttgaaaaaaatctcttgatccaccaatcatcattacccaagacaggatttgaacaagaatttagaactcgtagtcttatatttgtttgaatgggaagaggagagaagcagaccgtattgtttctaggcaaaatgtctgggaattcagtgaatacaagtagtactacgggaactttcattcttaaaggaaatcaatgacagcattaagttgtctagaaaatcagtttaactttagaaaagcataaagccgtttaaaatcaaaagagcaaactcttaaaagacaaagttaggagcaggtacgtactttggcgtctgaaaatgagcggtctaaattcaagcattttgacatgaaaaatgaaatgtgaagtatttggaattcaaccctgaatttttttgccggtaactcttgtgtatgttcaactaatttagcaaactgcactagttcacattttttaggtgaaacaagaaataacagaagttgcacctaaagtagtcaaatttcgtagagacagaaagtggaatggtgcttaccaggggctgcggcactggaaaggaacggggagttagtgtttaatggggacagtttcagttttgcaagatgaaagcatcctggagaatggttacacaacattgtgagtgtacttaatgccattgaatgcacacttaaaatggttaaaatggtaaattttatattgtgtatattttatacagttttaaaaactaaaaaaaaaaagtaacaagtcttcagcagttatattccacttcattgccagggtgtctggctctaaggggaatctctgcttagaggaccattaatccttaggaacctttttttttttaaaaaatctaaagatggttcctggacatcatttaccaactggcagtttaaatggcctgtgtaccataaattgtgaggttaaaaaaaatctggtacacaggaaacagtagagctgggtggctgggagagttgcttttggggttaatttataactaagacaaatgaatctatgaaaagaagaaaagccccgtaagaaatatgctaactgatggtgagggagaaaagggtttagataaaagatatctgaacttgtttggtctcagtgattttatgactgaggaattcaattatagatgtactggatggagcaaatcacaattctgtaaattactaataggacacaacgatctttatcattttctgtatgtgctcacatgcaaagttcagtcctgccctctgtaaataaactctctgcctagctatacccatgctatgaattcagggcttgagtgttgaaacataggcaatgcttactgccccaaccttaaaggcaggtggaactgagattaggaacgaagacaaattacttttgcttttgaattttggccttcgggtttgtttcatttttgttcatttcttttcatttttattactaaaaagctgattttttaaaataaaaagatcacaaccacacaaaaaaactattcttctgtagtttcttccagttttgttcacatgtgtatgctttttatttactgacagttaccgtatatacatcacttggccctcagcctctttcactgttaggtcctataaatttttcatttctacctggctttcagagttttcataatggcaacataatcttagtgatagcacgtaatttactaagccagtttttaggtggcttctggtgtttttattattgtataattatgttttattcttataccattacataccatgaatatctttatgtaaatatttcactcaattaaaaaaatattttcttcagataaattgccaagagaggaatttctttgttaaagtgtttgagcaattaattaccttactcttgcattattaattttatgacatttcaaattgcttggaggatatattaatagcaaatgaacaaaacatacaaagcataaatatattttggaaatacatttaaatgatttctgttaatttaaatgaattatcatttacttaaggctttgggtgtatgatagtggtgggaggctggagagtgaagcgcttcaatagttgtttagagattagaacgatgtgagtggtttatttttatttttattctttagaggcagggccttcctctgttgctcaggctggagtgcagtggtgcaatcatagctcactgcaacttcaaattcctggactcaagtgaccctcttgcctcagccaccggagtagctgggactacaggcacacaccaccgcacctggctaattgctaaattattttcagagatgaggccttgctatgttgctcagactggtctcaaacgtctggcctcaagcaatcctcctgccttggcctcccaaatggtgtttttttaaaaaacccagcttaatagcaaagaagttacagattatttcctgaggctatgtcaaatttaaataaaatgtaaagactgtgctgtgggtcccttaccacctttaagtctaagttgctagttattaggaagaaatgattgcttttgaaaatgcagatttaacaaagtaggactttcatagagataagttcaaatcagtttttaaaaaatattcatttaaaaccaaatatttttaaatttgtggtttgaatatttgagaaacaaatttaagaataaagatacaataagaattttaagatacaaaactatatgtttacaatatattaaaatgaataggaaaaagattatgggtgaaactctctcctttttattctcaactttctgtttgggggttcagtgtctccttccacagttttctttgcctcaaataaataaagccaattatgagctctacagtctgagttatagtattcttggttctttgggtaccgccaataacttatatatcacaaataatacatatacagtgttacatagtaagtgctcaataattggaagctagttccatggggcaaaaggaaagcaactgtgttctctttcatactgttctagttttttttttcctttaagcttgtgacttcttgttcttcagtccagatcctgtgatctgaaataatttaaattattaaaagttagatatttttaaccttttatactcccactagacaggacataggaaatttagtgacgtaagcatctttaataatccttaaaagtcataagacttggtggctgggacaagaaacaattaggtataaatttcagggaaataccataatggcatgacttttgttttcttttgttaacaagccacatggctttcctctcaagcccaaggaatacatagtgtgctctccttttaagatttcagttttgtctgcatcacagagatgtatgtttccctaagtttgctcactataatttgtgattgctatttttcttatctgcgaaggaagtacagcagctcccactggggaaataccatgttaagttgatcctaaaataagaaatctaagggaaaggtcacatcctaataacttgtgcaaatctaaattcccatggagctttgcaatcattttgtaggagtataaaaaatctattattgaacttcttccagatagcgtcgtaaaattgaagtacttttatatacagaagtaaccactaaattataaatacaattgacaagacctaattttttaagcaatctattatgaatacgtagagaaatctggcatgactaataaaccacaaaatctttcttgtcactttcactggaaatataaagtatattactcatgaagtattgtgataattacatacaatagtaatttcctattactatagagatatttaatactcaatttttactttttttttttttaactgatgctgaccttttagttatactttggaagaaccttaaccatgttgttccagggaaattcactgctttgggagccaggtcactgagttactactgtctttcctcttctgttctttggccatcgtttaagtttccttacctgttaagtaagaaaggtttatgttaaggatcaagtaagatcaaatatataaagggtttagaaataatttacggcgtatatttatggtattactgtaataattgccttgacttttttatcttttccaaatgaataaatcaaaatagaaagaggttgagtaacttactcgagctaacagtcaccggtacacgctaatcagtgccccactcactggtcaaatctaagtaattcttcaagggatggaatgtaaatggaaactgctcccttatgctgcatacagaggtattacattttgcagtaaggattgattgtttcctagcacgtagtaactaacctgttttgaggatgcgttgttagaaatgcatcttggacatttatgtatatatacgtgcatatatatatgtatgtatgtatgcatgtatgtatcgctagaggaatgtgcgtccttgctttcttactacaaattaaagctgaacagaatgtggtgtttgtcttttggtattgtctgaataaataccaatatctactagtatttatttccttgctggtaataatgtgttttcattaatttaagatttataggaacatacttgggtgctctgcctgctagaaactgatctgtagcatgagccatttgttgaaagtacttagatatttctgcatttatttatttctgtttcagaccccacaataactatattactataagaaatataggccagacacagtgggtgggtcacacctgtaatcccaggagtttgggaggccaggtgggtgggttacacctgtaatcccagcagtttgggaggcccaggtgggaggatggcttgaggccaagagttggagaccagcgtaagcaacatagtgagaccctgtctctgcaaaaattaaaataaaaaaattagccaagcatggtggcgcccgccagtaatcccaactactcaggtggctgaagcaggaggatcacttgagcagggaggtcaaggctgcagtgagccataattgcaccactgcactccagcctgagggacagagtgagaccctgtcaaagaaaaagaaaagagaagagaagactaaattgttttttacatgcttatctatgtgatgtgagttcaaagaatctctgcaatgattcaatatctttttaatatttttgtttgggaaaagcattaagctccttcattgtgttaattaattcagttttctcttttatgttatacaccagcatgaaaagtgtgagatgttagaggcccacatcagtaccctaccacatatttaccaggaaaagctgactttatgcttaatggcagcagtcacccctttaaaatgtgtggcctctgtgtccgatggcgtggactcacttcctttaagttcatggccttctgaagatcagctgggctgggatgagtggtggctggcatgtggtggagtgtcttgcttccctctgatacatggaagttataaaaagtctcactaatgaatgttcttaatatatatggggtaactaatttatgcatcagactttggaataaaagtaatagcaacagcaaatgagagtctaagaataattcatttttttgatacacttctgcccccaggtgccaaatgctacagggtggaggcggagggagacagaaaatctttctgtataggaacctactgatcgctgctactataaatttttctaaccattttatttccattgattattgttttagttcaggttttccttattcctcatttgggttattgcagattaactctctgaccaagcaatccatcgtttccatcatcctccagtccatagttatatttcatcccctttcagagagcattacagactctgtggtcggcccagcctacctcttcgatgtcatcacctccacctgctcccacaaatcttatgggtcagacacaccaggctgctcagtgtcctctcacagtgctgagtttatgactgggatggattgattttcatactattgttgattcaacattttttatagtatacttcttgagaacagagaccatgttcagggatccctagtgcttaatacaattcctaccaaatattatgcaagtaataaaattgcagtgtcattgaacattttcagatatgcatttatttctactaattaatcttagtagtattagcagccttgactaaatattatttctaaattgatcaacatgcgatgcaaagcatgctacagaattgaattaagaaaagaatttccatgagagatatgcatttacaattttgtagatttaatctttgcatagacttttttgttgcagatactgaaaaggaatccataaaaatacatagatccctttactagccacttttaatttacggatgaggaatattcagttcacagactggctagcgctttttagctttctttagcgtttgaagcagggcttctaagtcacatgaaagactagactagttattggcatttaaattttttggctcctacttgtatgtattatttattaaacaagtagttattgcactacctttatgtatgcagcactgttttagacaaaatagaattgtgacatattccttgctcatggtcttgtttcaaagacaatacctacaactgaaagaattaaataatagagccaggcaatatctgattgaggaaaagcatgcagtaaaagttcagagaagaagatacacgtgcagaactggaatggtcagtagttgcttcatgagatggttgcactgagctgaacccttaagtaaggatgtggatacatgagaaggaagaagctggaaattttaaacatgaggagcttcatggggaaagaatttcaagctatcaaaagatatcaaagattgaggaatttggacttggtctgggaggtattggggatcttgaagatttgggggtagggaagtgatatgacaaaagctgtgtttggaaggcacaagtgaaacagagttgggtttttttgtttgtttgtttgtttgtttttttcagacagggtctcactctgttgctcaggctggagtgcagtggtaccatcttggctcactgcaacctcaacctcccaggctggagtgatcctcccacctcagcctcccaattagctgggactataggcatacaacaccatgcctagctaatttttgtatttttttttaatagaggtggaatctcgctatgttggccagcctggtcttgaactcctgagctcaagccatcctcccacctcagcctcccaaagtgttgagattatgggcgtgagccactgtgcccagctaaaagagagattttgatagcttatatgatttgatgactgaataaaaaataaagaggatgaaaaaagtgaaaaatgaatttttggctgataaatagagaaatggaggtattaaaagaaattgggaagagagactctgtttcaggaggaagagggattagcttgatttttggatttgatgaagatgtgaagttaggtgaccagacctcgattcagattttagaatcagactctttgatttggtgtcattaacattgattgaagaatgttttgaaagctgaggtattaagaaacaacacaaaggtggagtttaaaagaggaagttgagcgtttggagagagtgccatgccaaaggaggggacttttaagaaaaggaagacaacacttagtacttctgtgtacccagccttgtaggaataactttacctgtgtaatcttattttattctcacagtaccatgtaaagtatgaattatcattgtccctatttgacaggtgaattaagtgaagtttattgtggttaaataacttgcctgaatgtcgtgctgctggtgcaaggttaatctggatttaaactgagatctgtctgtctaacccccaagcccacatatttttttaattgaaatgctgcaaaatggtaatgaaaggtcaagaagaataaaaaaaaaaagagtaaggccattagaatgttcaaggagaagatcattgtttaagattataaaagcgtagtggtaggaatatttcagcatttagaaggtaatagtaaattaatggaggaagtgaccctagaccattgctaatttgggcagcgagtaggacagttctcttctgaggcagctgagtcaagtacagcagagaagagtgctcatcagtggagaaggtgggaatagtgttggagaggtctcagaataaacattaagtaatcccagcactttgagaggctaaagcgtgtgaatcacctgaagtcaggagttcaagagcagcctggccaacatggtgaaatcccgtttccactaaaaatacaaaaattagccacgtgtgttggcactcacctgtaatccccgttacttgggaggctgaggcaggaaaatctcttgaacccaggaggtggaggttgtagtgaaccgagatcgtgccactgcactccaggctgggcaacagagcaagactctgtctcaaaagaaaaaaaaaagaatagacattaaaaagacacagacgatgtgagaaaaaagactgttcccaccaagtttagaagaaaggataatgaggttgatgtgcctgctgtgccggggggataagagaaaggtgtcaggcaagaatagatgtataaaagcactagttacaactatactttgaaagtcatattttacctggaagaaatctcaaaaaacaaagactacatggcagttaagtgacccaaatcaagtcactttccctcttcaggcctcagttttcccatatgttagacaggttaaattaggtgagacaaactgatcttttaggaccattctataatactgtgcttaactttctaagcattctggaatggagcagccttgatcttttcacagatacgtcaaccatatagctttatttataaaacgaacatgttgagataactaaaattagagttaatatcttcataggtacaaagaaacttttagaacttaagtccacaagtcagaatttctggatgaattcctttttcctcttattaaaaattgttaagatgtctgattagactagttgtaaattcccttgaaagcaaggatgatatcctgctctctactgtgtcctcagcatcaaggacagtgcctaacacagaacaactaccaatgaatatttatgaaatgaatgaaagtttgaattgcaaaattaaatgccaccaataaagaggctttgtgagcgagcgtggtggctcaagcctgtaattccagcactttgggaggctgaggcgggcggatcacttgagctcaggaggtcaagaccagcctggccaatatggtgagaccccgtctctactaaaaatacaaaacattgtctgggcgcagtggctcacacctgtaatcccaacactgggaggctgaggtgggcagatcgcctgaggtcaggagttcaagaccagcctggccaacatggtaaaaccccgtctctactaaagatacaaaaattagccaggtgtggtggcaggcacctataatcctagctacttgggaggctgaggcaggagaatcacttcaacccaagaggcggaggttgcagtgagccaagatcacgccgttgcactctagcctgggcgacaagagcgagactttgtctctaaataaataaataaataaaagtataaaaaacgagccagtgtcgtggtgtgcacctgtagtcccagatactcgggaggctgaggcaggagaatcgcttgaacccaggaggtggaggttgcagtgagccgagattgcaccactgcactccagcctgggggacagagcaagactctgtctcaaaaaaaaataaataaataaataaaggcttagtatagaactcttcccagtcttttttctccactttgattttttttttttttctcaatctcttccatgacaattcagggacacattaattgtgcaaaaggcagtcacttgtctgtattgtctatttttatatcacttaaattggtttttcatttggttgctatgttgacattttatgaaaagggaactaaacttgtgaattgactgacagtggaaatcataggattttcaaaaataagttttgtagttacttaaaaattagtattccagttttcggtcgttcattagtttaaatgttaccaataatattttctttataaaaagaaattatgttttatattgtagaggaaaaatgatttagaaaaacagaaatctatttctgaacaaatttagtgatgctgatgtaagaaaaagaaaaccacaagaagtcatcccaaatttagtaatgcttcctatcttaaacacatgatttcacttgtcttctggctagctaaaggttacaaaatgtcaccataataccttttacttccttatgagttcttgctactccaccccctacccccaaatatggtagatcgagttgtaaaaaccctgaagtatgacaatatagtttattgcacttatagttagaattattctgccaagatgagctgagaaatggaggaaatggatttaaatttacagcagtccagtgatacacaatatgcgttttccagaccactgaaacagcaagccaacttttaactttaatacttcatacagtggaaaagttacagctgtaataaaatcaacagatacatctctggttaatgttctcaaatgagaaaattgactgcaagaacatttgtccaaatacatgtttttatatattttatgctactttccagaatattaacagttttacatagcgctgttttggaagtcactcattgttttcatctttctgattaagaaatagggccaaagttgtacattgcactagtagtagacttttaaagatgtctttgtctctttttcagtactaagcttcaagttcatagattatccttgatctttcctttccctaggtagagatttagagtatttgtttatgtgagatatataaaaaaaaaaaggagattttaacaaatgactgtttgattcttgggtagaaactaatactgatcaagaccaaccaagtattcagacaagatcgggcgtgttcagggtggtacggccatagacgacaaccaagtattcaaacattgagtgttcagtggaggctgtacagatatcctgggttttgattcaagatagtgagatagccatcctatgagaatgtgaacttgaaataagattttgattacttttttttcctcctttaaaggtttgttcaattttaactattttttttcaaaatctgcattatcacagtatattttaaaagaatgactaatttactgtgatatatttgggagttaccttgaaagagattatcttgtaatttaaaataccagaggtagagtgaagagtcaggtggtaaaagagaaggagactggatgtttgtacccggtttgcttcttcccctttgttctgctgctggttttattttagctgttctgtttgcctcaccgcaggcagcgtcaccactccggttccaatcttctggacgtagagttttcaaaccatctataaattagcagtctaagtggaactttggcaaatgaggttgccaacaagcattttctttatatttagataatttgagctcatggcctctgggcatttggtaagaagtccagtaaagagaagcctaaagaacagaatctttattatgagtagtcgcctttttccactcagcagtttgattccaagcaccctgagaaaaactagagacatagtctagttggcaggttttttgaagagaatgagaagcccaaaccaaaagataatgaagaccacagcagagaactaccgaggcagctggcgcagatgcttttttggcactgttgagaaaggcttcagacccacagtctgaagagatggagaacccctcctccaggagcaaggaataagaatgacaattgttctgtaggacagttgacttagattcaggaaagttcttcagaaaatatattcagatcacaaaaaaggtgttaaaatcccaggatttttcagccaaggatggcacttgcttctttcagcatcactcatcaagttgaaatttatgagtgtcctttgttatcacaaacaaagcaagcaaactgaacaaatgagaatgcttctttagtatctacatagcactttaaaagctctgttttctttacaaaatgtgtgtatggaaaggtaaaatgggaataaatagtattaaattctgttcttagaacctactgtatagtgattgaacagctaaacagaacgaaaaagcatgcacatcttacagatacagagatcatgactttggtagatgagactaacatgtatgaaggtgtaggaagaatgtttatttttcagtccaaggaagcaattcacaatcaactgttagagaagcagcaaatagcgaagaaaaaattaaagaactagaacagaaaaagtcctacctggagcggagcgttaaggaagctgagaacaacatccgggagatgctgatggcacgaagggcccagtagggagcctctctgggaagctcttcctcctgcccctctcattcctggtgggggcagaggagtctctgcagggaaacagcttctcctctgccctgatggatgctttatttggatggcctggcaacgtcacattttctgcatcaccctgagccccatttgcttcccagccctggagtttttaccctggctttgcctgccacctctgcccaggacactcttccctcttggggtgtgtgatgaactcccaggagaggaaagatgggagccagggcaagataggaagctctgcctgagctttccactaggcacaccagccagaccaataaaaagcatctgtcccactctgctaagcctgcttttcttgagcagagggtgagagaggcagtggccatctccacctcagctcctgctccctctgcatcagagcccttcctttcttgggggatgggctcttgccctcttctcttttcccttcctgtatctttgactaacgcctcagctttcaggcctacatgtagcagacagaagaggaagaaagaacagacgttcacagctgaatctcagtgaacagaatagcagtccctggatggcagtctgcctaaagattcctttccctgccttctcccatacattccaaaaggaagttcaacagtcagcagcacctccaagactgtctccttttggccaatatcataagatggacgccgtaatcctgaggcctcctagaggctgagggggcaatggtgtgctccagctggctcatcccagcccaggtgggccaattattcaattttcaagaattttgttgcaagccagttgttaaacacagccattataattatgtaaatttgcaaattatgttaaaaacaaggacaataaatactcaaaatgcaaaaaaaaaaaaaaaaacctactgcatagtgtaatagtgctctcacttttctctccttgattctgatgtcaatcactcattgtcacctccactagagggggataaaaaggataataggaaatcagaatattttgatttgtagttcaactgttgatcaattatctttgagacttttaacattcatgactaaggaggattaataattaacatgagctgtagaattaaggtttgtatggcatgataagtataaaccagttttgggaccgctataattctaaaaaagcaggtagactagatgattagttgtacacttattactgctaattcttgattgtagaacaaattttcctatgaaaaccatgttgtgtattttatatctctattagttcgttaaaagtttagcagttttagatgtcgaaccagtaaaaaacaagttgcccattctatcatttttttttattgtggtaaaatatatttaagataaaatttacgattttaaccatcttaagtgtacattggtacagtggcattggttacgttcacaatgttgtacaactgtcatccctatctatttccaaagctttttcatcacccaaacagctctatacccactaaacaacaactccacatcacccactccccagccctggttatctctgttctactttctgtctctatgaattcggatattccagttgtttcatataagtggactcatataatatttgtcctttttgtatggcttatttcatttagcacagtgtcttcaaggtgcatccatgttgtagcatgtatcagaatgccattcctttttatggctgagtaatattcccttgcatggatatataccacattgtgtttctccattcatctactgatggatacttgggttgtttttgccttttgctattgcagataatgcttcagtaaacattggtgttcaagtatctgttttagtccccacttttagttcttttgggtatatacccaggagtgaaatgctgggtcacatggtaattctgttttgctttttaagcaactgccaaactgcttttcacagctgctataccattctgcattcccactgcaatatatatgggttctaatatctctacattgctacaacacctttttttaaaaaaaaaaaaaaaaaaaaagctgtcctattaggtgtcaagtgttatctcattgtggttttgatttgcattttcctaatggctgctgatgttaagcatcttttcatgtgcttattggtcatttgtatgggttctttggagaaatgtgtattcaagacttttgtccatttttaaattgggttgtttgccttttgcctttctattcttctctcacttttaaattgattttctcccatatttctccacaaagtcaaaaagatgatttcatttgaacacagataaatgctgtcagccttccattgccatatacattgaattaaggtcaaatgctttttgtgctgttgctaaaatcacttgagaatctgtctctcttcaactgaaagaattgttctggatgcgttgatgctgtggaattccttgtactctctcccaaatctcatttaacaagctcacatttagggtgtgattcactgtgaagtattccagaaaataaaatccattttctcagaatgatgagaaattttacaccttgaagagaccatctcttttccaaactgagatccacagattcttggagatccacaaatatattcttgggctctgagagttttagaattttaaaataatctgtttttatatcaataatctaaaaggtcattagaaagcccacatttcacaatacaaggacattttcctggaatgagactgttttcttacattagtaagatggaagtgacttgcctaagataacacagcaagttaaaaccaacactaaaactcatctttggaagcttttctcagtgttctttgttactagtgtggagatcttgcaatgattctgtcttcattaagtctacaggtagtggggaaagcagaaaaagaacaagtattaactaaaatgatgagtgctgtaagggagagaaatggcagtatgagttgtgtagaatgagagcagttgcataggatgagttaagttactgtgagagtttgaggaggtggtttttatgccgatagttgaagagtgaattggagttaccttaagggggttgtgagaagaaccatgttacagatggaggaaatgagatgtgaaggctgtgatgtgggaaacagcttagtttactccctgatttaaatggagaaaaggaatccagtgaggcttcagagagaagcaagaactaggttattcagggtttaagacaatcaaaagtcaaaatagagtttaaacaggggagtgacataacctgatttgcatcatgctggctgtagtatgcagaattgattggagaggcaaggatggcagacaggacgccaggtgggaagctatggaaaggtgcatatggaagaagagagtgtctttggattccagttggtaagtggaagagactgaagcatgtggctgaatgtaaatgtttaataagtagaattaaaaggacatggcgattggtttgatggggatgtctgggccttcaattatgactccctgtttttggcaatgatcagctgggagattggtggcagcatttactaagacagggctcattgaaggaggaccagttttagggaatagaggatgaatggagtttttaacctgttgagtttcagttgcctgtgagatatttcaatggagttaccaaatagatatttctatgtagtgtcaaggttcagactagaggactgaggcagagatataaatttggtcttaatatatccatagtgcttgaaactatatgtgtggagatagttatatactaatggttgtcaaattaagcattttttccaattcctttcccagaatctagtcatgtgaaatgatgaggaactggaatgtacagtgtatacattgttcttggcaaaactaaatttaaatttctgcttaacctaatcaaccaaaaagccctttttatttctgcctgtgtaaaatctttcttcaacatattaagccatttttctgtcttggtaaatatgatagggtgaaataaaatttaaattgaatttagatagccctgaattgatgattcaagaacttttagaatcttagttttatttttgagtagcaaataacattatactgtagatataaaaaatgttgaagattatcccaggaagtgctctggaagctgcttttaaaaataaataacttttaaactgccttttctcccttagcatttgcccatttgttctaaaggtagaagaacaactttcagtgtgttaagggtttttaatagttaatcacagttatatggcatttgtttttgtttaatatgtggatttttatgtaatgccacccagaggcctaggtatatcagtacattcctcagcattattaatgtcatccaaatagattgtctttgattactgatcactgactccatatatagggcagtgatttcaaaattattctactaccattgcaagtagacatgtatacagtaaagaaccatccaaaggccaggagcagtgactcaggcctatagtcccagcactttgggagaccaaggtgggaggatcgtttgagcccaggagttcaagactagcctgggaaacatagtgagaccccatctctacaaaaaattttaaaaattggctgggcatggtgggatgcatacttgtagtcccagctacttgggaggctgagggaggatcgcttgagcccgggaggtccaggctccagtgagccatgttcacaccactgcactccaacctaggcaacagagtgagatcctgtctctaaaaataaaaattctgaaaagttacatctaaattaggtttgagtaaatgaagtcatgagccaactgcataggtgatctttctagtggtagcaataccaaagtgggccttgtaaaaacaaacaaacaaacaaacaaaaacacccttttaaatgtagttcagggagaaggaagctagtatttcaacttactgtatgccaagcacttctaagtgctttacattattctctttaatattatttcttatattcatcaccacaatcctcatttacaactgaggaaacagaaggaggttaaatagctttgcccaaagttacaccactggcatgtggtaatgtagggcttccagcttgagtatatctaattttatagccatcattctttctctttccatctctgtatctctctgggagtcaggagacctatattcctgtgtttttgttgttgtcgttttgagacagagtctcactctgttgctcaggctggagtgcagtggtgccatcgtggctcactgcaacctcaacctaccgggctcgagtgatcctcagctgtgccatctcgctatggaaccttggctaagccacgttctgagctatggtaaagcacagtaataggttcacattcactctcccccatcatgcttatgccccctacctcgtctagaaggctccacacttcctttctgtgtgctcgttcattcagtcgtcagtcatttcgtcagttagtcagacaacagactttgttcatacgacattagtgactgaggttctgttgagtgacgcagataggaaataacctagctgcatggttgctgtctttcaaaaggccgtactcttaggatccacatacaggcccccatcttctgtgaagccattgtccccagccatcccattttgacgagtttttttgagtccctgtgaaactttggcttttttacatttatctggcagttaactaggtgctgctttgtgacagttcttctattattggatgcaattcttaattcaaatcatgtatcattacttaacttttcacctctttgcagcttctttctcccagaagattacaagttccttaagagcaggcttatacttctttgtataatatttcccacagtgtctcttaaatagcaaagttttttgacctgatttactaaaaaaaagtttgttgacttggcttaaattttattttcttttctttttttctttttttttttctttgagacagagtcttgctctgtgaccctggctggagtgcagtggtacgattttggctcactgcaacctctgcctcccgggttcaaacaattctcgtgcctcagtctcccaagtagccaggattacaggtgcccaccaccatgcccaaccaatttttatatttttagtagagatgggttttcgccatgttgtccaggctggtctcgaactcctgacctcaagtggtccaccctcctcggcctcccaaagtgttgggattacaggtgtggaagccaccgtgcctggctgacttgggttaaatttttaagtttagagtttactccctggttgaatgatttgggccaagttacatagcttctgtgaacctcctcagttttcaacaaaatgggaataattcctacttctcaagatgaaatatataatatatgcaaaagtgctctgtgaactctaaaagactatacaaatattactgattattttatactttttagtcaaagcccccctgtcctgcattgttccagtagacactttatgtaccaacatgtacttcagctgttcacattatatacttttatctctgttatcctaccatctaggtcaatacattttaacatctttatttgctgtaagtttatttctaattttttattctttattttgtttattcccatacttaacttttacttacgactacggatttaagtagcatgaactgtcttcagactggcctcctgtgatgagtcacaaggcccatcataatggatccagattgcaaaattgggagtaatagaaattactgttaattttcttgtaaggtagtttaatgcatttacttgcagtttcagatgggtagaaatggtacgttgttaggaattcactattgagatgatttttagtctgtattagagctctgaatactctgcaaataatatgtgagcactggtaccatcaaagcatgtgttgccttaggtggtgtttacagaccttgtcagagttggtagtaattccagaatataatcatttcaatagctaaggcttatggttaagacttccaaagtgttcagaatttactaaattgaattatttgaggttttgttactgtgttacttgtagtcatcaaatcaagctttattttactgccttcattgaaataagcagttttgaccatttaaaaatatttttaataggatacttattttctctagcatttttagagtgtggttcctgtgtggtgaatgtctgtcacctcttggaagccttgaaatacacaaattgactattgttgtttatgttgaaagatattaaaatgagatttgtaattgaaacgggcattacttatttcacatctggttgcttgaaaagtggccagatgcaacaattcttaatgcaagagagcctacggcaaaaactttgcaattctcaccctctacaaaacagctgccctgtgtgaaccttcagtggaaaaagaagaagaaaagcaaagcaaagaaaattcaccccaccacgttctaattacagatttccaataaaagtattaatatgattcctacatcaatgagctaatcattagaagtagaaggcaatgtggggaaaaaaaaaaaaaacaagaatggcagcactgacctagtttctagttgccaggaccaaagacgtcgtgacaccactgtcctttctaaatctccttaccttgcttaatcttaaagtgatggtatgtcctggtttgcctgacagtcctggtttatgcctgttgtcctagtgtgattttttgatagtgccctctttcactcttaaaagtgtcccagtttgggtaaggaggtatatgcccatcttaatttaatctctttatctcagagacattaattaggaagggtaagaagtgggagttatgagaatgtatcaaagggaaaatgatactccagttgagacagtgctggaaccaaaatgctgctgatctgaattctccgtaataagatgagaattggtttgcgaacacattctaaacatcacaagatacatcagattaatgctggttgctcttggggagttgtggggaggaggataaccaggtcaggagtttgtggtatcttttatgcaacactaacgttaagcttcctgtctgaggttttccatgttgtgagttttcacctcttgatactctttgaggactagtgatgctgacatctactagaaacacttcagagaaaaaaaaagatggaagataatagttctttagaaaaatggaaacatttacattattcttgataactttgttcttctttgaaaaagattagctgaacatccctgctgattaccttaataatctactctgaaattaattttatctactctagaaggtttgctgtggatagattctcctttagagtcctccagatttgatagctattattttttaataatagttaagtgcctttattttgtttaaagtactgaaaactgaatcaggtctcaggaactagttatgagcaactgattatttagctgggaaaagaaggtaaggaagaagaatatttgaacaaaggcctttaggtttttataaagacattatgcaaagagtgataaccatctttcttacaacctcttctcaaagtaaagcaagggggctgagcttcttgtggacatttaagtttgaatagggtactctcctgaaggcctttaaaaatacagtagcttgtctgtttggagtttagcaatcaatcaatcaagtcttgaacacctaatgctgcgctaagaattataaatgaactagaaggcatactcttttcatgtcttcaaatgacttaataatatacttggggaaataaaacaaatatacgtgaaacagatcaggtctaaattatgtggtattgactctatgagttactaggatgaattggcattcaaagagcatttaatttgtgccaaccaatagaaatatctcattgtgttacagcataagaaagatcaggaagccagaaacaagtcttagtggatggcagaaaataagaatatatacattcatttctacactaatgcatctattcagtatttcttgaggacttactgtatactataggcacataggagtgagtaggtacattgttctgagtagaacttatgtgttaggaaatagggaacaaaaaagtgggaggacaggtgggtgtgtgggcagagtatagcaataatattgttaacctatgcaaaggttaggctgattctgaatagagcaagagtttataatggaagattccttttaacacttaaaattcatgaaacgaagagctcaaagaaaatcttagaagccatctaatctactctcctttccctatctccacttgaaaaatggggacttaagagcagagctgttgcgacttgcctgaattcataaaccgagttagtggcggagctgaaagtcgagcctggctcttctgtttttaccatttgcagttgctcccacccctgcccccattcatgggttccacatccatggattcaaccaactatggatcaaaagtattttttaaaaataaataaaaatagcaatacaataattaaaaatagaaaatgtaaaatacggtataaacaactatttacatagcattacattgtattagttattatacataatctagagatgatttaaagtatatgggagaatgtgcataggttatgttcaaatactatgctattttagattagggacttgagcatcttggatttttgtatccacaacgtcctggaaccaatccttcatgaataaggaaggacaaataaatatatccttctgcctcttcagtcttaaagttagctaaaacatttcacttccccatgccaactctgtgaataccagatcttagatcctaaactaaaggtttggaaggcaatcattattcaggcataggtaggaaagtatgacttagaaaatgaatctgtttcgtgtctcaattttaataaaagtcttgtttataaaatgatgaaaggctcaatgagattaacaacatacaacttgtaataaatgttttgtaaccatgacactgatgagctgtgttttagacctagctgtcactaattggctgtgtgatttttgcacaaattatgtctcctcttttgtctttatttatattatgacagaatttaaattgtttcagttattttattactatatagatatctctctcttaaaattgcttgagtacagcacagacttcaaggaaaaaatttcttatgattctcagtgttcacataatttgtattaaatgtaacttaaatatgtgtaaaacaagttgtaaactatgtttatagctcttatatatttacacaaccaaaataaattttaaaataagttgtaaagcccttaacattaaaggtacaaatatggaaattactgctatagcatatacttttggggattcaacaccttttgctgcttaatgccatatctgattaaatttttccaagacttttttctttttcaactcttctgtgaaacattcctttctacagtattactggatctagtttgaacttcagttaactcagatgaatcatttacatattaaaagtttacctttgttcttctttcactaaccttagacaactaaagttgtgatattgggcaccagtgaaatcacaggtagaaactgtggcactgaaactgcttgtctgtattcagttataaaatcatacatataatctaaaatatgaattcttatacattttatgtcattaaaattaaggtaaaattgaaaacagagttaaaaacttttcctcagaaatcggaaacaatctaaatgtccatcagctgaatggatagacaaaatgtgctgtatcaatacacagcctaatctaggcagttcagcagtaaacaggcatgaactgctgacacatgccacaacctgaacctccagactcaacctcggaacctccaaaacattatgctaagtgaaaaaaaaccaaacacatgagaccatatatcatatgattccatttatctgaaatgtctaataaaagaagcaaatctatagaggcagaaaagtataatagattaacagttgtctgggattgggggtagtaattggcgtttgattgtaaatcagcatgacagatcttactaggtgatgaaaatgttctaaaactgatttatggtgatggttgcaaagcttggtaaatttactaaaattcgttgaattgcacattcaaaatggtgaactttatgctatgtaaaatatgcatcaataacgctgttttaaaagctttttatgaagacttctagatctcctaagaatatttaggtatcagatattttcgcccttgacccttccaaggtcagaagacacagctgaaaaaatacttttagtggaaccaaagaatggatccagtaactacagtatcgtggattctagctttgactttgtcactgactgtacttgggcaaggcctgggcaagtcacttaacctctttttgctttggtttccccatctgtaaagagggtgttagtttaaatgttctccaggatttcttgcacacatgagagtcgcatcctcacatttctgttatctgtgaatctctacctcctaatgattccccctccctcaaatactctaacaaagcccctttattcagcatggcatatgtggcatattgcttgtctgactaattcttgctcacgcaagcttcctgaccttactgcataggtctttcaggtacacagttctcaaagtgttgatctgaaagttccgtacaagactggctccccatcactcattaatctcccagaggctaccttctcatcctatgtaactctcttatggaagctctcccatagataacaatatacttccccttcaggcagtacatggaagaaacaatgggctatacaatggaaccatcctatgagattacacagaatgagaacctggcccattgttttctcctgctgcctaaggaaggagttgtgctctttggatccctgtacagattttggcttgtccacctccctgaattcccaagtaacaattaagcaatctgcctccttccgtcttctcatttcaatgtgtaggatatttgtcaacttgcccagagttgctgtaggcattttgagctattcatctgactgtgtgcaatagataacaaaaatataattaggaggaggactgaattaagtctgaattttatttttatttttattgcgggggagaggtgcttactttagagtggtaaaagttacttcttgtccaagttttcatcatcccctccttccctctgtgtttcaataaaatgtttccaaagtttcaaataaaaagtttattaaaatagaggccgtgtttttaaaaataaaaatgtaacatcttacttcctagaggtatctgaagaaaagcactccaggagtataaagaataaactagatggttggaatgtggtttattagtccacaaacctgtcaggaatcttggactcttttcctaaagctatgcagacatacaacataactttggaagaaccagttaagtttgtattctaactatgccctgtaatttaggaataactacctgctaaacactgaaaatctgttggtggaaatcatcgggtaaaaccaaagcataagttatattattaggggttggtaagtggttttgtatatgcaataaaaaggattagatggctgggcgtggtggctcacacctataatcccagcactttgggaggccaaggcgggcggatcacaaggtcaggagttcaagaccagtctggccaatatggtgaaacctagtgtctactaaaaatgcaaaaattagccaggcatggtggcacatgcctgtagtcccagctacttgggaggctgaggcagaagaatcgcttgaacctgggaggtggaggttgcagtgagctgagatcacgccactgcactccagcctgggcaacagagcgagactccgtctcaaaaaaaaaaaaaagattagatatttgaagaaccatgggatgggtgtcccgttaactgtccatagggccaaggaaaatggagaaagatgaatttgaaataaaattctctaaaaatagctgaaaaagaaaaacttagatatgtaagtgttttatgatgtgaacattcaatgaacagaggaaagagatgtgcctaggaatgtttggtgttgaagatatttacctttttaataaaagagaacaaattaaacaagcagtcttcctttcttgtaggaactgtatttcagggtaattacatggctttagttgctgaaggaaagatcttccttatagaaaaatgcctgctgtctgggtacagtggctcatgcctgtaatcccagaactttgggaggccaaggtggacagatcacttgatcccagaaattcaacaccagccttggcaacatggtgaaaccccatctctacaaaaacatacaaaagttagttgggcattgtggcacgcgcctgtggtctcagctactcaggaggctgaggtaggaggatcgcttgagcctgggagtcagaggttgcggtgagctatgatcgcgctgctgcactccagcctgggtaacagagcaagaccctgtctcaaaaaaagaaaaaaaatttcctactaataaatgtggaaagagtggtggaattagaaaaacatttcataaactccaagtattgattcaggaaaagatgataaagtttgttacacctttaggtgaatgattaatgaaactgaacatccttgtaataccaaagtaacattgcactgatgactgtctaattgaaggagaaaaagtaactgtacaatggagagatgagacatatcaccattctaacttagtggtagattttaccatggctgatggtcagtcatatattttgccttctgatgtgatggaataggaagtacacatcccctatggtatattcaagcctaaaatgtttaacttgaatccagaaatccttggatatagtgtccagtttataagaaacacaggggatggagaatcaagctaaatgatacaacaagaaaacaaccagacaaattcagaggttgagacattctatctgataactggcctgacctcttcaattagtcagtggccttaaaattaaggggaaggagtagtcatgctagatttaaaacagcttaggaacatacagccaaatgcatttcatcatactggattagattagggttggagcaaaccaactataaagaacatttggggtcagctggggaaatgtgactatgggctgggtattgtttgaaatgaaaatgtaattaaatgaaaagatggagattattgacttgaaaaagcagaggactaccaggaagtaccatatctcattttgattaaaaaatacacatgctgtatgtatgtgtatatgtgtatgtgcttatgtatctgtatatacatatgatcatacatatgcccagaaaaagacccagatgcataaactttaagagttcaacattggttatatctggtagtggaagtataatcattttgtttttaccagtctgtattttctaatttttaacaatgaacgcggattggttctataataatgaaaggtggttttttttttttaaacaaaaaaacccctaccttttcagatagaaaagcagcagtgtattctttccttcaaggaaaatgaaaatgtttccttggaggaaagaagatataaagactagaaaacactctagtatctttaaaaaccaccaagctttcaaatacaaagatttaacatatgtaaactgtattgtacttcatttgaaattcagtatctttactaaagagatttcttttatcctatcctacacacgtacagtattatttaatgatgtgcacacagaactctgccagcctgaaacagtaggtctaagacacgtttgttgtttttggctcccctgtgttgatctaaatcactgcctagtagcccttggaaatttctatcccaaaacgtcccacaggtgcccaataccatggattctcattccccaagttcattctcactcttctctcttggttgagtcttgcctttcttcactctgttccctttccttgttcctgccatccaaagcttctctgtctttcaggctcatctcagatttcctctctttcctgaaggctttttggattccttccatctccatgcacagtcagaagggctctgttcatctctgaatatctttcgcactccattgcatctggtttaaatcccttctctgcctcttattagctatgtgatctcaaaactcaatttctttatctgtaaaatggtgataataaatgacttcgcagggttgagggcctcaagtcagtggcgagtactgcagtagaggcagaatacatagctcaacagaaattactctagtaatggtcatgattgtttgcacttctctcaaaccacctactcgtatattagagtgcattgtgcttgtcttatcctctttactaaaagtaggaaaatggcttgagaattgatgctcagtcttatttatattattctatccctagttatgtgatacttaactgtattgctcggtatttagcagcccattatctaatcataacatcaccctcattctttctgagcttgtttcctttttgtgaaatggggctaccattcaatctcaccgaatttttttttttttttttgagacagaatcttgctctatcacccaggctggagtgcagtggggcaaactcggctcactacaacctctgcctcccaagttcaagtacttatcgtgcctcagcctcctgagtacctgggaatacaagcatgtgccatcacacccagctcatttttgtatttttggtagagacagggtttcgccatgttggccaggctggtctcaaactcctgacctcaggtgatccacccacctcggcttcccaaagtcctgggattacaggtgtgagccaccacgcccagccaatctcacagaatttttataaagtctagacaaatttttattttaaaagacttagcacagcccctgacagcgtaggcactcaataaatgtggaatctgaatcttacttaaagctagtttatattttcaagtcttcttacttttactaatgctgctttaagatatattctataagttcaaatgtaaagttctagattgggaaagaatttataatgtgtctaataaagattgttagagacaaacttttagactgaaccatctactattaatggactgatgaatcttaccggaaaataaacataaaatatactctgtgttgcctgtggtttaattgccatcaaaattaagtttattatgtactgatttcacagttacattttattttcagtcaaatatctatttgttggtgtgaagaaaatatgtctacttccgctaagtgaactttaaaaatttgtacttgcttttgaagattccatactctatataccgtctcttcctgaagcgtatttatgtagctcctgttaacataagagcgataagagtgttgcttgatgactgctcttattgctttattaaagtgtcatgtaagatttaaatatttgattataagaattcataatataattttgaaagcctactctgttccagacgctgatttatttaaatcatctctaattctcacaactccgaaaagataagaaaacagagatgtgacaaggcttgaatgcaaacccaggtctgtttgactctttgttcattttgaataaagacaaattactcaaagctttactgccaaaaactattatctggttccacattgaaaccctattcaatagttgttattattttcttcttttgctttgaataacctcccagcattgttgtgagtttcaaacgaaataaaaacactatacagatccaaggtgtttttttttagagtattgttacctcaaagtagaaattttcaaatagtaatgttatcattttcttaagagcaaggaactttgtcaatagaaacaaaaacatcataccagaagaaccccagaatgctgggatgactcatgaagaatctgtgaatgaggcaagagaacattcgtcagcaaaatgactccgtgaactgatgttcaaatattatcaaattttaattaccgagtcataattgagtacttactttgtagagagcaccatatctaaaccctgtggtgaatgatgacattttcataggtaattcctccacattaagtgattcatcatagaaaaatgctttcatgctgatgacttccaccatgactgttggcattaaggatcattgacctgaagaactgatttgaacgtcttactgcatcattttaatgagatagagcatcgtttggagctttggactgggaatcaagaaacctggtttctagctcaaactctgctgctaatttatctaggtcatgctttgggcaaatcatttcattcctctggaacccattttccttatatcaaaaattaagagttggaatatgctaatctccctcctattaagtttcgtgagcccgtgatttcaacagtacgtaaatttcctttagtacagtcacagaactggtaagtgacaccagctgaaactgagtgcagctccgcggctctacgcttgctgtagaacctttgtgaattcccactgtgcttcaccagtgacaggatgtgctacccaataaatctccatataactgatcttgaaaaattcattgataaaatctgaaaactgaaaaagatacatgttttagaggtttaggtttcccacaacatgaaaatgtgtcagttgataatatagttcatggtattttactatgctagaaaacagcttactagagaatttcagatattacatgcaacgacaagttaacatagtttaggtgggacgtctttggttcaaagttacagtaatttcaaaagtgtttagttgatccctagaaagtggttaaacaggttagtctctttttcaggtattagagggaagttaacttttgaagctgggcagaaaaggaagttttcagttggttttttccttttgagacttttaatttatcatcagacactattttttcagatgaaagtgccttttatactgtcacctaggtatgagtcaagtatgaaaaggaaatagtaactcaggatcagaacatgaataagtatgcaatatggagaatttccattaaattttaaataaatgaattacagtcatattattcagtatctcaacattaaaactcaaaaagaccttaaggattattctgttttgtggaaagggctttttctgattctagagatgagaaatgtggacccaaagagttgacacagtaggtttgtggctgagccaagacaaaaacgtaaaacctaggctttctggctccaatgtcagtgttcttttctactgcttctgagttaagaagacctttttttttttgataccaaagatacatttactggagttattggcttctttttttttaagacagggtctcactctgtcacccaggctagagtgcagtgatgcgattacagctcactgcagcctcggtctcctgggctcaagcatccctcctgcctcagcctctcaagtagctgacactacaggtacatgccaccatgcctggccaattattttatttttttatagaggcagggtctcactctgttgcccaggctggtctccaactcctgggctcaagggatcctcttgccttagccacccaaagtgctgggattgcaggtgtgagccattgcacctagcagcattattttcctttaaatcaaaataatataattgtttaatataattatgtccataaaatatattacttttgaaaatctgaacaaaattacagtttttggttaaagaagaatggatttgcctttcaaaaaaatgatacacgagagactgaggcaggagaatttcttgaatctgggaggtggaggtaggttgcaatgagcctagattgtgccactgcactccagcctgagggacagagtgagaccctgtctcaaaaaaaaaaagacacagctgagtgtggtggcgagcaactgaaatcctagctgctctggaggctgaggcaggggggtcacttgagcccaggagttggagactagcctgggcaacatagcaagaccccggtcaaaaatttttttaatttaaaaaattttccaaaaggggcacagatacattgaacattgaccttcctttgtctgcttttatgggactatccggcttgttgtgatggttgtggtgaaatttacatccaggatacaggattatttgttcttctcaaaggagtgtcccattggcccagcatttctctcatgttgtctctcccctgggactatgaagaaaccctgaactgatgcaaccaccacttgaaaataaagttccaagccaatctgaattgcactaggaaaaggcagccattcttttgggtagggggagaagtgagcttggctggtcattctggttgttagcaattatctggcttccgtgggagcatcatccagaaatttacatcttattgaaacaagaagaaaatggatgctattatcagttcgttaggtctctaaactccttcttgaatgatacatgtgatatggatgtgctgttctttcattactctcatcatcaacaaaaacaatatgtgtgttttaatgccaaccagggactctgctaggttctagggatgcaatgagatctaaatgcttaaccttttagaagctagcataaatgttagtagcacttacagcattaaatgaagcagatttttaaatgaggttatagcaaaagaaaaaaatactgtacatacaattttataccaatactaacatagcttatttcacacaaaagaaaaagctatttaagcaattttaaaaattcatattcattctagagaataaattccaaatttatagcaaaaaaagagtgaagttttcattagctttcaagaataatgcaggctccaaagtatttaatattctatattatgggaatattttatgtaagtcatcccaacaccaagtaatgctaaaaataactttatataggttcaataccatgattttattaactatagatttttagaccttttcttactttttgttattgaatcattcacagcttttattggttgaattgccttctcctaaaagtaccaaagtgtgaagagtttttatggctgagtaatattcagattcttgtagccaaagacaggttctgtgaagtaatattgaagactaaatgttgaagagtagctttctctaataccaagcggtcaattttttcaaatatcatgaactggggtagagttaagttttcatcctcctcattatagaatcattcctcattatccccattctttctcctgctgaggatgtggtggtgtactcaaagtcacatccatacccttctgtctccaaagtcctaggagagatggccctcttctcaacctctacattgcacagaaccttacatccctcaacagaaggagtacatagtgcataaggaaagtggtcttttaccactcctcctcactctgtaacattaccaaggactatcctgcaaggggaccatccataggatgaatagcaatagactgctgcattgacgtgcaaagtgctgacaacccattggtgtacaaagcaccctaagcaagatctaaagttctaagatcttatcatgtaaatcaccagcatgctgttttatgtatcttattgtaatatccttccaatcagtattataaagggcaggacactgggggaatcttaaggctttgaagatagggatagtcacgtgcatgtcttataaattctctgatgatcatatactgtttactggtagtaatgactgtacttaaacaaatatattgtttctcatatcattgcatgccaattgaccttcaagtttaagccaatgaaaagatcactcttttaagtatatttggataattttgatatagttacatgtgaactcattaagtatagaaaccttggcttattatttaccacctaagcctaggtcagtacctggtgcttagtaggtatttgatgaatgatgggatgaataaatgtggaaataagtcttttcagtatctaaagacaaaacagatacataataagatacaaatgagattggctcatctatctttattttcattcatttgaatgtccatgtaagcaagttatttcttaagtgacccagcactgcagtgcaactatcattaacataaaatatgattaaataatccacattgtataactgttttgttagtaatgtagggatgctttgcgtgttgcttggtttgtgtatgctgccaaaagtgtaagcaacatttactgagctgctatgtggcaggccctgtgtttattaaaattgtagtttttgctaattgactgttttttgacacatccgtcttgttcatcattgtctacctagcacctagctttaggcttgccacatattatattggcaatgaatatttgttgaacaaacaaatgcatgaaatgtaatgagtaagacaggttttcgctttcaagtaaaacatagtctgggggaagacggaatgtcagaatgtggtgggtgctataggagtaggtgttatcagattctgatgctatggaataataaattgttaaaatatgtaatcttatgtttcagaagctaaagcacagtatgggaactattagaggcttagaaggcctcactacccactagactcagaagttgaatagtgtctgagaaaaaagagaatagaagtaacagtagatgaagagtccagaagtgagaccctttgaggacatgaggacaggtggaaggactgcatctgtgtgttgccaaagagtaacagagactggtataggacttgagttcaattcagtcatatccttaagtattgtgccatcgtgtctggattactttgtagtataagtaaatttccaagcatggggaggaaaggagaagctcctttattgagaattcaactgaatatagagaaaactaattttacacaactgtaatcactgtagtcatttggacaaattagcaaacccaagttttgctttaacttggattgccttaataaagatgttttggggcttaatggcacagttgctcaactcccccactttattccgtgatgttcagacccagccagcatttccccatcaggctcttgcaccatgattgacagggacacttttactagtccccttgaagaatgaatagttactcaatggagattaaccagatatatatttattttactcagaatatcacgataagtataattcagagaattattgccttctaatatactgccctgtgtgggggcgtctttgaaagtccgcaaagtcactgcaattctaataggccactcatgtgacaagacctgctcccacatcggtaatttggcacagctagtatttctccttgccaaaaagggcaaaggccttgagcaagaagccagctttttcctgattacaaaactgaccacaattcctcgccaacctaacagcgtaagtctatttttttctggtggtgtgttattcttctcatagagaactccattttttcattatgacatagcacttatcgtttaaacatcaattgatgttcaaacatcagctggtgtaacattgctgcagttgctattgatggataagctgaagtttttaagaaagcaaacccgatgtataaaattgaaaccatatcaaacccttcttcattctctcagctatttaattttacagaatttagatagcagtcagtatcattttgggcttcacaaatcagtagagtaagtaccttaggaatataacatttcagtagcatgctgataccaacgtttaaactatggatacatatttgaattccaaatttttcttcaaataatgtgattagagattcaaccaggaatagacaccgaaagaaaactttgcccaaataagctttctggtatttcataagcaagagatttaagttttccatttaagaagcaattgtgaattttacaacaataaaaaatgcaagtggatattgaacagtctctgctctgataattctaaatacagtacagttcacgcccctcacaagacactgaacatgtgggtcaccggcgagacagtgtggcaatattttccctgtaatgtaccaagtcttgccaaagcagtgaacattatgacacaactttttgtcacagctggctcctaataggacagtgccagccaattcaagcccagtcctttctgtgtttattcccatctctcccaaatatttggaaactgatgtcttgactcatgggtgtattcacaaattctgttacttcaagtctttttcttttaacggattgatcttttgctagatagagacaaaatatcagtgtgaattacagcaaacccctattccatgctgttatgggtgaaactctgggagattctcctattgacccagaaagcgattccttcactgatacactgtctgcaaacatatcacaaggtaaagttccttccagatacggctattggggacgtgggggcatttatgtaagggtaaaattgctcttgtagtttgtcttccaggttgtgtttgttttaatactatcatgtgtacactccagtattttaatgcttagctcgttgctatcgcgttcatttaaaaacatgttcagaaccttaaaaaaggaaacctaacctaatctattttatctctgtgcatggctcccatttcctgaattttaagcattaaaggtatagttatatccaaaaacaatcctgttcatttttatttcctgagtttgcatagatttcccaagaatacataagggctttttagacttgaagggtcactttttcctcttttcatctcatatgttagagatctctcataactgtttttatccctcttgcagcacttttattcctcttgaagtactctcagctcttttctgttctattttgaaatctaggtattgtgtgtgcacttcagctctcccaaagaattgtaaattcccagagtgtaggaccaagtggtgctctttattagatttcttaggatacttcctagcatagtgcctaatgcattgcagaatagattgtcggaaccttgaaaaatatctgttccaagcatcacattttatgcataaagaaaatgaggtccctaaaacagtaaatgcctattgcaagtgactacctattaacttctcttcagatgtgtcagaatcagatacctccttttcaatatttctttcttggccattgcaaaatataagttctccatttctatagctccttctactggagtttcttagcacagccttttctgttttgtattgtctcgtattgatgtctatatttctattcattttatttttctcttctcagattctgtgtaaaaatagattgttagctagtgtgattcatgttttataatataagtgctaaagcattaaaattaagtcacttaattgctgaaatggatggctttacattttaaccttttaattttcctggaagcctgaagtttgaacatattagtcaccgtttttaaaatataaagctttttaaaaatgagtaagaaaatgtttcctgaagtactgttttattttattacagtaatttgattcaacatgtatttctatcatctaagcctcttaactaggagttttgttttattccataaattgttgttattctgtttttctgcaagccataaaaattgttgctatctttcttcagttattaatttagcctgcctcagggcagaatgtcctggctatactgtgaaatagttcttgagtcaaaatttgatagttttgtctattttgaaagaacatgtctagaatgcagtgcaacaaatatcaacaaataggttaactgagaggcaagtactgtttgtggtaagggatggttatgtgattcaagttagttttcattctgtgctaatctctaattttatgctttgaatttactctgagtttaatttttttgagtctcaatttcctctaaaagaatgatccagtacttttcttcctaattaacatagtgcagaatgaaattattagcaattaaaacattatattttgtaccaataatttaacccttgtcttatagggtctctggctactacttcttcataagcactgtttctctgttaaaaatgtgagctcctaaaggcccaagacctatgattgttactcctattgcattttgtaaatgacctttaaataattactccacctcttccaaaacagacagacttaaaaataaattagctatatgatcatcattagccgaggccagcagagttgaacactgtggagttgaggtatttggcatgggtacagtagtcctcttaggtgctccttcttcctcatcataggcaaagtgaaattgggggtgttgcaaatggttgggtactgctatttaagaaaaagtggcacatttagtgtgaatgactcagatatccaggtagattggtcatattcatgagattaaaaatctcgactacacttagccactatgcccaaagaggacttccatactttttccaaggctccatcattgctgtgacccctttatattattcccctttctctttttatcaagagctcctcaagcaaccccaagtaacctcatgctggctctgaaaccatttccactagtaaaaattggcaagattgaagggaagcttccacaagctcaagctgaatatgcctcctgcttttagtgccagacttagtcctgtgtgaattctacaattttaagtcgttgcaccagagccttgaaagatgatgacacacttgtcctttggagctgattgagcaatggaaatatgccttagagacatgataaatgctgcaatagacaatccttcaaaacgagtctctcctgagataggagtgagtgattgattgcatgccatttttattgagggatacttaatctgtggttacatatctccaggcaactgtatattcagaaacatttagataactgaccaaagttttcacctttccagaagtttaaagggacccatgtagtaccagggaatataaggaccagtcctttgttggccacatatttgctgtgtgaatttaagcacgccatttttcttctctggccttctgtttccacatatattaacagaatacacaggattaatgggaggattaaatgacacaatacttgtgcaagtagatctaaagccctatatggaatttattgctttagccttgtagcgttaatcacttgtggctagaatagaaggctccgtttaaaaaaagaaaaggctgggtacagtggctcacatctgtaatcccacaactttgggaggccgaggcgggcagatcacgaggtcaggaggtcaagaggtcaagaccatcctggctaacacgatgaaaccctgtctctactaaaaatacaaaaaattagccaggcgtggtggtgggcgcctgtagtcccagctactcaggaggctgaggtaggagaatggcgtgaacccaggaggcagaggttgcagtgaggctgagattgcgccactgcactccagcctgggcgacagagcgagactccatctcaaaaaaaaaaaaaaaaaagaaaagaaacctacattttaaacactttatggatatggaaaaacaaaaaccgcagaactctttattgcacaagagtaagtggcagttatatgaatgaagcggggcatccgcatgatctcctgtgagtgttttgagaagatgatcaaacttagagaaagcatctttgtgtctaatttttttaaatgatgaaattatttcccactttcattaatattttcctgtgaagaaattgaagttattctttgggcctaaataaaagtgacaattacatgttttcttctcagaggcattgagaaacttggattataatgtttttcgtacactgaagtagaagtccagaaaagatttgagttattgacacagatcttcttttttttttgagacagagcctcactctgtcacccaggctagagtgcagaggcctgatatcatatttcaccacagcctcaacctccctgggcttcggtgatcctcccacctcagcctcactagtagctgggactacaggcgtaccttaccacacccagcaaatttttgtaatttttatagagacaggatttcaccatgttgtccaagctggtcttgaactcctgggctcaaggaattctcccgcctcgacctcccaaagtgctgggattacaggcgtgagccatcgcagcctgcccctgaattccataatttcacgtgtaattagaattcaagacctttttcttgaatattactcttgtccatattaatttttttctgagtatggctctagctttatcatttttttctgacttaactctgattaacctcttttttcatcaccagtacttggcagattttgtagatttctaaactctgaaaatcactgtttttctgaaaactgtcatttgtctcatactttcctccaaaattatgaattataggaaacaccccaaagaagtatcatttacattagctgtttacaagaaaatacagggtttcatttttaattttattttcccctactatctctaaggaatacaacttgtcttgaaagctccctgacagcagctatccatttaatctgccaattgcagtataaaaattggttattaaatgaaaaacaattgtatacctctcacagaggttgtcatatattactatttttgtcagcattctcacttataactctgttaggataatcctgggaaaatttctaaaatcttcatagctctttcgttaggtacatattccttgagacagaggaaatctgagcaaagtaaatttcttcattatcttagatcaacaaaagtgatacagagcttctgtcctgttagctccctttggacgcttaaaataggcactagaggttgtccagtaaatgcttcatatccatctactagtgctgaatatttgtgaaaatataggtgataatgaattagactcgtttgaatggaattaagtttctgtaaagttttaccagattgtcttttttttgttttttgttttttgttttggtaaaagcagttttgcacctgtaactaatttaaagacgaagaaattgcacatgtaactgatagcaactgccatccaactcttataacctcagaatcaagatcacgtggctatttgagtacacagtgttttaaaccgtgtaatttttatttgagcaagggattgccaacacaagatcgaggttcccacaagtggtgaatggcacttgtggttaacactgtaaagcagatttaaaacagtcaactgtcaattgcctacaagggaattattcctcatcacctcatgccaggtttttatatggccttttagctgaccttctaaatgagaaactttgccatccagtgcaaactgccaatagtcctaaaatgcctatctttattatcagtctaataatatttattgagtgccgattttcaaggcaccatagtgaatgctgtgaaatctagacactttttccctggctttcaaagctctttataatccaggcatattttatatattttaccttatttctcaccacattccaggcattggcctgtcttgctctgttcacactaatctctttgtcccaagagtaaggccgacccacccttgctccaagcctagtatgtcttgaaatgcctttcctaattcttccatcttttcaaatcgtccctgtccttcaaggtcagcttcaagtaacctctactccgtgaagcattctctgaattcattgctgttcattgctccctctctcctctaaactgaaaatgtgttcagaatatctctcttctgccgcttccactgccttcagcccagtccaggacaccgtctgtgcctggctgctagtctcttgatggggttttcagcttccatcctaacctcacaacagcctagtctcaaccggtcacccacagagatgatgctcaaatgtgagtcagatccgtcactccacccatagccctgcagtggttccccatttcacttgtaacaaaagtccaagtctggcccctacctcctgccctaccccagctgacccctctggtcttctctctctcttccacccactctgctccaagcacgccggcctccttgctgttccttccacattccagatgctctcctgccttcgtgcacctgccccagctcttgttcctgtccaggaccctcttcctctggcattctctgggccacctctgtcaattccctataatcttggctcaaatcttaccttagagtgagggtgaccttggccttccctatcctaggacaggggaattacatatcctccccattgcccttcctcctctactctacaatttcctatttaaaaagcatttatcgtcttctaacatgccatgtaatttattggtggattctatgtattgcttactgtctgcttcacctccctggaatgttaaccgcatgaaggcagagatctttgtctagtttgttcacccactgatgtattccaaatacctgaatagtattgctcattaatacttgctaaatgaaagaatagaatcctctaacacttacggcttctatcacacaatttagccctgagttcaaactgtctggtattatttcctgttttatgtattccctaagccaaatcatatagtcactgaagaaaagatccatgttttattctatattccacaaatgccaaacacataataagtataatcaggtcttgttgacttattaataccaagctgatctcctaaggtcagagactggaatatatttagcaaataaatacaaaattttagtgtatgttaaatattattctaaaaccaatgctaatataaacaaaccaagtactggatatgctacaaaccaggcacaaatatgttttgaattatctgttagttaatttgcaccgtgtccctccattagtttgagtagcattcattgaatatcatttgaatattaatttaaacatcatttgtttgtgagttacccaaatccctggcttcttctgcaaatctacccaccttttgatacttccattatttatttgaacatccaaaacacttatttgctagcaatgtttaaaaaagagtagcttatttaattagctaatatctaatatatgaagcacttaaagtattaattgcctgatatgtaataggtgccaaacacgtcagttctgtcttcttctcatctttaaaatggaagttaatacagacataatgtctccccttgggtcttttaagtcagatctttaggaaaaagtaaaatattctcattattcttattattttgcttgcattagcaataaagtatgcctgatttaagttcactggacattatcttactattatctatactttacctaaagccctgcctttagttttgtaaataaaattatagacctattagatagattgagcaagtttgcttagtggattaaaatatgatgctaataagagccaaagtgagtttgataatgggttggccagatttacacagaagtctttgccatttacaaagagttctgtttgccattgatacagtcacatttctagccacaattacccaagatatgtaaacagttaactcaggagaaaccaactcaattttcaggtatatgccatatacaaaatctcatcacctttgctattatatacacttagtattatttcttaagcaatatcatgtaatataaggggcacgttgatgacagggacatgtacctttttcttgggatttcaatatgaatgaccatccaaatcttgatcatcccaatggctccacataatttggacaccatgtctaccagaaagctatccctgattatttcaggacatgttagtatctttcttttccacatttctaaagtacttactatctctatcacgagtctggtctctgtacttccttctgctactaaacatctctcaccttggtaagcttctcaagaaccacaatactatgtgtttcttgtaaggcctgaaaaacaccttgcacgtagtattaggtgattagctatcttgatttaaggttttagattactgattgaacatttactgagctgaagatatagagaaagaaaaatgccaaagaaaataaaatgaggaagtttggaaaagagaaacacactagtaaaatatgatggtaacttctaagaagcaaggtttataaaatagattgttgatacaaagaaaacattataaaaaaatgggtagcttgaatggatttaacccccaactttatttaatttaaatggaatgcctcaaaagactactcagctgatccaaacatagtaacttcccaaacacaagactcttgacgtaggcctcagaatttggggaaaaaaattcctgcattgtttaaaaatacagtgtccttgtaaagcagaataggccttatatacaagccaaatatatcagttctaaagcaaaaacaaaacttttcctacttactcttttatttcttttttttttttttttttgagacagagtctcactctgtcacccaggctgaagtgcagtggcgccgtctcagctcactgcaacctctgccccctgggttcacacaatcctcctgcctcagcctcccgagtaactgggattagaggcacccaccaccacgcctggctaattttgtatttttagtagagacggggtttcaccatgttggcagggtggtctcaaactcctgatctcaagtgatccgactgcctgcacttttcaaagtgctggattgcagatgtgagccactatgcccagcctgcttcactcttttagataaaatgtacaccctttgaatttttacttccgccatttacactgatttgaagtccttggttgaatatgtatttagccttcactgtgcaaggaagctggttacaaaaacagatagtttattaaaatacttgtgttggtttttaaaaaagaataattttaatacagtttttctcttctttctttttgctctttttgttattttttaatagagacacggtctggctatgttgttcagactggtttcgaactctggcctcaagtggtcctcccatcttggcttcccaaagtgctgggattacagatgtgagccaccatggctggccttaatactgttttatgagttctgaattgaataatttttaagtgaatgtcctaaaattctatgacaatccttttaacacaactggaagagtttttgttggcttacttggtttgtctgcatgtttccttctgtcatcccccactcctaggacccatatggaacattctctcttaattaactcttttattgaagtataatatacttagaggaaaaatgtccaaatcattttcacaagtgaacatacttgcgaaattagcacccagacaaaaaaaaaaaaaaacagaacaataccagcactccagaagccctctgactattctaatttctaactcattgttaagttttgcccagttttgaattttatataaataaaattacacattgtttactcttttgtgtctggattcttttgcttagcatttattcgtgagattaatcacactattgaatgtaattgtacttcattctcattactgtatagtgtttcattgtataaatatatcacaacatatttatcctactgttgatgggcattcagatggttttcagtattgcaaatagtactgctatgaacattgtcctgtaggtctcttagtgaaggagcgtatgcatttctggtagctatatgcttcagccaataatagagtatgttgagcttcaggagacgttgccaacagttctgaacaggactctagaaatctatacttctactagaagtgcatgagtgttctagctcttctacaccatcactggtacttggcattctctgtctttttcacgttagccattctgatgggtgtgttggtatcatattctaattttaatctccccttttctgatgtctaaaaagttaaacactttaaaaagcgtttgttgtccatttggctatcctttcttgtaaagtacctgttcaagtctttcacccatttttatattgagtactttaggtaaacgttctaaagcataccttgtcagatacatgtattgtaaatatctcctcttactctgtgtgctttttcgtttacttaataaacagatatttctaatcaatatagtctgatatactagatttttcttttacagtaagtgctttttatatcctttggaagaaagctttgcctactccaaggttgataaagtgtgtttttattttaaaagttttctggttttatatttcacatttagatccataatccacacagaattgacttttgtgtatgttgtaaggcaagggtttatctctttcatggggatatccagttgacctgcttcgtttattgaaaagatcatcctttgcccactccccagcagtgacatttctgtcataaaccaggtgaccatataggtctgggatttattctggacttactcttctattgcattgtatttttgcaccaattaagattgccttaagtactgtaactttataaatagtttgatatctggtagtataaatcctccagcgttgctcttccccttcaagatttccttgccacttggcctcttgaatttccttataaattttagactcagcatatcaattaccacacaaaagtgccgagattttgattggaattgttctgaatctatagataaattgggagataattgaaagctttacaatattgagtccttcaatccatgaacatgaactatcctttcacttatttattctttaatttttttaaatagtatatttgagttttcattatggagatcttacacatattttgttagattttttcccctgggtatttgattgttttaatgctgttgcaaaaataatttttaaatttcattttctacttgttgctggcttatagaaatataattggtttttgaatattgaccttgtacccagcaactttgctaaattattttattaactataatgagtttttttgtggatttttaaaaacacagtctgcctaacatggtggctcatgcctgtaatcccagaactttgggaggctgaggtgggtggatcactttgagctcaggagttcgagaccagcctggccagcatagtgaaaccctgtctctactaaaaatacgaaaaattagccaggcatggtggcatgcccctgtaatcccagctacttgggaggctgaggcaggagaattgccctaatgccagaggtggacgttggagtgagctaagataatgccactgtactccagcctgggcaacagagtgagacttcgtctcaaaaataaataaataaataaataaataaataaataaataaataaataaataaaacgaacaacaacaacaaaatacagtcatgtcatctgtaagtaatgttagttttagttttatttcttcttttccaattattctttgtctttttcctttgttgcattggatggatttccagtacagtggtgagtagaagtaatgatagtatcattaccttgttgctgatctcaagaggaaggctttaaatatttcaccatcaggtatgatggctactctaggatttttgtttgtttatttgtttgttttttatagattttctttagcagactaatgaagttccctttccttcctaagaggttttttatttaaaaaaaaaattatgagtgaatgttgaattatatcaaatgctttcatagtttgttgtggtggtggttgtttttgagacagggtctcactttgtctccaagctggatcatggtgcattgcagcctcaacctcctgggctcaagtgatcctcccacctcagcctcttccagtagctgggaccacagcacatcaccacacccagctaatttttaaaaaattgttatagagacagggtctcactgtgttgtctaggctggtcttgaactcttaggctcaagtaatcctcccaccttggcctcccaaagtgctgggattacaggtgtgagccactgtatctagcctagaatattttttatagtgctcaggagaaagattaaaagtatgaaaagtgtctactatgtatactttaatatcatattgtaatacatttgaagatactatatggtataactaatgaaaatcttcaaatcagctcataaccactagagatctggctgtatctgttttgacacttttgttctcagtatctgtttagcttaagacccttgtcttctcattaagagtgcttgacacagtaagttgaaaacataatttcaaaagagcatagagtgtcacatggtttgccagactaaacaactctgagtaagaaagtggctttccccctatggtaatgccaagctactagaggaccttcagtggtaaagtatgatttaaaaccctgaccccatctgtcttttcccatttgcagtaagtcctttatagtgtttgaaggtgggcacagcagggaaacagtactctggcagatctgcggtggctccctcctttctgagtcattacacactcttctggatcattcctttcatttttccttttcctctcctctcccctattttcattcccctatcactgcaaagccaaaaccaaaacgtggaaggggacctagccgaggaaaacattccagcttcttttttctgatctaaacaccgttcttcttcttttttattttttaattaataactttatttttagggcagttttagtttcagagcagaattgagtaggaagtacaaagagttcccatatacttcctgtcccccaccacgcacaatctcccccactatcaacatcctgcacccaagtggtacacttgttaacagtcaataaacccccactgacacatcattatcactcaaagtccatagtctacattaagattcactcttcgtgttatattctctgggtttgtacaaatgtataaggacacatatccaccattgtagtgtcatacagaatattttcactgacctaaaaatcctctgggatccacctgttcattccgttctcccccaaacttctgactaccactgatctttttcctgttttgatagttttgcgcttcccagaatatcatatagttggaaccatacagtatgtggccttttcagtttgacttctttcacttaccaatatgcacttaaggttcttccatgtctttccatggcttgatagctcatttctttgcagaactgagtaatatttcattgtttggatgagccatagtttatccactcagctactgaagggtgtcttggtgcttccaagttttggcaattatgaatagagatgctataaacacctgtgtgtgggttttttgtggacttaagttttcaattgatttgtgtacctaccaaggagtgtgattactggattgtatggtaagaatatgtttagttttataagaaatggccacactgtcttccaaagtggctgtaccattcatcagcaacgaatgagagtttctgttgctccacatcctcatcagcatttggtggtgttagtgttttagattttagccattctatttgtagtggtatcttcttgttttagtttgcagtgctctcgtgacatatgatgttgaagatcttttcacatgttcacatgccatctatatatcttcttggatgaagtgtctattcagatattttgctcatttttaaaacagggttattcactttcttattattgagttttaagcgttctttgtatattttggataacagtcctttatcacagtagtccctgacctttttggcaccagggaccagtttcatggaagacagtttttccatggactggggtgggcaggaatggtttcaggtgaaactggtccacctcagatcatcaggtattagattctcatacggagtgtgcaacctagatcccttgcgtgcacagttcacaatagggtttgtggtcctatgagaatctaatgcagccactgatctgacaggaggtggagctcaggctataatgcttgcccatcagcagttcacctgctgtgcagcctgattcctcccaggccatggactggtactggtctggacctggaggttgggaacccctgctttatcagatgtgttttgtacagatacattctccccatctgtggcttgtttactcattctcttgacactgttttgcacagagcagactttttttattttaatgaagtccagataatcagttatttcatggttcatgtctctggtggtgtatctaaaaagtcctatccgtgctcaaggtcatctaggttttctcctatattgtcttcagggagttttatagttttgtactttacatttagatctatgttccattttgagttaatttttatgaagagaataagctctgtgtctaaattattattattattattgttattattatatttttttgcatgtggatgtccagttgctccagtcccagttgttgaaaagactgtctttgctccagtgtattaccctggtttcttcatcaaagatcagctgactacatttatgtggtcctatttctgggctctgtattctgttcctttgatctatttgtctattcttttgccagtaccgtactatcttaattactttaactttctagtaaggcttgaagtcaggtaatgtcagtccttcgactttattcttcttctttaatattgagttggctattacgggtcttttgcttctccatataaactgcagaaccagtttgccaatatccacaaaataacttgctgggattgttattgtgattgcattgaatctatagatcaagttgggatgaatgacatcttgacaatactgagtcttcctatccatgagcatgcagtgtctctccatttatttcattctttgatatctttcatcagagttttgtagttttcctatataggtttcatatatattttattaaatttatacttaagtattttacttttcggggtgctaatgtaaaacaaaacagacattatgaggaaaatgtaatgtctgtttgggggtaatgtgtttttaatattaaatttcgcttgttcattgctggtatataggaaagcattatgacttttgtatattaaccttgtatcctgcaaccttgctataatcacttactaggtccaggagattttttttttttctgttcttttggatttttttatgtagaagtcatgtcatttgcaaacaaagacagttttatttttaccttcccaatctgtatcccttttatttccttttcttgtcttgttacgttagctaagacttctagtatgatgttgaaaagcagtagtgagagaagatatccttgccttattcctaatcttagtgggaaagcttgagtttctcaccattacttatgatgttaactatatgttttgtttgtagatgttcctaagtttaggaagttttcttattttgtcaaattctttttctgcatttattgatatgatcatgtgatttttcttctttaggctatgggtgtgatggattacattaatttgttttctaatgttgaaccaaccccacataccttagctaaatctcacttggccatggtgtataattcttttcatacattatcggattcaatttgctgatattttgttaaagatttctgcatgtctgtccatgagagattggtctatagggtttattttccttgtaatgtctgttttgttttagtattagggtaattctagcctcattgaatgagttaggaagtattccctctgcttttatattctgaaagagatttcagagaattggtataatttcttccttaaatgtttggtagaattcaccagtgaacccagtccggtgccttctgtttcagaaggttattagttattgattcaatttcattaataaatgtaggcctattccatttctctatttcatcttgtatgagttttggaaaattatgtctttcaaggaatgagttcatttcacctagattatcaaatttgtgagcatagagcctattatcctttaatgtcaatgagatctgtaatgatacccctctttcatttctgaataactttcattcattcttcacgtactagacaaagtagaatttcaactaaaccaaagcaactgttcaacagatttagccttagtcctaatcagattattagtaatatctccctttagaaatatatgaaggtacttttagcagaggaaccaagcttgagctagtttgaccataatgaatttttgctgaggaagcagaagaaatgtttatattggtgagggcataatcctgtaatcttttctgtgtcctgatacctcaggaccagcgtaagcaaactccctagacaagatgtggctcatgcaagaggaaatatgcttttgaaaatgaacatgggccaagcatagtgactcatgcctgtaatcccaacactttgggaggctgaggcgggaggattgcttgagtccgggagtttgagaatagcctgggcaacataatgataccttgcctctacaaaaaaaaaaataaaaataaaaaaataaaaataaaaaaattagatgaatgtggtggtgaatgcctgtggtcccagctacttggaaggctgaagtggaaggatcacttcagcacagggaggtcgaggcttcagtgaaccataattgtgccactgcactccagcctgcatgacagagtgagaccctgcctcaaaaaataatagtaaaattaaataaaatataataaaaaacatggtctttctaataccctttgttgatctgaatttgaaaatttcctgtgagaccttctggcttattataaagaaatttgcatctaaagatacatattggaatgtttcaatctcaaagctatcaatgggaaatcaaacttcagaaacattgaatttggttttgaatatagtctaagtagacaataaaatgaaaatacatttgtttatattgaagaagcaaatgacacaccaaatagttaatttctaatagttttcatttttttctttttcttttttgtttttttttcagacagtgtctctctctgttgcccaggctggagtgcactggcatgaactcggctcactgcaacctccatctcccgagttcaagtgattctcctgcctcagtctcccaagtagctgggactacaggcctgcgccaccacgcccggctaatttttgtatttttggtagagacagggtttcaccatgtaggccaggctggtctcgaactcctgacctcaggtgatcctcccaccttgtcttcccaaagtgctgggattacaaacgtgagccaccacgcccagcctctaatcattttcttaattcatggtgcccaaaataaaagattctatattcagagaaaccatgacagaatttaaactctagccccaatacctatttaacattgggcaagtcacttaacctttttatgtctaatatttttaatctgttaggtggtaataatacttgtgtataacaacataggactgtttacaacaagcacttaataattgttagctattgttactaaattgtatttctgctgatgggttccagagtcttttcctccttcactaaacaaaactcaggatactatgtgaaggaaaagaagtgagttggtagaatttattttttaaatgcttgagtcaaaaggagagccatttgtggctgaagcatcaaaaccattttctgattttctttcattctacttgaaactacattaaaattttctccaattttccagatgattgcatgataattccttttaagaggactttaacacatgtaagaaatagagttactccctctgttaggagaaatcatggaaagatattataattaaaagatagtgaattttagcttaatttttacctttatctaaataacactcgtacacagctacagctttcagtgaagaagagatactcattcccacagctaaatcccgctcctcataggcagtgattttacctctttcacatatttcttctggcatttaccttcctatctctagaataacatacttacattaatggccaggcatagtgactcacgcctgtaatcccaacactttggtaggtcaagatgggcacatcgcttgagcccaggagtttgagatcagcctgggcaacatggtgaaacctcatcagtacagaaaatacaaaaattagccagcagtggtggtgcatgcctgtggtcccagctacttgggaggctgaagttggaggatttctcgagcccgggagtttgaggctacagtgagctgtgattgcgttacagcacgacagcctgggccacagagagagaccttgtctcaaaaataattataataataataacttatactattatttttaaaattgtattcttatccattgacttcttactgtgggagataataatttagtccttttactaccatattcccttttccaaaacacatacttctccctcccctccatcttcacaatgtagttacttgtaatttggggttaaatcagttgtctgtgcttacattgtagtaactgaaagtgctgcttaaggttgagccaagcagtgtgctatgattctgtttcctctcctgcttagctatttacttttctggagttaatttttgtcacttagtcattgctcattttgttgtcatttcttgctatgtactcatcactaattcatcctcaaactctctgacagagtaataaaaactcctctgaaagtggtcagacatatcgggcattctggtttctcaggtgatcccacctggccttcttcctcctgcattttctctaggctgctctgtatctgtagcctgggactaccttccacctctctcctgtctttcagatcctttgtttcctggtcccatcttttctcttcttggttctggtggagaactctgggaaagagtacgtgggaggtaacttttctggatgccttatcattctgaaaatgtctttactctcatacttgatggacgatttggatgagtctaaaattctaggttggaaatttttttttctcttgaattttggcaacattgttctattgattttctagcttccagtgttactgttgagaagttcagtgtcattctgattcctgatcctttctatggtactttttttttttcctgtcaggaagtacttatgatcatctctatagaaggggtattaatcttgacagtgttcctttctgtgtggtttaagaaatcctttctctcttgggttttgttactgttttataaatccttgatcttagtcattctaaggttaaagaaaaactgaggaacaactcaggaatacgtttcaagtacatgtgataaaaggcaaatatgcagaggatgataactatatgtttaaaaaatgggaaaaaagagatagtcgcaaacttcaacataggttagatcatcatttctcaaaccatattccatcacatattaagctcctcaaatattgcacactgtgcttttttctctcttttgtgtattctcgtgaacattagcctgttagtttaagaagtctcacagtaaacctatttaaccttgcttaacctagcattgcctaaatttacttgatcaccagattttttttgttttgtttttaattatttttaaaggaacattattaacatatgtataacacagttggggaaatgccagataagacatagactttcctggctgctaaagagcaattaagcattggaatgagtaaccaagaggagctgtggactctccttttccagaggcctttaaaacaggacatctgttttaggcgtagtcctgtttaaacaatagggctttgctggcggttcttcctcttcctgtcccctagtggtagtgttggaggcttttagcccaccttttatatgactgtagtactctggtgactaatgtgtacacaaattactgttatactattaatattaattatatttattgagaacttattaagtatccagccctatggtaagtgctctacatacattatctaatttaatcctcacaacaactctaggagggagacaatattaatattctacagatggagattagatatgaagagatacgaacttccagcaatagggttggattggaacctcgggcatctgacatggagctgtgcccatccttcttcaccgttaatgttcaaaacagcaaacggcacaaagcaagcaaacaacatttgtatatctgtacttactatgtaaaaacaaaccaagataatgcttactttattagactattcaagactattccctacgccttttgattaattcagagttcatgacttttgttagaaacaaattctgttacagatttagttcttcgcattttattctgtgataatttgccatccaggaaatggttccttacatgagactttttccctcataaatttgatgacattcatatacattcactaaagacccccaaaaaataaatctggatctgtgaaaagtggcaaaggttaaaagtcccattttcagcatatttacatgtagtaacaacttgataacacagcgctgagaatgccaggctcagaggagccaagctgggctcccgtccagtcagcctctagctcaccaggaaaccctgagcaggtcactttgcctcattttctttatctgtcaaatgagaactcagatgatctcaaaacagccttttctgctgtagtgtttcaggatgattcttgtctctggatgtcgctgtcatgatgggagaggaattagtaaattcccaggtcagtttacactgcagagtgatcttgatctgcatgaatcagtaaggatgggctggataaacaagttggaaccacagttatgagtaccatgacattaactgaaacaaatgagaagggattgaaaaatcggcggttaagtgtcttttaaggtcatttccaacaaaactacaaaggacctatgaaaggcttttcaggcacgtactcttgttgcctagctgaacacatttctccaataaagctttcatttgagagttactcttcatagtacatcccctgcccccctgcctgcctggcacattataggtattcatgaagatttgttggaactgttaaataattgtttaatatagaactggaagatcaggaagaaataatgtttttctaaccagtatccagtgtaaagtcacaagtgtgggctatggagcttcagaccatctggattcaatgccagttctactgcttagttactgcgtacttttaggcaagttacttacttccaggtccatgcctcagttttcccatctttaaagtaaattataaatgcacctacttcctcgggctggttgtgaggattaaatgacacaatccgggcacaatatttggcgtagtactttgcacagatttagtgtcctgttagtattagctaatgtaaatatgaagaagatgtaacattttaccagctattctaatcatagcttttcttttcttttcgtaagggacaacataaaaccccaaaggtaaagcatatatttctggtgttcaattttacaatttagcatcttttccaacccacttccatactcccaaataataatgcctatcagattaaagaagttactttatttttgcatgaaattggttgtatttttgttgcactacttcatcctttgagtattgtgaaaagtctgcgcattgactataatagcatttaaagccaagtttgaaggtctaagataatggcacacatccatgtcctttgctcacaagttctgcctaaagactttagcctgcttgaaacactctaaaggttgtgaaattaatggatataccactgatgcaacacaactcagtgtcaccagctagggagttaagacatgttcttgttactgagaagggctgttgttcatgcaaatattttgttcatttgttctttcatgggtaattgcacggagtaacaaaaaacacctcctcaacttacagcttggcagaaacagtagcttatgttttctagagacaaaattagaagcaggctttctggacccatctctaagtcaaaataaaataaaatgtctagggaaccactgtgcctcccagtaactatggtccatggaataatattgtttaggtcaaggtgtcccagagtaaaagggaagggagaagggcaggggggaaggggaaaagtgtgtttgggcaatgttttcatagagatgaagaggcaagctgtttttctttcttactttgtcctttcaacttagaaaaataagaaaaccatctaggaccacaaccttcctcttgtaatcagcaaaagagaaaaaactgaatatacatcgttaaggggaatggttatggcttaagttgtattttattgataatgttgaagattaacattttttggagagaacttaagtcttaacaaaactaaactattgagaaagtattgttatttttccatctttagtagcaaaatgaaaatttactctactcttctgcataaaatatgatcatcaattggcaagaatttggttaaaaaaaaaaactgtgcatagaatatgcacatgggaagatagaataataagatgctgtccttttactccagactggaagtctaatggtggagatagttatccagataattatatctgagttaaaggaggaggtacaaagtgctgtgggaacacagagaatggagtgtttttaagttggaggattcatagatggttttacagagaaagtagcatttggactgggttttgaaagacaaacaggcttgtggcatgaagaggtgaggagtaggaagaagatacagcagcctcagtaacctgtatgactaaaagaggcagggcatgtttaacctgggcagatagtatgatatgcccagccaccagatatgccaagaatgggagcgaggtctgggataaccagtggaaataagactgaaaaagtaagttagggctgagacatagagggccttgaatgccaagctaaaaggccagtgtttctcctgcttttccaccagtatgcccttactagtagaggacagcaaaaccataccattcttgggtggaggaagggaggaatgaataggtggagtatggggtatgtttggggcagtgaaactattctgtgtgatcctctaatgaatgcatgatattatgtctttgtcaaaacccatagaacttggctgggcatggtggctcacacccgtaatcccagcactttgggaggcagaggcaggtagatccattgaggtcaggagttcaagaccagcctggccaacatagtgaaaccccttctctactaaaaatacaaaaattagcagggcatggtggcacacgcctgtaatcccagctactcaggaggctggggcaggagaatcatatgaacctgggaggtggaggttgcagtgagccaagatcgtgccactgcattccagcctgggtgacagagcgagactccaccaaaaacaaaaacaaaacaaaacaaaaatgtagaactatgcaacagaaagagcaaaccttgatgtaaatcatggactttaggtggtaataatgtgtcaatattggttcatcagttatagcaggtatactacactgtgcaaggtgttagtaataggggaaaaccatgctttgtagagaggggacaggaggctggggaagggctattttaagagctctgtactttctgctcaatttttatgtaaccctaaaactgctctcacaaaagtaaaggctactatgaaaagcaaaacaaaacgaaaacagaaaacagcatccttttagccatgagatgtactacaagtacagagttttctaggaatttcatataatatttttaaaaattacatgaacttttccttctttccttaacacatagatggctattttcacattaaaaattttcccaaaatttccacaatgtaatacacgacccctagggatatgacttttgtaataagaagcatgactttggctgggcacagtggctcacgcctatattcccggaagtttgggaggctgagccaggaggaccacttgaacgcaggagtttgagaccagcctgggcaacacagtgagatgctgtctctttaaaagtgaggttggggaggtgggagagagagagagagagagagagaggaaagaaagcagcatggctgtgattgataggaagtcactgaaattgtatgttaaaaatgaaacaaagcaaaattaaaccagtaaaatcatgagcaaccaatttctctcccaccccagatatttgtgcatccttattttcatttcccagtattcatacaaaagcatatccactacctttaactcactttgtcagcctttattctgtatgcagaaaactttgcaatagcatagtgagaaataggtgataaacccacctttgtggatattacagtgtagacaagggaaatatactttaatatgaaaataagttatactaagaaaagtagatacagaaatgaaaattaagcctgccaaggagacagacaaagtaaatggaatgacctgggttagacaggtttggacgaattttgaaacaaaggacacagttggatgggtgccctgtccttaggagcacagacttttttctggatgtcattgagacctagaatgacctttaactatcaccagtacacattcccctttttggtgtgcagtgttgacactgaaacacagataacttaaggttgtttgggtacttatttatgtagatagacatgtgaacccatacggtacctaattagtcctcttgaaaccacaaacgcgcattcacaggaccagtcttgtttatattttcaaggctttttttttttttcttttgagttggagtttcactcttgttgcccaggctggagtgcagtggcgtgatctcagctcaccgcaacctctctctcctgggttcaagtgattctcctgcctcagcttcccgagtagctgggatcacaggcatgcaccaccatgaccagctaattttgtatttttagcagagatggggtttctccatgttgatcaggctggtctcgaactcctgacctcaggtgatccaccctctttggcctcccaaagtgctggaattacaggtgtgagccaccgcacccggcctcagggcattttttcttatgaagatgacagccgaaatcttcaatcttcaactcatgcaaaagtttgcctttggagtgaatttcttggcaatctgcttggtaagaaaaagcaagtggtgttaaagtgagagcattaaaataaaattgctccaaaaaaatgataaataaataaaagaaaagaaaaaggaaaagcaagaggcccatgcacagatacacagaggagagtggcccctcctccataagcctgtttcatcaatgagagaatcaagagagtatgtatatacagaagagagtttcagggtcagtcttgagtttgcatcttctacttcctagctagaggaccttgaacaattcactttacttctttggtcctagcttgcttatctataaagtgggaataatatttcagattatgcagaagaaaaggtaggatgtaccgggcacatgggaagtgcttgatcaataccaatttgcttccctccttccctgccccttctgctgaaacttcacagctatctcattaagtcatcaatgtatttagtatttaataaataaatatttaacgagcacctactatgagacaagccctttgttagccagtggggatatgactgcaaacaagaaagatacgcctatgatttgatgaatcctggagtttatgagcagctcatctctgtctcccgtgtgagcagtcctaaatttacacagctctccactggtgtttttgaccacagagttaacatttaaaatacctatgactgcttttttggcaccactttgaataatgaactggtgtcaggtaaacagagtccaggtacctattgcagaaagttttccagtctgcaccctcggtggctcacaagttcacatgaagtgaaccaaaagagttttgttgcacttactgtgacaataaatcatgtttagaaaaatgcatgtggcatacatgatattgggcaaatgattcatgaaacttgctattctgtggccttagaatccatgtaagcatttttcctttgtcttttatgtgttttcttgtttctatctctgttttgttttgtttttgttttggggatggtttaaaattaatgctgggctagagtctgattttgacactctcgggtgtgatcaaatgtttccacatatctctctaacctttctattctcaatgtggggaaaactttctccgctttaagaaaaggtgtatccacagaaaagattattgagtaatttttcatagtacagaagtaataattgagtgatttttccctttaaaatttttttatttttgtattattttaagaacaaaattattttaggatgcaattaaagaagaagttcatttacctaaatttaatttgccaacttttctattacacaaaagcattataaatacaagtagaatagcaaaaatttcatcctaaagagaaaaatattttgggcttctaatttcaagagagtaaaattgtcctggaaccctgtgcacactttaaaaacaatcattaacagattgcatcaaactagaaacttcttcaccacaaaggaaataatcaataaagtgaaaagccagcctacagaataggggaatctgtacatctgatatgaagttatggattgcaaatcgtacatctgatatggaattaatattccaaaatatgtaagaaactcaacaaactcaattgcaagaaaacaaataacccagttaaaaaatgataaaggaatatccatttctagaaagaagacatacaagtggccaacagatatatgaaaaggtactcaccatcactaatcatcagggaaatgcaaatcaaaaccacggtgagatatcatctcacacccattagaatggctgttatcaaaaacacagaagataagaagtgttggcaaggatgtggataagagggaacccttgtacactgttggcaggaatgtaaattggtatagtcattatggaaaacagaatggactgcctcaaaaaattaaaaatagaactagcatatgatctagcaatcctacttctgggtatatatccaagggaaatggaatcagtatgttgaagagctatctgctctcccatgttcactgcagcattattcgcaatagccaagatatgaaatcaacctaagtgtcaatggatgaatggatttttgaaaacacagtatatatctgtatatatatacacacatacatatatacacatacagatgtatatgtacacacccaatagaatattattcagccttaaaaagagaaggaaatcctgtcatttgcgacaacagagatgaacctagaggacgttatgctaagagaattaaactgggtggtatttgacacagaaagacaaataccacatgatccacgtggaatctaaaaaagtcgaactcataaaagcagtgagtaaaatggtggttgccaggagctggagggtgagagcaatggggagatatcagccagagtttcagttatgcaggataagctctggtcaccttctaaggtgatcatctgctaagtataggtcaccttcagcatggtgactatagttagtgatactgtatggtatatttgaaatttgctaagacagtagatgttaagtgttctcactacacatattcatactcaaaaaggtaactgtgaagtgatgaatatgttcattaccttgattatgataatcatttcatagtaaatacgtatattaaaacatcacattgaataccttaagtgttttgtttgttttttggttttttgggtttttttgttttgttttggtttaggttttttttgaggtggagtcttgctctgtcacccaggctggagtgcagtggtgtgatctcaccttactgctacctctgcctcccaggttcaagtgattctcctgtctcagtctcccaagtagctgggattacaggcgtgctaccacacccggccaatttttgtatttttagtagagatgaggtttcaccatgttggccaggctggtctcgaactcctgacctcaggtgatcctcctgcctccgcctcccaaagtgctgggattacaggtgtgagccactgtgcctggcctgtataccttaagtttaaaaatttttgtctattatactcaataaagctggacaaaattttaaataaataacagcagtcattaacagactcaattgatgacctaatgtagaagttaatgagagcaggcctgttggcaaaaaggcatttatatggatacactgtatgtatctgcactgtttcaggatcctctattatgatacctgggtaaagggtgacttcctttctatcataaaacagcctagacagcactaagaaggtggttatgttcttttctgttgttgtgagcgcccagatgagattactttgccaaagactcttttcatttctctttctgaaactctgtgagattgctgtgttctctaggacttaacttcacagctagtctatttttcctttcagaaatgaccatggttgacacagagatgccattctggcccaccaactttgggatcagctccgtggatctctccgtaatggaagaccactcccactcctttgatatcaagcccttcactactgttgacttctccagcatttctactccacattacgaagacattccattcacaagaacagatccagtggttgcagattacaagtatgacctgaaacttcaagagtaccaaagtatgatgtttattttcacttttcagactactaggactagaattggactcatctctcagtaaccctgtaataaataatgctccagagactagaaatctaatagagaaggcattcaccattcatttattcacccatttatccatgaaatattaggtatctatgaaatgccaggaagggagctggcacgaggtcaatcttgccttccccgccccctccttccttcctctcttctttcctttcttgcttacttccttcttagggacattttctaccttgattacactgtcagttgtatctcaggctaagagtccatcatccaaactttgaattattttggccccttataagttaataagtaacaattccaagtcactttgtattatataacttatcttcactatattactgctactacagtacattttttctagtatgtcctttcaggagtttatactgaaacctacttttaagcacaaatttgttttaacattgtagcctattgataaattttcatgccattaactaaatcaacatcaaaacatcagactcaagaaaaactagaactgcactttttgagataaaatgtatttctgtgatgctatttccttgatttttatcatgtgtgggctgacatgctggttttccaaagccaccactatgtaattggcaatcattacttgacaagtaagaacttcctgtatttctagtggcttttaaagataaataatatgcttagttatatttatctatgcggttttcagttagagcctaatatggaaatttagtagccctgagcccaactagtaaaaggtagggcttacttccataagttccgccacgctctgtcaaagattatttcacaaaccacctcctttgactgaacactaatggtaacctgggctcatatttttcatgcacctcaagctaggcataccatgaccttttcacagtggtgttccttctgtggttcttttgcaagttgtttcaaagtacttataaaatggaatatttaaataaaatgtataatttaatattgtgatgaataccaaagacagaacatttcctagcaaaataagcttccttgtctcaaatcctctatgttgtctgttacagctgtagtattgcaggctactgggggtcatagaaccacagacttaattctcattcccattttatatttacaggtgaggcttagagatgttataacttgcctgtgattacaaacctttctttttcttgccttaactccagtgttttttcatgttccactgtgcttttacactgaaacaatacaaatacagcatgaaggtgtactatggtggcttgccctgttgcctttttaggactgttttcatgggataattatcctctcacatgtctccatacacaggtgcaatcaaagtggagcctgcatctccaccttattattctgagaagactcagctctacaataagcctcatgaagagccttccaactccctcatggcaattgaatgtcgtgtctgtggagataaagcttctggatttcactatggagttcatgcttgtgaaggatgcaaggtaattaaaaaaaaagtcttcaaagaaattgttgaaactttattatttcatttcagcagaaccccttttttaggtgatacaatatatgaattttttttcttcatggaagagtatcttgctctgtcacccagaccagagtgcagtggtgctatcctagcacactgcagccttgagcttctgggctcaagtgatcctcccacctcagcctcccaaaggatgatataagatttgaaagcctaagaaagtggataaaagttgggctgctttgccccacatttgtttctccaaattgattctttgagacactgatctaatttaatccttgcatcttgcagatttttacaaaaaggtgacttctccaaggtgtcatggcaagacagtgatgacctggaaccaggatgcagatttcctgcattctctagttgtttatttatttatttatttatttattttgctataccgtgtaatattgtatagacagaagattttacagattatttatatatgcatatctttggatccctagagcaatcctataagattggacttctttatggccacattgcagatgtagaaattacaggttagtaaaacttgccaaggtcatcccttagtaagtggcagaccgcagtctagaccctgactccttaggtggtgttggctctcaaagcagtgcctcatgtttccttattccagcatcaatgtgagccacatacacggacaggtaaggaggtataacagtgtgggaaaggagatactatttatcctcatctctttcctttgtgaaaagggtattttggaaaattcagacgtttagtaatttattgcttaattattaagaaaatatgtgaatccactcatattttgatatgcagtcttttaagataattttaatatacacaatgcaaaaatagtactaatttattatatacgcattgcacagaataaactgttcataaatattcactttataaaataaatacctgcttattgggctttttattcaacgtaaagatacagaacaacagttaggaaagttttaggacatcttggttcctaaatggatggtgggccaaaaaaggaaactgatttttattgaattcttactacatgccaaatactgtatgaggtaacgttttcatacatcagtatttaaccacatcctacccaggttttctcatctataaaatgattgtggctgagtgtggtggctcacgcctctaatcccaacactttgggaggccaaggcaggaggatcacttgagcccaggggttcaagaccagtctgggcagcatagtgagaccccatccctacaaaatttttaaaaaattaaccaggcatggtggcacatgcctgtagtcctagcttcttgggaggtttaggtaagaggatcccttgatcccagaagttcaaggctgcagtgagctatgatcataccactgcactccagcctgggtcacaaaagcaagaccctaactccaaaaataaataaataaataagtaaataaataaaatgacactgaattacatgatctctaaagtcccttcaattgaaacagtttttactctaaaggcaacctaatacagtgaaaagggacaaaccagaggtcagctctgccactttccaaagtcattagccagtcacatacacattgtatccttcatcaggccccccatatgtaaaatgacttggttagattggctacacaaggtcttattcatctctaagttctgtaatttcaaaatgacactttgaaacactctggcaagagatgctttcatttaaaacactaaaacccgttcgttctgtaatttaaaccaagttaaaatatttatgaccttatatgaaatcattgtattaagtcagttatctaagatcttgatgagtagtaagaacatgtcattttattgacttagattttttattgaatgttttgtggttttattgagttttattttagatttaatgagttagagtttatttttactgagttggataccatttttgagtgagtaaactgttgctaaattctgagccatatttatctgaagaaaccattctgttttggtcatgttgataatttacaactataaataaataaaaacagcatggttggtttaaggttccacaataagttattgttttttatgggctagtaaagcacttagaaaactaaaacttttaagcaaatagttccaccataatcctattagtcacaaatttgtggaaagctaacattactgaaaacagctgaaaatggaaagacaagaacattgtcagtagttggttatagtgataaatctgagttctgagggcactaaaacttaaaagcaagcagggaagaagagtagcaaaaagagaagagagaggaggaaatccaagtgccttcaacttaggattagaaagggtagaaagcagggagggagaaaaaatacttaataaaacctgaagactctaggggagtccttaacctatcatagattaaaaagcaaacatagaagaaaactaagcgtattgtatactaacctgcagtaatttgcaaaccatccaaaatgtggattccagaattcctagactaaaatgtaaggaaggttttactcccttggaaagggaaaatagacatctacacgttttaaaggtaagaataagaaaaatattattcttggaaaatttaaacatttagtaatatactacttaatataaagaaaatatgtgaatccacttatattttgatatgcagtctttcaaaataattttaatatactcaatgaataaaatagcatttattgtatactgattgcacagaataaatttttcataaatatttaccttataaaataaaccctgcttcggctggggtttttattcggcgtaaagatatagaacagcagttaggaaagaattaggacatcttgattcctaaatggatgatgggtcgaaaaaggaaactttttttgaattcttattctgatttttattgaattcttagtatgtaccagatactatgtgaggtacatttgcatatatcattatttaaccacatcctactcaggttttctcatctagaaaatgattcagatgatattggtaggatgtggttacataatgaaacattatcatttggcttcttcaagtatacatcagcagttcccaaagtgtggtctggggcttggaccctttcaaggcatccatgaagttgaaactatattcataataatgatttttattacttttttcactttcattctctcaggagtgtatgtggagtgttctggaagctacatgatgtaggatgatgacatagctctggtagctaatggaatgtttgcttatgtgttcttgtatataataatttctcagttgtaatttctagtgtgataaatgtcagtaaagatagcccacataaacaaaatctctttggggtcttctataattttaaaaagagtaaagggatcttgcaaccataaagccttcagtctcattctgaagaaatgcagttactcattctttgctactttgaaactagacaaaattgctgccacattctgaatactgctgcattagaccagtggctgtcagtaaagacatctccttagcttataaccaatacgcaataaaaagccaggaaaatggaattagcaaatgtgtttaactcatctgcatgtattttctgagaggtgttttggaagcttcacatttgctgttgtagtaaaatgtgggttatattcataattaaaatacagttgaccacaaagctgcaggcttatctatggattgaaaagaataaacacagcataaaacaacttttggtagatcttcctaaacaattttacaatgtaaatggaacaggtttatattagtgattcttgccaaaaattcagtcagacagatgagaatgagtagattgggtttgaattaaggtgaaatagttacagattcttgggtatgttaatattgcaaacttatgtaaaataaaacctttagcaactgaaagatatatataatttagagcttggaaagctatcatttatttgttgtttacatgttggagatatatttttttctttggtaagttccatcctattttttatctttagtgaaagatcattttggaaccatagccgtacctaaagatataagtaaatacagtctaccatacaatacaatgtaatctaagtttgtatttctgtatacaaaagaatgccgtatgcttgttagccacttgtatgtctattcatccctacttcagaaagagttttaattcttctcacctgccagtcgtagcttattaatccaacttccaggggccagactgcttcatgggaaagccaactgcaagcccagcacagggctgttaatttcattgtaaaatcaacaacaccattctgaggtctcattgtccctgatgttttgttaaaattaaagcaattaaggagagatcaaagaaaatttttcaaatgatatgaaaaatttgtctgttactttctagcagacaaatgtgcagacattagaataaatatatacacaaaacaattttctcagatggtgactgatgcatctctaacacaccacatcacagacttcctgatcatcagaagagtaagttgttgaaaatacattgttctatggactctaaaataataaaaaagtgttattagagtgtttcttcatcagtaatatgaagaaaatttggagaagccagccttgttctgtaaatcgataaataattttacagaaaagcactcgataatatccttacatcttcctctctagattccttgagtcacataacaagaaaacacttggttatcatgaactcggtgtaaaaaaagtaaaagcaagttccaagatgcatgctaggatctgtgtattcagttcaagattttatttacatatacagtgtataatgttcagaatgattattcattgaaagaccttggatcatcacaaaaaatgtgatacacttttgaaagtcatcagctgagtcatgtcagaaatttccattataagagttaaacttaattctctttttttttttttgaacatgtgtcaaagatttatttaaaacccattaacgagggaaaagcaggatggtaaatctagttcaaagaagaacttgaaggaccaagaatatatagtcactgaaagaaagaatcctgagataagattcagaatggttaatgttctacagggcaataaaaccataaccttgaggttatcttttcttttttttattattcttatactttaagttctagggtacatgtgcacaacgtgcaggtttgttacatagttacacatgtgtcatgttgatttgctgaacccatcaacttgtcatttacattaggtatttctcctaatgctatccctcccccaaccctccaccccctgataggccccactgtgtgatgttccccgccctgtgtccatgcattctcattgttccactcccacctgtgagtgagaacgtgcagtgtttggttttctgtccttgtgatagtttgcttaggatgatggtttccagctccatccatgcccctgcaaaggatatggactcatccttttttatggctgcatagtattctatgatgtatatgtgccacattttcttaatccagtcaatcattgatggacatttgggtcagttccaagtctctgctgttgtgaatagtgccataataaacatatgtgtgcatgtgtctttatagtagcatgacttataatcctttggatatatacccagtaatgggattgctgggtcaaatggtatttctagttctagatccttgaggaattgccacactgtcttccacaatggttgaactaatttacacttccaccaacagtgtaaaagcattcctatttctccacatcctctccagcgtctgtttttttcctgactttttaatgatcatcattctaagtggcgtgagatggtatctcattatggttttgatttgcatttctctgatggccagtgatgatgagcattttttcatatgtctgttggctgcataaatgtcttcttttgagaagtgtctgttcatatcccttacccactttttgatggggttgtttttttcttgtaaatttgtttaagttctttgtagattctggatattagccctttgtcagatgggtagattgcaaaaattttctcccattctgtaggttgcctgttcactctgatgatagtttcttttgctgtgcagaaactctttagtttaattagatcccatttgtcaattttggcttttgttgctattgcttttggtgttttagacatgaagtctttgcccatgcctatatcctgaatggtattgcctaggttttcttctagggtttttgtggtgttaggtcttacatttaagtctttaatccatcttgagttaattttgtatatggtgtaaggaagggatcaataattctcttatcaaaaaaaccttcctctcctagccatgccaaataactgagcgctctgtgagccatccagctgtcagctagccaagtagcattttcacccactaatattagtctttaaaaagcaagaatcaaaagagaagtcaaggaatatcataaaatatctatgatcacaatggcaaacatcaggattttcaccaacatttatcaatgagaacagttctatacattagcattctgttcatctgtgaaaaaaaaactttttgatatctgaaggtcctcagaaccctttgagaattaaagagacttcaactgccagcaaattctacatcgggcatattctttaagacattgctgatctcacaagaggtagtgaaaactctccaaaacaacatcaatgaaacaaaatgaaacaaacataccctcagttccaagctgtgagctgcaggcacacttagcaggtcagggttttccccatgatagatgcccagagaggtacagtggtgagcattgccccaaaggcagatggctgtagcagttttctgagcaataagtgagaaggagctaagtgtagggcttctgaattaagccaggattctcaatagtgtctgaaatagtcataagtcagtaacacccctggctactgaattcctaattcagactttgtaggagtcccccagtttaaggtcaagaaactagttccaaataatatcagcaagcatgtgagaagctaaccatcttgaatgacattcatcatcaacaagaaaactgatacagactccctgctcttcccctacctggggaaagcagaaattgggattgcctgatacagaatataaaaaagctattatgaattatttaaaggaagagggcataggcttgcaacaataaactattaggaataaccaggatgatttgaaaaccaagtgaaaaaaaggtgaagcttctaaaagttaaaagtataattattgaaataaaaattcagtggaagggttagatagcttactggacacagcagaagaaaaacctgaaactgaaagagatatgcaaagaaattaccagaatgaaagcaacagtgtcttaaagaatatgccctatccaggatctgctggaatttgaaggcttttagttcttgaaggattcataggatctttgaatattaaagaggtatgtcttcttcactgatcaatggaagagtaaagtgcagaactgttctcactaatgaactttagtgagaaatgtttgtttttacttttgccagtgtaattatatattttcatgttattttgcttctgttctgatttttactttggcaatcaatattagtgagtaagtagtgagaagaagatggaaaataaaaaagaggcattcagaaatgtgaaggctagaataagaaagtctagtacttatctaactggagtccagtactgatgaacatgtgaagccgtaatgcataaacaacatatccaagaaggtaaatgaaaagaaattcatgcccaaacacactgcggttaaactgccgaatactaaagacaaatagagagtataaaagcaaccaaagagaaaaggtagatcaccttagaagtaaattgacaagagacttctcaacagcaaaatggaagcagaaggataatggaattcaaagtgttaagagaaaatgactgagtacttggtaatctctcaagaatgagagtgagccaggcgtagtggcacatgtgtgtaatctcaggcctttgggaggccaaggtgggtggatcacttgaggctgggagttcaagaccagcctggccaacttggtgaaaacccatctctaccaaaaatacaacaaaaaaaaagagccaggtatggtggtgcatgcctataatcccagctacccagaaggctgaggcccaagaatcgcttgaacctgagaggtgaaggttgcagtgagccgagatagcaccactgcactccagcctgagcaagagagcgagactctgtctcaaaacaaaaaacaaacaaaacaaaaagagtgaaatgaaatatctattggttgaataaacaaaaatactgaaaaagtacatttcaaggatagtaagccagagaagatatttgaacatctgtaacagacaacagattaatatctagcatattttttaaaaaagtctaaaattcagttttaaggaaaagacagttagaaactgggaagtgaaaagccagggacatacaaatcaagatttaaattcaattttatacatttcagattgtcaaaattaagaagtctgacagcaccaaatgtggaagagactacaattttcataaagcgcttgtggggagtgtacattggtagccactttggaaaacaatttggcattatcttgtaaaattttaatactcacacattgtacaacccagaaatgccacttaaacatatttacaggaatatttagagaaactcttctcataatagcaaaaaattgatatttcaaacgtccatctgcatacaaataggttaataaattatagtatagtcatacaatggaatactatataattatgaaaatgagtaaatcatagtctttcactaacaagaacttaaatgttagaaacctcataccaaattttaatagtgtcccagaaaactacatatagtataataccatttaataaagcctccaaacaagcaaaattaaatagtatattattttgttttacatagtatgtgataaagctgtattttcttcctttttttttttttttttttttgagacaatgtctcactctgtcacccagactggagtgcagtggtgcaatcataacttggcttactgcagttagacctcctgggctcatgtgatccttccatctcagccgccagagtagtagctgtgactacaggcgcatgccaccacacctgcctaaattttttgtatttttttatagagacaaggtttcaccttgttgcccaggctagtctcgaactcctggactcaagcgatcaatccgcctcagtctgtcaaagtgttgggattacaggtgtgagccaccacacccagcctatattttcttaaagatcaaggaaatgacaaacccaaaattgagaataatgattactttgtcaaacctatcgcctttgtaacatctcagtcacaattgggaatcacaaactaccagagatggaagtgctttctcattttatagttgaaaaaggtgaggcccagaaaggaagttacgtgacatctgtattaattccacaaattttaatttagcactatcataggcatttggattccatccaggggtataagagactattcctgccgctgaggaacttataattttaattgagcagtgagggaggggcagaaaataaacactaaaacaataataagtaaattctgtggtgtgttagaaagtcataagtgctattggaaaggagaaaaactggagcagagtaaagaagatcaagagttccagaagagaggtggggcagggacaggccacagtattaaataggttggcttagccccattgagaaggtgagatgcaaaacttgaaggcgatgaaggaaataggcaagtgtgtatttagagaaagctttcttcttgaggaaagaaagaagtcaagagtgatttcaaggattttggcttgagaaactggaaggatggcgttgcgtctgctgagatggagaaagccgcaagtgaagtgagtttgtaggggagggtcaggacttcaatttggacaggctggcttagagatggctattaattatttaaatgaagctgtcaagtaatcagaacatactcatccagagttctaaatggacgtttggagaaagtcaaaatgcatgtcaatgaccaaagcaatactaatgcagtgctttttgcaccaaacagggccagatacatttgaaagaattagcaattaagttttatgaagatgaacacaatagaaatgaataggaatatgatgaacccaaaaaatggagtcagaaaacacgtccagttcgatttttttcagctctttccaaagatgtaaatatagcagaatattcagttggcctcaaattgacatatttgccattttgagatagcagtcgattttgtgaggatttatctgattacttctcatgttattcccatagtctctttctgtctgtaagccacaacaatgatggggcacactttaaacaacataaataagtgaaacaaattctgcaggaaattatgcaacatagagaattccaaaaaaattatccacatgtggatttttattggccctgatcatgttttagaatgaaatgattataactttgccaggctgcttagcacaattacaaaggctggggcatgctgttggaatgatttgcagagagacttaactgattacacggtgttttatttgcattacattaaatccagagcacttcttagagcatgccgaaaaccaaatgtagagccaagatccaatgaaagccgcagctggatgtggtcagtgtctaagagctaaaaaagggacctggagatcctctggttctttattttatagcagagaacatttagttccagagaggttaagtgacttgtctaaagtcaccagtgacagaatcgtgtcaagaacctgccttttctgattcccaggccagtatacctttcgctgtaggttgctgcttccatgtgtcataaagacttaaaatttgcttcttttttatccctttgcagggtttcttccggagaacaatcagattgaagcttatctatgacagatgtgatcttaactgtcggatccacaaaaaaagtagaaataaatgtcagtactgtcggtttcagaaatgccttgcagtggggatgtctcataatggtaagtaaacagtcatcaccatatactttattattctcattatagctgccagaccagtggacactaaagccattgccaaaaatgtgtacagtttttccaccaaatgccagaatttagaatattgcatggcgataaaacatttctcttttaggtcagtgtttttaaagttttattatagaacctttctctctgtggttgggcatctgccatgaggagaaaagagacttgaaaaatctgggggattatgggaaaaactttagtgttagaacaaatataatgatcatcatgattaatttttatattgcctcatgcattaaaaacagaattaaaatttacttttgtgtatcagtagtgtcgttctgctttaaatgtaagaaaatcctgaagatgtctgggtctgaaactttaaatggcatatgagaatttagattcatttaattttttttttttttttttttttttgctgtttattatgcaaagacgagtattcgtttccttcacttcaaggaacgtccatgagttgtggaaagggtaaaacaaattatttttatagttctgcaaaacttcaaagccatagaaacataagagaataaaactttctacttttgaaacctgtgtctaaagtcaagcttatgactttgggtgtcaacttaagggaaatgatgtagaagacctgagaaaagacccatgttttcatgatctgtggaactaactcagtaaggtcctggaagacaaacgtgtttgaaaaaataattcttggtcactatttggttctgattggttgcctggctgacaaaataaattttaggtgtaacttgatagtattatatgtgtctagtattaatcagttattttcaatgcactcaaggaataaaaaatgccaacatgatcaaattaaatttgaagtttcatttcatcagctatcctattttttctttcttttgttttcatctctctcaaaactgatctagtaagaaggcagtcttcatctatatgtactctaaagcatctgagaaaattaaatttttgctctatcatgcagatacttggttttcacagtggaaaccatcaagatatttgagagtcactcattgattaataacctaccctttaaaaatagttcacaaaattctatctgtatgattactaatgggtcagttcctctaaaggcaagaatgtattttgaatagagctatcagcagtactgaacaggatggaaatttggtccaactttcctcaacaattgactacatctgctgtatacaactgtagtcatggattgcaaaataatttgctggttcagttccatcagtttcctttttatttcagacctcataaaacataagggcaagcttccaagtcaagggttgtattttaggtgatgcaatcaagttgcaataaacttatttcatcttcatgaagaaatcattgactttgaggtcattatcactgagacagcctaggaaagcatgccagttccgcttttaacactaatttttgcctattaaaaaattatcacttcacacattcatgtaaaatataattcctgttacttacaggcagtgcatacattgatgtaaaatatatttcctgttgcttacaggcattgcatacgtttacttaaaatcaatctgcaattgcttattgtttataggcaaatattatttaaaccccaacctatgtagtatggatggtataattttctcctcccataaatgtcaaagaaagctatcataaacttgataggtcatattttgacttcatatgacaatttattttatttctagagagggtcaatcttgatagggagtgtttgttcagttctagcaaaagcaagaaaatatatgaattaagtgtcatgacatcagagacttaggcagttcaacacttaaaaaattgcaaacataactaagaaaacctcagaggtttttatgggagtttgtttgctgcacagaaaataaacatcagactaacaacaaggttttgattagttttgcctgttagctgtatgaagaaaacatttctaaatacaaagttttctaggaagttgagtcactatttaaaatccattgctttgaccaatgtgaagccaacagggttttcattcatatagaatgcctttttatcaaaagaggctctgagtgttataccaaaatcagcacccagctgttttcagtatgcgcaagaaaacatgaacgtcccccaaagcaaatgtactccattccgtgttaaccttatttctgctccctggtctctgattagtctggttgatgaatgtagcttcccctttggccatgcactcacagctttgaaggaggcttctgaaggaactggtagggaaccctaggggctcttgctaatgttgttggatagtcactgaaatcagtgatcaccatgtcctttcactttgaaaattctatgattctgtataatcaaacaacctaactcactggatttttcacttttcaaccagctattccgtgtcttacagtgctctggtcttcacagataggtaggcacctggcatgtcagttgcctgaatttgaaagttttcacctgtatgttttggtacgataaaaataaaaatgtaatttatatatctgaatcaggtctgtatgttatgatcaattgctcagcaatttcgggcagttggtttgatggttatgtagtaatgtagcctgagagcagaaatacagagcctctgggctagagaaagtataaatggcatcctaggctatgtagggttacagctcttcagaaggaactttcattttcattgtgacacatcgtctacatgttgtagaagaacatagtttcagaattcttccagttagaaacatagtttctcaaatattcactttcagcattgggtagaaaaagtacccaggtgatggactgattgatatgcttcagaaatatgttttttcctgcaagtaatgaaaataaacacacgttcttaattattttggtcatttaacaacccatcatttctggaccatgggttaattccaccgattgctcagaagccttcctgagtcatctcaagcacaatcaattcactactgtgtctagacactgcccttagaggaaagctcaaaatgaaaatgaagcagaaatacagacccacttcctaggccactcagcggtgtatgtaacttaccaagtgatcattgcatcaactactctttgttagtgaagctggtgtctgcagaatcttgataaaaagactcatggataatgttgcttctttagtcaaatgggctcttgcatgcatttttatagattttcaaagtagtcatttttgttttaaaatcctgctgccaagtcctttatagtaattgcattttaaaaatatgtcttctttattttttattattatttttttttgagatggagtctcgctctgtcgcccagtctggagtacaatggtacaatcttggctcactgcaacctccgcctcccaggttcaagcaattctcctgccttagcctcctgagtagctgggattacaggtgcccgaaaccatacccagctgatttttgtatttttagtaaagatggggcttcaccatgttggccaagatggtctcgaactcctgacctcaggtgatccacccacctcagcctcccaaagtgctaggattacaggcgtgagctaccacactggccttgtcctctttatttttaataaaattatttagtcattaagaattttggcttgtgggccaggcatggtggctcatgcctataatcccagcactttgggaggccgaggtcagaggaccacttgagctgaggagttcgagaccagcctgggaaacatgacaagactccatatctactaaaactacaaaaaattagtcgggcgtgatggcttgtgcctgtggtttcagctactcgggagtctggagtgggaagatcgctttagcccagggggtggaagttgcagtgagccatgattgcaccactgcactccagtctgggtaacagagcaagacccagtctcaaaaaaaaaaaaaaaaaaagaattgtgactagtgaataattcatattcagagctctttttaatgtatgaactaaataataaaatagtaagtttaggctaagtgccctttttatttttaaaattttctgtatttattattactatttttagagatggagtctccctgtgttgcttaggctgggctcacctcagcatctggagttgctgaaactataggcatgtgccactgcacctgacctatttaagaaaataatctagagaagaattgacatgttatttatgaatcattcagttaggttttctctataacattgagatttggttaaaaatatgtttttcataaatttaaaaactattgaaatcttagctttgctgactaggatgtcttattatataaatgagagagagtttgtaattttttaaaaaaaactgacaactttcaaaatagtttctcagtggcttcataaaaatccagaaaaaaagatttcacaaatttttgtgacactcaacatttttaaggtagttctctcagtgccttgcaaacagcagctctagtgtatattgagaaaaggaaaaattctgaatggcaaatactagatttcaactttaacctattcctttttattattattattattattattattattattattattattattattattgagacaaagtctcgctctgttgcccaggctggagtgcagtggcgcgatctaggctcactgcaagctccacctcccggattcacaccattctcctgcctcaccctcctgagtagctgggactacaggcgcctgccaccatgcccggctaattttttgtatttttagtagagacggggtttcaccgtgttagccaggatggtcgcgatctcctgacctcatgatctgcccacctcagcctctcaaagtgctgggattacaggcgtgagccaccgcgtctggctaacctattccttttttttctttagtcttcttggttgtgtaaagaaaaattacccaaatcttaactttcagaaaaggtaacaaactcctaatgcatgtggcagtacatgtttgctccagctgccctgtccctctaccctgcgtggactccagaaccgcccatgttggagcccacctcctctccccacccctgcccactttccactcacacctcaggcaaaccctgcattttgctgttcctggaaaatggcttatgcttggatacctctgggcctctgttgatgcgtctgtctgttccttgtggaaattcttcctgacattcaaggctgcattcaaatgccttccttcccatgagacttttctgattccctgctcttccttttctatgtgtttcataccttcctgtgatatcacattctgccttaaaaagcaagagagtgatcagatacatattaccaaaaaaaaaaaaataccgatagcagtaaaaatgatagagaaaagactggaattgggaaatccatctgaagaccaatgcaatattaggaaataagacattgagaagggtgagaagaaaggaaattgagagaaatatcagagcagtgaccaatgaataaaagcgcctgaagggagagaagttgtcaaagattatttaggatatctaatttgggtgatagaatgaattaaccaagagaggaacacaggaataagagccagtttggaggagaaaattttaaattcagttttatattgtgttagagatgcctatagagtatccagcaactacgtatagaggaatataggaggatgtgaaaaataaggctccaaatttcagtgaagagagagcaggaatcatcagcacccattgtaggttagagaggtcacactagggaccacagaatacaagctaagggagaggcaccatcagagagatctggagagcagctggcagaatgttagaggacccagaacagcaggaaccaggacaagaaattttggaaataagagggcggagatggtcaccagaattaaaggctgggagaatactgaagagctcaagtctattgagaacttagaagaggccattagttctggccgagagaaaagcattcaggatttttacaaagttttggtaaatcccagtgagcgcaaagctagactgcagtagatcgagaagtgaatagaaagtgacaaacacagacggagtgaaaacaactctttcagtaagttcagtggtggaggaaagatagcttaaagaggaggtaatagtagagtcagaaccttcaacctgggcagaaaggccagagccagtacagagaggcacactagagaaagactcatctgtgtaatatacccagtctcccctaccagacatgtcctttccatcctttcccccagccccatctgtgcagcacagtgttgcatcaacgaagtgttcagtgaatgaattaaaggttgtcaggaagacttcagggaatcagagattgagttagaaggtgagctggtggtgttttgctcatcttcatttttgaaagaaacctaagaaaatgtttaaatgtcctctacaaatagtgtgaaaaatggtacctctgcataaaaataatttaatattagtgctaaagttgctccttgttttcctttagaggaactacaaaaggatagttattagattgccaaatcctgcagaacctccagcaggcacaagttggtttttctccctcaagaaagagaagtgagccaagcgtggtggtgcatgcctgtggtcccagctactcaggaggctgaggtaggagcttcccttgaacccaggtgttcaaggctgcagtgagccaagatcacactactgtgctccagcccaggcaagagaatgagaccctgtctctttaaaaaaaaaagaaagaaagaaagaaaagaaagagaaaggatggaagggaggaaggaaggaaggaagggagggagggagggaaaaaaggaaaaaggaagggaggaaaagaaggaaggaaagaaagagaggtgagccaggtgtagtggctcatacctgcaattccagcactttgggagactgaggcaggaggatcacttgggccaggagttttggcgagatcccatgtctaccaaaaaaaaaaaaaaaaaaaattagctgggcatggtcatgtgtgcctgtgggcccagccacttgggaggctgaggcagaatgattgcttgagcccagaaggttgcagtgagctacgatcatgccactacactcccacctgcgtgatcgagaaagaccctgtctctaaaaaaaaaaaaaaaattttaaagagagatgggaaaacaacttattggcaatagcacatgttcttgtttgtatgcaacaaacatataaaaagtagaaaaattgaccataagacatagccttactatttttcaaaagcctgataatgattgcaaattcatcccttagatgtggaaagacaaaaataagacttgtcttatttcattctgttattttctattgatttattattttgaaaacctgctttaattaaccttagtaattaagtagcatttgtctttaatgcttctacaattaggtagatgttttaaaaacatgccgattaattgtttcttagcgttatacccagatccaaaaagcaggacatctaactattccatgtgcttggtgtttgtgtgttcagcaatatcagtactaaatacacaatacaaatctataacatgctagtagtagctacattcagctcaatagaagtgtgttgtataaaggaatgccaatatgctttcccagaagttaatgagtctctatcaaacccagtcttcctgaagggagcctaccagctctgatatggataattttttttaccaagataccagatttctctgtaggtgatgaattattccaaataggaaactgcgtgccagtgttctggaagttgctctgtgtgacaggtgccagatctgtagaacagacagaatgtaattttttttgagcctcaaaaactagacaaatactgcttttaaaaagagagcagagcattttcttgagtactatgtagacatttgtagaactttagagctaaatttagagctagaggaaggaaactttagaatcttcttttctaagttcctcattcagtaaataaatcagttgaagaccagagaagttcagtaattttcttaaagccacatagctagtttgtcactgagctgaaactagaaattaagcttcctgactgcattcagtgcagtattcattcccttgctttccagagaggccaaaagttcttgctcagtgactcacagtaagacatgaagcattttccttttaagattaatcagcagtggtagaagatttggaaaaatacacttgtatatgagtacactcagcctttatagttctgacccccaatgcagaatgttcatcttctatttctaaggtctgacttcagtctttcaggaaacacctcccaacctccttcgctttcctcctcttggttgtcagattctccacatgaagggtagaacctaaggctcaagaattacttaactaaaaaacaccatctcacaaacaatttaaagatggaaagatagaaatagagataggcagacagatggacacatagattaggttttcagattctgttctttctctgtgggagaggtcagcgtgccatgactaccagcctggtctagaacccacagcagccatagttaccaagaccacagcaataaaagctgtgtttgttaagcattgccatgcacctagcactgtgttaaacacttcctgtgcctcctctcatcacctcacgtgaggtagataggtacaattatgtgggactcaaaagcaacgaaataataaaactggcttttttcccccttaaaaaaggtatgcgtgcctcagctgaaagacagaaaaaaaaaaaaaaagtaggcaaataaaaatccttgttttctgtacaatttcagatttgtgtatgttttatgggaatttagtctcaccaaatgggatcgatttttcattccttttatgaacttctggtgtataaaaatgttaaaatcacctatataattggttgcactggtagttaaatggaacctaatttgtagcatgggcatttaacaatacagataatttattcattagagttagcctttggggggaacttcaacttacaaaaatacgttttagtgagattatagcagagggatctcactttaatatatcctaattctaaaatggtttttcggggtattttttggttatatttgttaggtgatagaaaagcaagactagtaaatgtagtaagtggctatctttggctgtttgtccatttaaattaacttttttgattacccattaggaaaaaattgcttttctaggtgtgtaaagttttgcatatgattatagcctcttacctgtaaaaactgaatcagagcttagaaccatgcctggcgcacaatagtcattcaacaattattccttgaataaagagacagtattgtgtggtctgtgaaataacaaaagttcaggagcaacagacacttggtgattctagtcacctctattttgttataggataactggttttctctgagttttacaccagaatgccttcttcttttaatacgccttcttacttagtgcttttctcatgatcattttcccaaacttcctaatggacatagtgtctcattttctgtctgtttttaaacctgatactttggagtttaatccatcaaacatttattgttaacctactatgtgtattttgttacacctaggaacaaagatgagaaaacatgttactcatataatttatattcgagtagaataactgatataaaccaacatcatagtatagtaacagtttaatacatgagctaatgtatgcatacaacaggagcccagcatttaggaagctttttataaactgtcccaaaccccaggttttttatatactcctaattgagtggatggatggcccatcaaaatgtcccgtggaagacatataatgtcagaagttaccgagtgactctgataggctctgcctcccctaccctccgcactcctcaattaggaactactggtgaacaagaaatgaatgtagtacagccatccctccttattccctgggattggctccaggacccactcagataccaaaattcctaaatgtgcaagtctctgatataaaatggcatagtatttgcatgtaacctacacataccctcctgtatactttagatcatctctagatgacttataatatctaatacagtataaatactgtataaatagttcctatggccaggtgtcatggctcatgcctgtaatcccatctctttgggaggtggaggcaggaggatcccttgagcccaggagttcgagaccagcctgggcaacatggtgaaaccctgtctctacaaaaaaattaaaaattagccaggcgtggtggcacacacctgtagtcctagctacgcaggaggctgaggtgggagaatcgcttgaacccaggaggtcgaggctgcagtgagccatgattgtgccactgcactccagcctgggtgacagaacgagaccctgtctcaaaaaaaaaaaaaaagttgttatactgtatttttttatttgtcttattttttatcattgttttatttatttattttagagacagagtcttgctgtcacccaggctaaagtgtagtggctctatcacgactcactgcagcctcaaactcctgggctcaagggatccttccacctcagcctcctgagtagctgggattagaggcgcacaccaccacgcccagctatttatttttatttttatttttgtacagacagggtctctctatgttgcccaggctgctctcaaattcctggcctcaggcaatcctttcactttggcctcccaaagttctgggattacaggtgtgagctaccacacccagcccatattattttttattggttcttttttccaaatattttcaatccacagttggttgaatctgcagatgtggaacctgcgggtatggagggccaactgcataaggaattctatctgagcaaagtggtcaggaggtcacagaggattttgaaggaatatgctatctggggttttctttccattgtatttcaaaatacagtagacaaggacttaatatgtgccagaaattgtactaagtgctgaggatacaataatgaacaagattcctgcctttgtggagattatatggcaagggaggaaagaaaacattatagattaattcctgtgatcagtgctgtgagataaggtcatatcctgagggacccagacaagcctagcaccaggggctggggtcaccagtagataaaaatatgaacaaccataccccagccccatggaacaacacagaaagaaaatggggaagagtgagtagggaacaggatttttgaccaaaacctcctagtttaaaggtttctatatgaagaggccatgtaccaaggatatattcactaaaagtatctaaatataggctaattcaatttaaaggaatcccaactgagaggtaagattttcttcccctctaacacccaagtctggtctctaaggaggcccctaccaaacaatagttgtattagtcagcgataaaatttatttagggtcaatggaaatgaatttatgaatttgagactcaagggtacatgtcagtttcttcttgggaaaatccaaggtaatattcacagagtactcagatgggaaagttgtcgtgtgctgtcatgtctcatggtagaaatgctacccttagcataataacatataaaataactatctctggctgggcacagtggctcatgcctgtaaccccaacactttgggaggctgaggtgggtgaatcacttgaggtcaggagtttgagacccacctggacaacgtggtaaaaccctgtctctactaaaaatacaaaactgagccaggcatggtggcccaccccttgtaatcccagctactcagaggctgaggcaggagaatcgcttgaacccaggaggtggaggttgcagtgagctgggattgtgccactgcactccagcctgggcgacagagcaagactccatctcaaaatataaaataaaataaaataaaaatctctttgttctgggattcagcagagacagagtcttgctagagacataaacaaatatgacagtctctgcgctcgaggagcatatagtctagtgaagccgatcaccataaaaacgcatggctgtgataccacatcgtgagtgtaagaacagagctatgtatgcatggggaacagtggacatgatggccaggtacccttattatgggaaacatagaacccaaagtgtgttcccaaaggaacatgattcaaaataatattttgctgaacatattggtaagaaggaaagaaaacatatctgagttgaaaagttacagtttattttttccccaaactagtccccactaacccctcttacattttccttgttgcttttctttctttcattatcttctttgacacttcctcaccctacaggcagccagtttgtctttctgacaaacatcattaagtggtaactctggagagtcgggagataactatggcttctctccgctacatgtaaaagtgctctctggactagtaaaatgtgataaagcaccatccatatttctttttaacagagacaaacaaatcttataaactccctgagaacaaagcctatgtctgtacaactttgaattctgcacagtttcgtattttaattcgtgaaacgtgttgatccttctagtgcctgaccttaggtcaagtgctggggatacaaagaaggtgacctttgaattgggtcttgagggatgagtaggagttggttctcaattatttcacgtttaagtcgacatacttccctccctttgctaaactcgaattctttcactttctcagcaggagtatgcattaacttttaaaaatgaaagttaacggtttaatttttactgatggtctgtgctacttttgtgaaataaaaacatgagcaaagtggtagacagaaaccaggactcaagagcagtggaggaggagggcttctactgtgtgggaacgagggctgggagagcacagtgtgtgttcagagcagtagtaatccaatgattcatcctgtcattcctcttcctctatagccatcaggtttgggcggatgccacaggccgagaaggagaagctgttggcggagatctccagtgatatcgaccagctgaatccagagtccgctgacctccgggccctggcaaaacatttgtatgactcatacataaagtccttcccgctgaccaaagcaaaggcgagggcgatcttgacaggaaagacaacagacaaatcagttagttctcttctgctgtcttcattgggggaggcgggaagttgttttgggtttttgtttctttgagtaaatggtttactgcgctacaaatgcacacacagaatattgttcaactgttggctgttaacatattgcaggctgagtctgaaacgcaggaagtgttttcagatagcacaagtcaacattattttgaaaagggagaaaagtccataaagtttttgagaatagtgtaacaatgtattggtcatcctaactttaatgaatgaacttaagccccctgagcctatcaccctcttttaggatccatctcctttctcggcatcaaaataactggccacagcaatattcattcaagcagccttgctttcctctgggaagaacccgacctaggtttagaaaaggtattgaatcccactatttcacctttcaggagaactaccagagttacctctttttttttttttttttttttttttgagatgtcgtctcactttgtcgcccaggctggagtgcagtggcacaatctcggctcaccgcaacctccgcctcccaggttaaagcgattatcatgcctcagcatcccgagtagctgggattacaggtgtgcacgaccatgcctggctaatctttgtatttttagtagagacggggtttcaccttgttgatcaggctggtctagagttacctcttaagaagttcaacatgaggcataaaaatagattctagatattatgttacctttctttccttgtagcattcttgattattccggggcaactagaagctctatccttttattacatatgtgaattttatcttctgcaaggctctgagctgcctggactacttcagtggactctccaacatctgttcactcattgagcagcactgtttagaaaacccagaatgggttgtaattgttactgagttaggttttccaagcagcagagctcttctctgactggaaactgagaaaacaacatggaattatagaataaaattgtacctgaattctagtcccaattctgccatcagcttggatgacctggatcatgtctctgtacctcagtttgttgttgttgttgttgttgttgttttgagacagagtcttgctctgttgccaggctggaatgcagtggcgtgatctcggctcactgcaacctccacctccctggttcaagcaattctcctgcgtcagcctcccgagtagctgggattgcaggcgcatgccaccatgcccagctaatttttttgtatttttagtagagatgggttttcaccatgttggccaggatggtcttgatctcctgacctcgtgatctgcccgcctctgcctcccaaagtgctgggattacaggcatgagccaccgcgcccggctttgtagctcagtttttaatgacagggtttggctttgattctgatgtctgcacaacgctcccagggctgtaagaactgcagaacacactgagaagacaccgtcccagccatggaaagcccttctatgcagtcatttattttcacatgaacacctcccagagagctatgcaatgacttgatagatatgtgtaacttttcccctattcagatatattgttaggaaaatctcattaacctttcatgtattttgatgactatctcaagatggtagttcttctgtttagctaaactagtaagagtagaatcagttaatagaaaaaggaaacttatggcataaagccatatggtaataaggacaatgagttttctgatttgaaaataggtctttgatacctcaacaataatatacctggattcaattctttacagtataaaaaaaaccttgcacatttgttaggttcgagccacatgcacctgactactgctattattatcctctttattttagagatgaggaaaataaagtccagagaggttaaacattttgccctaagaccccacagcaagtgggtagaagacctgggactataatgcaggttttctggcctctagttcagagcattcgtagcatgctagcccctcagtagcatagtactttaggaagctagtctttcccacttgctggtagtaagccagggagacataatacactaagaaagcttcggtctgagaaaactttccatgattgttttttctcaatttttagaacagtaggaattcttcacctcatctgctatcccaacatattcacaattggaaaatttttgtgctgttctgttcttttcaaattacaaaagtccttgactaggactgctggcttttacatgcacaggactgcacaacactggtgtttataaagctcattcgttcaatgataaaattggccatagcaaatcaaaaataaatgaagacctctgcgtagctgattggactacagaaaataagccattcatatccaggaagaaaaaattaaaaggattgctgaaaaggaaagagccctaaagcaaactatctacagttttggttagttttcttttcttttcttttctttttttttttttttttttgaggtggggtcttgctttgttgcccaggtgggagtgtcttcttatattggtcaggctggccttgaactcggggctcaagccgtcctcccacctcagcctcccaaagagctggtattacaggtgtgagccaccagccatggttagttttcatcaactgctttctcaccttcttttcatcctctaattcatacctgcaatccttattagaaatcctgtcaacttaatagtaccagaaagtcaggcaaaagactgataaaaaaaaagcctcggtggtcaagaacttaaaattacactactggtgtgcaacgtgctcttatctgtgttactggaggacaccctcaagatacctcactccagttgactccttggctctaaatctttgagttaaaaaataaggaggttctttatggaataaacaggtattaagctatttaaaggagagggctgcgaaatgcttgattatgggcttttcaagttcagaggccaagcgtttgtcattttcttccagtaactaggactgtgtcttgcccctaatagttactcagactatatttgcttaattgaattaaacacagttgcctatgccctttgaaattctggactttcaacagagggcctctagcccaatatttgcttaccaaactggacatcattgatgatctggattcaggcagggtctggaaaaagagagactgggccaaattaaaataatccattcactgatgacacaaaactaaactacaattgtttggcaccctctcttctccttatcttgcaaaatcaaattaagcactagtggaaagaaacagttcagagaggaatatgggaaaggaaaaaaaaaaaccaaaatgtgatttccaacgagactagagatttgttctttatctacatggtcatgttactcatttgatagcatctatctcaggggtattatgttatctcttggccaggactcatgaaagttaagatttgcattgataggaaaagttttgcagaaatatggactcttgagagggtgggaggtatataaaagtggctatggctgtgcagcagagcaatttgcatttcttatacaccctgcttgagactgatgtcattagtgttggttaggccaaggctgggggaggctactcagaatagtgggtgaccaattacccagaacctttggaaaaggaaatgacttgattgaagaggccattctttaaatgtatcttactgctcaatttcaccattgcctattgtagaatgcgccctgcccgctcagcatttgcctctaggcagaccaggactccttcccctccccaactaatcttccttctcctgtatcttattccctagggccacttgcacctttcaaaatggataaattaaattcccctgctccccttctaccaactttaacatcatatccttggtgtatgatgccctacttttcattgttttgcctaaataagagtatgcttgggaattttaggcttagggctgggaaaagatgggatatggaatcgtcagctatagattgccggacaagaaattttaggagcagtagacctttcaaccgccctcaataggatggaactgactgtccccacaacctatttccctttcagtggcttgctccagccaaggccccttatttaagagatctttgtgcgctctgaaaaccatgcatatgccagaactaggtgctctgtttcatgaaggcagtttgataactgaatggactttggaagtgcccagtgtttgactattaccctggtgcgatgatcacactgggcgtatcattgtcacatgatcccatgtttgttgatgaaaataaacagtggttttcaaaaaccattttcagtgccatggtttgtcataaaacaataaatagaaaagcgcttgatgtacctgccaacttttcacccctatctaagagatggcgaagctccggctgcactctgtctgcaaataaggaataaaactttttatttgtgctatattggactttgggttccaaagcatcacattgtttatggtaggtacatgtggagtcactgtatttataattataagagcaaactggtgccattggaaaaaatggtctttctaaatagtgtgtgaaatatgaaactagtgaagaataaaatcaatatggaaatgtaaacttctatgaaaacatttccttacccatttaagtttgtgcattctgaaatttacaatggccatcaaacccagtgactcaaagctattggaaagatatctgtccttttaaatcctacacttacagctaaacaacgtatgggttcttttccctttatctctggaaaagcccgactgagctggaatttgctccccaaaggaaagacatcaggcagaatcctcagagaaaggggcttagggaccccagtagaaataaaatcaggatagtagtgccaattcatttctggggctgctggagaagttaggcttctgggatcattcatccatgtatcaatattaataaaataaattcttctattgccaggactgtcaggaatagctaaagatgtaaaagatctaaaccagtgtgttctttcagagaataagttaaaaataatattttatagagttaaaaagaaaagcacttggattttttttttccaatggctggactcagttggccaatacccttgtttgcctgctgagtaactctttggctggcaattgatttttttaagagctgtggttatgtgctagttcattagcatgtgaataattcttcatattaagttttcatttgtttgtcgtaaatctctaaaccctgcaggaaagcagaatatctttgacagctttcaaacttcacttctatcacacacagcactccaccagcacctctaggaaacagtggttcaaaaggccctgccccaagaccccagcatgttaagagcgttagtttaaaatctccagttcatcctagaacaatcattttaaaaggaaaaaaagaagtggggaagtcctatagaaagcaatggaaagggaaaagttctcaacccagaatcggggcttaggttctagttcctggtttgctataaatggcactttgactttggaatgtctctggcttccgtttatccattagtcagagaatgatgggacagattacttctgaagaccccttatgtcctataaatctcatagttctcaacaagagggaaacgggaacaacaggggcagaaaccaacgagaggctgaggaaaccaaaccaatgagttttggattgtagctaaccgaggagaaccaggtgtgtcaaaggtgatgaaagtcagatgtgtaaaaagcaagaaggaaacaaaatgaagaacatgagccctaagaattcagtgtctttccctggtaaaactaagaacatcaggaaagccacactcgatgaggcacacatttttccaagccagttttcactctgacagggttacctcaagtgattgtttgagagagggtagaggggttgactacactcattcaatctgccaaattagaaaagtcacccagaataccctgtgctttttgagtgattttcatgtttatctcccgtagcttgctattttgttattcaaaaggagtgtaaacttagggcattcatgtataatacctttcataactcatgttaaaatgctgatgttattggatttctcaggaacactactgttctatttctccattcaaaaaggtaaaaaaaaaattaattactctattttcatcattaatcccatttcccccattgtctttgtattctacataggaagcatgccatagatctataattgaatttactcatctatataaaacagtacttttaatcccatcctgaaaatcaaaatatatttttgaaaatcaaaatatgtcaaaattgaaaatcaaaatgtcaaaatattgaaaattgaaatatatcaaaattaattatatttgatgtatccctcaaaaaattgatttctccttacagaaatcattttgctttcctggaaaaacactgggttcaagtgcagctttcttcattccgttctggtctgtccagtatatgaaaagcacaagcacacaatgaccagtgacagattcaccatgaagctaatgaagcttcatggggcccttcccttgtgcagaagtccttccagtgcttggggaagggccgaagcaattttattctcataatttgtaatattttccttagagagactccactactgtgtatattttatgccccacaaaacctgaattcaccccatcatgtcccatttgtaattaagctttctttcctgttaaggagggacgcttacccagccctttgatgtacggtctgaagataaatacactgttagcccccaactagaagtgtaaaatcattaagacaaaatttgagaatgatacggctcctataatggcaatctttggatgatactgtccaagctgatggaaagtgtaaggactccactttgctttgtaaaaaatacaaaaaaacagccatggaagtgcagtacattttgtatggaacattgtaccacattgtaccaaatgtcatgttaaattaatgattcaagataaaatgcagaccaaatttgaccagggttttaagaggttctctctccataaagcaggctggccacgatcttctcactaggtttgagggtaaggaggtcccctgtgaaatatgaaagtgaactctctgctatctaagaattggtgaattggttgcaaagaaaggcagaccaggcccacccagggatcactcttgcagtttgacagatctacctggaggctgaaagaatctatgcagccttcggaaatgcagtgaaaacagtataatcagatatgactagggaaaaaataaaacaactggtgttcatttgcatgtcaacacccagaattctctgctagttcacctcttcttcagaatgcagaaaggattgaaaaagctggaatggggccgggcatggtggctcatgcctgtaatcccatcactttgtgaggcagaggtgggtggatcacctgaggccaggagttcaagaccagcctggccaacatggtgaaaccccgtctatactaaaaaataaaaaaatttaaaaaaaattgccgggcgtggtggtgggtgcctgtaatcccagctactctggaggctgaggagaatcacttgaacccaggaggtggaggttgcagtgagcctagattgcgccattgcactccagcctgggcaacaggagcaaaactccatctcaaaaaaaaaaaaaaaaaaaaatgaaatggtttggcatgatggtggggtgctgattcctctctctgtccttgagtatttactgccaggaaatcctgaccaacatcaattgccaaggggttaaagtcacattgttgttaaattgggagagaaaattagcaggattttgtgccctatgttcaactattacagagtttcaaaaacaggaacctggagctttatatgaggggacaggggaagtaaaggggaagagtgacaagggtgatttatcagggcatagttccagataaatcacttacatggaggtgaaagaatttcatgcatatgttctgtgccaagaagccaaatggttgagcagaagctctgaaagttgaagtgggcagttctgggtacagtctttccacatgtgaaaaggtgatgattttatattcatgttatttgtactcctgcatgtgcagttggtcttttcaggtgtccagatcatcattttctcatgacatgaaagaaagccaataaaggctagttgtggtggctcacacctgtaatcctagcacgcacttagggaggccaaagcaggacgatcacttgagcccaggagttcaagaccagcccaggcaacatacatagcaagacctcatctcaaaaaatgaaataatttttttttagaaaaagaaagtaaatatttcattaatataaattataatacactgtaaaatgcctggaggacaagaaacacgttttctctaggttctgtgaaagcatcattatccattcacatttttctcataattagaacctgacgttctggaaaaatacagtaaattttcatcgatgttacttgctctgccccccttgtattcctcccattaataatattaatcctgaaaagaaaaaaagaaaaaggaaagaaaccacccaagcaaaatgtttaagaaatacggtaaggacagtttggtcccaatttccttaaaaattagagccaccaagtaaacctgtttgggggtcctcacatctgtcctcttttggagtttgctaagtagtacagttgaagtgaattttttggtaacaaaagtaaaaacttccagaataactccagtaaagggtgttgatgtgacgtacaagtttggaaatatatttaatatctgagactcctcaatgttggtgttatttcctccagtttagaacaaacttaatcttttgatgaaaatcatagagttccatagatatgaatagaatctccaaccagtgcatcttgaagccggctgccacggccactcatgcaccttctctcctttcaggagagaattgtcagcatctctgctcaaaacaatctttacttttagtccatcagagacttcatgtttgtcgtgcatgcacactcacacctctccacacatatgcccactccccacacacatcctgcttctgagaaatgcaactagaatttcctccggagaagagatggaaacccctgattgagaaatttaaggcctaggaaaggtaaatgacttttcttaagtcacatggctcaccacagaaccaaagctggaacacacataccctcagctcttcttccagtgctttcaggtatacaagtatttgaacaggattcaaggtttaactccttatgtgtcattcagtgtatccagtgtaagtaaaatgttaccccttagtcagaacagccttgagaatttctcaatgactacaaaccttgcttagttctatacaagggaagtaaaagagagagaatgtcatgaccaaatgacttaacttttgaaggcagcctattgcaaacttgaataattggggcatgtattttattgattgtttgacctataaggacagatattttaaaatataaattcaaaattgcttttttgcagcattcacctgtaggccttctatatctgctctttgtgaaatagatggcttccagagcattaaaaaaagaaatagacattttcttggttcaagagctgtaatctgctttccgagtgatttttcatagttaagcatattttatgtgcacatagtttcatttgagatctgagaggatttcatctaaaacggaaaagttattacctgtgaaggagaacaaaggaaaaggaaaaagaaattttaagaaaaaaaaatttttttaaacctgtagttactttatgttcaagtgggtattttcaacgctgagttgctgaaatggttttttattgaaagaaggttaaaagtgtatttcattgaaagccaagataaacagtagattttgtatcattttaaaaatcaacaatcggccgggtgtggtggctcatgcctgtaatcccagccctttgggaggccaaggcaggcagatcacttgaggccaggagttcaagaccagcctggccaacatggtgaaaccccatctctactaaaaatacaaaaatcagctgggtgtggcagtgcatgccagtaatcccagctacccaggaggctgaggcacaagaattgcttgaacctgggaggtggaggttgcagtgagccctgattgtgccactgtaattcagtctgggcgcagagtgagactctgtctcaaaaacaaacaaacaaataatataaaaatcaacaatgaagactccccaaacaaaagaaatcaggattcttagccagtcataggtaaagtgttacagtgtaaattgaagggaaagaagaccaaaattggtgaaatatgtttggtcccagaagataattaagatgaataaaagaacttgagagtattttctcattattaagcatcttcagctttaaagattttagttagcaaagcaagtttacataaacagttttctgaacctgggatggcattcactgtgagttagaaatctccaagtcatccacgttttccctgttttatttgcagccattcgttatctatgacatgaattccttaatgatgggagaagataaaatcaagttcaaacacatcacccccctgcaggagcagagcaaagaggtggccatccgcatctttcagggctgccagtttcgctccgtggaggctgtgcaggagatcacagagtatgccaaaagcattcctggttttgtaaatcttgacttgaacgaccaagtaactctcctcaaatatggagtccacgagatcatttacacaatgctggcctccttgatgaataaagatggggttctcatatccgagggccaaggcttcatgacaagggagtttctaaagagcctgcgaaagccttttggtgactttatggagcccaagtttgagtttgctgtgaagttcaatgcactggaattagatgacagcgacttggcaatatttattgctgtcattattctcagtggaggtaagatttgtcttttgatcttctatgaaagagggtgggatgatggtggggtggccaaaagaattttggatttccttagtgttagtctgcattgtcactttaagtgccagtggcatgatgccatgaatcatcactacacgtgcaaaacactgtaccaagaaagagtgtcataggtttgcggtgtgaaggttataagtaacccaggatcttctctttcatccctcaacaatatattttttccagtcaaatgccctcttctcctttttctttttcttttcttttctttgtctctttcttttccttccagaaaggaagattagaggccagtctaatctttggttcctgtaagtaatggcatgtataactttgcttaagacaatgctcacttgatgtagagaagggaccactaagtatttctggtcaaatcatgctcctgccccaccatcagtaagatactactttgaattgcttttgtgatatcaggaattaaggaatacctactgacctccacccactctcttgtgtggattcctctgatggcttcccttaaagtacctttgtgaggtagttggttgtgattaagaatgcaatgtgaaccgaacacacaacatagaaataaatttagttatttagcaatttgttgtatttttggccctgcaagtagtacatgatctgactaaccaattccaaaagccagattttcttctgagtgtgacttttttcttttttttttcttttttttttttcctttttttttttttttttttttttgtgagacagggcctcactctgtcacccagactgaagtgcagttgcacagtcatagctcactgcagcttctaactgcagttagtaagctatgatcatgctacttcataaaagtaatacgtggccattttacagttgggctcaagtgattctcccacctcagcctcccaagtagacaggacaacagctgcacaccaacatgccctgctaattttaaaaatttttttgtagagatgaggtctcattatgttgcccaggctgatctcagattcctgacctcaagcaatcttctcaccttggtctcccaaagcgctgggattataggcataagccaccacgcacaatctaaacattactttcattagcctctcatgagtagaagaaagttttactttcatctctctgtataaaaattgtttttaagtggcaagttttcctattgaagtggactttaggtgagctttttgtatgtactctacagtgtatcctctgtgaaaaacccgtcgggggatagtggtaaactgtatataactgcacaatgtattataaagagcacgatccctttgtcatcttttgttgtccagttgaaaggagaatgtttctgaaatcaggtgcatagtgcagtagtcataagaatagcaaacatttatttaatacttgctgtgtgccaggcagtgttctaagcacttcatgcatatttattcaatcctcacaacaattcagggaagtaaggaccattttacaaatgaggaaaccaaagcactgagaggttttctcatttgcgcaaggttacgtggctagcaaaagatggagacaggattgtgagccaggcatgctggctcagactctacactctctaccatcacatcatgcggaataccggcctttaaatgcctagggtgcaaatagatcacagtatggcatagtttacctttggagctgtgaagtccagggtcaagtcgtgattcactttaaaataactacttgatattgtgggtttttgttgttgttgttgtttgttttttgtttttttgtttttgaggcgaagtctcactcttgttgcccaggctggagtgcaatggcacaatctcggctcactgcaatctccacctcccgggttcaagggattctcctgtctcagcctcccgagtagctgggattacaggcacatgccaccacactcggctaatttttgtatttttagtagagacggggtttcatcatattggtcaggctggtctcgaactcctgacctcaggtgatccgcctgcctcggcctcccaaagtgctgggattataagcatgagccaccatgcccggccgacgttatgtttaatagaacaaaaatatactacctggcatggtttaatatcttgaccaaatttacttcctaaattaatccctggctgtctggtatctttgattaattcagcaaaaaaggatgagattccagtatataagaggtttgccagaagaaaaatattaaattttgaaaaaccagattagaaaaacagttgatattatttatctagtattttattttacttcattttattttattttattttttgagatggagtctcgttctgtcttgcagtggtgcgatctcggctcactacaaccgggttttccgcctcccgggttcaagtgactctcctgcctcagcctccctagtagctgggattacaggaatgtaccactacacccagctaatttttgcatttttactagagacagggtttcacaatgttggccagtctggtctcaaactcctgacctcatgatccacctgcctcagcctcacaaagtgctgggattacaggcatgagccactgcacccagactatttatctactattttaaggcacattttatttttaataaaatttgaaaatatattaatatttaatttatttcaaatatttttcctaagcatactatatatcccatgtctattcttttcacttagtcaatttcccatgtcattacatactctttgttaatagtttttgttaactttttaaataaaagtattacatggtcattttataattgagagtacagaaaggtataagtgaaaagtaaagggctttgccctcaggataaaatagaattaacaaagtcctatttttcctatcaagaagtttacatgcacactcatgtagatagatacatacatacacatatgtgtacgttcatagcagtttgtattcctacccacatatacgaagggaagcatttgaaatgagccattcaaaggtacttagtttctactaggcaaggtctagacaagaaacagtcatgagaattctgggctttatgaagtgagatctgaatctcaggcatctatcgaggatgagatccacctccccgattgtgcttccttagagtaagacaaaatttctcaattagtttttcctcctattccagattttccattcagctaagcaggaggctttcatccactaaacaaatttctgatcctacccagtcttaacaagagtgattgttttctcctctgcaatttattcgaaagtctatcagttactttggtggtttcagaaagaagtgcttttgttggggatccagttggcctcattctgagctggctgtggattcacagaagaacttcacttcagcaaaggctcttagggccccagactaaaagaaagatgagcaagatgtgcgtcatctaagagtgggcgggggtaaggaattggggattaatgggggtgtccctagaggacccaaagaggagatttttagatgaaagtaactgatttgacccaactcagtatttgctggggaaactggagttgctacctaagattgctgccattgaacttcagccttaaaaactgctgataccatttgattggtacttagatttgcctgggcttagcgtctctgctgttcactcagctctcaaaccaagctgctgagaaagatgacctagttcttctcgagtctttctcctctctctctttctcccctgagcttgggggcaagaattagactaaatgaaaggaacagcaacctattctagaaccaaagttcaggacttggtacctttttaagggcatttcatgttcattctctcattccatcctgacagcgctcctgggcttttaattctcatttcacagaaagaaaagtgagggtcgtaaacttaagtgatttgtctgagatctgacaaactagtgccaccgtggaactaacactgaaacctgggtgtcctaactgtcccctctggccctggccagtggactgtggtcagcacactcactcttgtgttggtggctgcaacctgttctctattcactatatccctaaggtaggcccatacctagaagccaggaacagcgcttccttggtcatcatggtaaacaataacttcccttgcactccctagtcttactgacaggctgggcggtgtcaagagtaataaaactgcctccagcaaagccatgtttgcaactggcgccgcagcatcatgccagccaccctagcaaactcccaaaacctacccagcagccaaagccaagcgtaaagctcagtgaagctgacaagccccaggacactctggtggatgttttgcccccttgagtgtttgctgttttgtgaagaaaaagtgtaggagagttccagctggaactctgcagcaggcaaaagctctttttgttaattcaaaacagtttggaatccatttcagttcttcctaaacctccaagatacgggggaggaaattcactggattttacaatatatttttcaaggcaaattgccatcgccgtcctaatgacagagaagctgccgatatcactacaacggctgcagatggcaagtcatccagcctcctcctgtgccctcctgagtctggcttggtgacgcaaaccacctcaagggcagctccttctttttccagcagtcccagcactgttccttctctgtgaagccactttggatggctattcttggcatgatcatagacttttctgctgttgagtgggcaaggagaatagggtagaagcaggggaattgttctcattgctatgcatttatagatcaaagaggagcagatattttatgttaattggataacacctagttctatcaggtcagtaacctggggtccctggggctcccccatgggtcataccagatagatagattttttaaaaatttgttggaattaaagtagaatcaaagcctagtgctagcccagaataagttattcaataaatgcttgttgagtgaataatcatccgaaatgattataatactgcctaccattcgttgaaagcttcagtatgtgggagaatctgtcctgggcactttatatacacccataatctgtttggatttcttggtaggaagactacatggctgcatacatggtctttcattacctccattttatagatggagaaaatggaaatttaaagaggttaagcagtttgccgaaggtcacagagctactaatcggtgaggtcaaggttcagacccaggtctctcagactttaaaactggtgcacttaaccattagactctactttttgcgtattgagatgtggaagcatctcaattaattgcttcagtcttggagttctttggcggttatcaaaaactgcctatttccatattgcctccagatattgtaattaagaatttccaaggccaggcacagtggcttatatctgtaatcccaacattttgggaaaccaaagttggaagatcccttgagcccagaagtttgagaccagcctgggcaacatagggaggcttcgtctctacaaaaaatacaaaaattagccaggtgtggtggcgcatgcatgtgtagtccaagctactctggaggctgaggcaggaggattgcttaagcccaggaatttgaggctccagtgagctgtgattgtgccactgcactccagcctgggcaacagagtgagatcctgtctcaaaaaaaaaaaagaaaagaaaaagaaaaaagaatctccagattatagttcagatattacgtattaatatccaaagccctccttaagacaccattttaatctgtctaacaaaattaacaccctaggttttgacaattgcttgaggagggagtagggcctggtgatagagctaaagactagtgttctggttctttaatttgttcagccagcaggtacctggaaataatgatactgtttgcagaactccccacaaaaatggacagtcaactttaaataactaagtaaacacatctctgcttaatcagataccatcttatactaggttctaatatagataagtggttgcagaaacatttatgagaggaatgttaaattgtcgaaataccatccagtcccttcatttcttcctgcccttcagaaacaaacagaataaccctgatgcagctgtcacggcagaacactcattccagctcacagaacaccagtgttcaatcagcactgagtttgaggagcaccgggtttgggagtattcatctctcttccctgtcccatagctgcccttcaaactcttgagactgttcccagctctaaaatggaaagggtcgtcttctctctggaacaaaagacaggatgtacttgcttgaataggccagtgctttcctggaggaaactccggcttatggagcctctgcttctgcacagcccagtgccttccaccccctcttcatctgctagcatctacattactagttaactggagaggagaccaaacccaaaatattacaaaacatagatattaaaaatactgtgaacaacaatcagcccgctttctcccacctctcctgtaccagctaaatatttacctccctcatccgtagagggtttttggacaagacaggctggtgcctacatggtgaaagttgtttttctctcttttcttgtaatattgcaaataaacaaggatatctgctttctcttgagcaggacaacagccaaagagtattattgcatagttcctgtcccctatctgggctacgattgtgtctgagagtaatagcacttatttattaactggaagaaattttacaggcacctatgttgtttctgcctagcttctgaggctcctctcttaggccactcctctcaccatgcccccacagctagttggtaaaatggctttgaataatgactcgctttgagttatctagaaatgtcccattagttcactattttcataaccccatagacttggtttgacaagggtgaggtttatttatgagttctcaactggcacccaatttttaaaaaccacagagctgggggcggggatagaatgatggggaggagatgaaacatcctagaatcatctgatatactttaaacatatacatatacaggcttttgttgtttgtaaaatatagaagcatctttatctgtgactggttgagaaataaaatcccttccccagcccaggcatggtaggttgggatcatcccagtgagcgagcaagcaattggatttgccctcagagactgactatggggtcgaatgctgagtcattcctgtccccacaccagcagtcctggaagaggctcagtcgatcagtcagtgggctgctttctggagcactttatcattttgggctctcacaatgtgtgtttaaactctgagtgaccccaggcagccttccagactggcacagttcaccaagacgttcagacagatcatctgcaagtgaggaagaatgaaaacccagcactggttcaaatcactcctagcagaggtagtgaaggcatcactcagtcctggagaaatcttcggagggctcaccagcgtcacaagtaggtagaccagaagaggcaggctggcccattgcaaagccctggaatcagagggacaggagttccaaatccccactctctctcttcctagatgtgtgcttgcggcaattatttatctctctgagccttaatttccttatcaggaccctgagcaaaccaaataacatgatgtgaagcctctggcacaatgcctgggacatgttcagcacacaataaatgctaattttcccttttgccctatatgatatgatttgaagcagcgccactcaatcctgccagtcacattgctggaaatgccaccaacagtcattcttaagatcgcttattacaatataaatacccctaggggatatcagctaatcgctttatcaactatcgctttaaggggattaggtgtggattgagaacaaaacccagaaggaaagagatcctggaggaaggggagggcttggaagtggggaggattcggacgtcctgtggcccccgaaggagacggggaatggcaggtctgctggattcccagccttcaggaattcccatgaacttcttggggacttcatgtgtttagaccatatttagagagcgtgcatgtgttttgagatcacaggtttttctgagagacattgggaaggaggacagcgggggagtggagtggagagaagtcatacctggcagcttttaacttcacttactgcccttcatgtgctgttgccatttccagaagttgagggagtaaggaagggtaggagttcttggtattcccttatctcttcctttccctccccttatcctgcccagagcatcgcagggtagagccaccagacggattcagggcatggagatggcaggttagtggtagacttggaagggatcgttcttcctatttcagcaccacccttcttcctctacctcccaccctgcatttccagccccagtcagattccttcttggacagagaaggagcagaaatgtacgtacatcactaggcttaaggggggactgcagatggctcccctggtcctgacaaaaaggtggggagcaaaccgcatggctggacgtaaattgagtgacctggaatgactagaacgacagggggcctctaaccccagggtgcacagaggtagggacccaagggctttccggggtcggacagaaatctcgggttccattttcactctgagagacccagaaatgacagagcccatgctcagtttccactggtggtgctgttgagtggaggggctttgaacatggcacacaggaaagggttgcccaccctgtcaccagatgggcttgcactgttttgtggtttgggagttgcatattggaggtgggagtggagtgttgagatgaggcaagttgagatgtaatcgctatttaatgggcagatcaaagaaaacattggctggtttgatttttattatggttatcccgctccaccatcctggcccagtcatatatattattgttatcaggcatagataggggaagcaattaaatgtgaaactgttatttaaaccggcaagtgtcagaatgttaacccacttcagagcgaaggctctaccagcaacatgtgtgttcactgcagaatgtgctggttacagatgatctttatctgtttgtcaaagcatttgcaagatctctattttatgtcatcccctttccctgaaagcagcagcagtaaacgacattgctcctcaaatcatccatggctcagacctctgattaatttaagctggccctgctagcgttcttataaatccccagcaagatgcaggcccaggagtggaaaggggaaaacatccggaaagcagcggggggcagggagggggaaggctgaagggaaaagaaaaaggctgaagggagcaataattgaggaagaaagaataggaaaaatgtagaaaggacccaagaaaatcagagaaatgagaggaaaagaaaggtaagaagaaaatgaggcaagtttacagagcagtaatgaaaatagtaatagctaatttactgtacaacagacactgtgctaagcactttccgtatgtccctcagtcctctgaccaacactatgagttaaattaccgctacagctccaattgttaaagtgaggaaactgaagtatagaaaggttaaggaacttgcccaaggttacctagcttgcaaagttgtaattccaactgcgtctcactcagctggcagtgtgcacccttggccacacattagaatcacccaagagctattaaaaatcctgaaggtcataccccaggcaagtgaatcagaatctctagggatgggtcccaggcattcgtttgcttttttagtctccccagataattttaatatgtagccaaaattgataatccctgcactagaccaagctccgattcaaatttaaatattaagaggacacatgtataactttgctgaataattttttcctatcggtaggatggtgggaaggaattgctataggccacaccatgatactttgctgaattggatcagaaaagtaccctcaaattcccagcatcatttcttcaaggaagtagtgaattggggcaccgtgggttttttgttttgttattgttcttaaaccaccttgcctatgtgcactcaactacaggaacgagaacttgcctgaaaccccaaacgtgtctgcatcaggcattatttttcttgagctcctgaatttctgctctaaccaagaacaactcaaaaaccttcaatttcataactgttgatatgccacccactcctacttacactcctgaccccaaccccatggaaactgcctttattcgaacaaacacaagaattataatatgttctaaagttcctctacctatttcattctcaccatacgcttatgaaagaaatgtcattgtcttgaaaactaagcctaaacccagaaagattagatgatttgtccacaggcacacagaaactaagtggaagagaaacaggactcaagtcttcagtttcccaatccactgcctcctagaacatgcctgtgaactgagggagcagtgcaataaaggaaacttgagaggaagcgcaaaaggaacttaaattgcaaagtactgggttccctaagtagccctgcctcccctccagttttcagcccacacctgaactaaggtctttcattgtctgtggatcaatttacagctgccctgcaatcacatttgttttgtttgtttgtttgttttggttttgaacgccctagggacagtcggtttcagattagtctctatcagagagccaatagggaaagatgcagaaagccaggagagcagctcctagaatagagacaaaaccacctgcattttttctgcctcttcttcaggagactccactgtggtcatctggttccctaattgagacacctcctgagaaaatctgtgctagggaaacacccagcccaggtgggcagatctcaagaggaccagaacgtttgaatctgcttcagataaaccctccacttaacagtaccagatctggacgagatggaagctttgtagatttgcccataatccacagtgctctgtaatcaattccaggaccgtgtggatggagaccggaaaggtttctttcccaattcttcacagcctggggagtagggaactagtaattgactccagcctcctcgagtgctaagtcctggagtctgagtcacacacacttcccaaaagggccttctaagcagcctaccccagcagagaggacccttggccctggccctactccagactcaactgtaacctcagcaaggtgcagggagaggatctcaggtgggcctcctggcaacagtgccttttcaggcactaggctgttgggaatggagagagaagagaaaggccctggcactgtctgggtatttggatggatttctgtggcacaactgtggcacctggcttagctcagtaaaggactgagtgtgcgtggagcagaaaggggaaagagactagtggggagctggtgaccagttggagggtggagggtagggaacaaccctggcagatccattttgcccttgactagagcttaaagaccaaaggaagcgttcttgtttttaagtaagtcaggtgttctaagtttaatgttaatatgctttttcaattagatgtttgagtatatttccccagttgaattatgtagagggaattacaaatgagaatacatcttacaatttttgaattagaatctttgagattatctatttagtccggtctgttttgtttagacaagaaaattgagcccattgatcttaatcagtttgcccaaggtcacagagctggtgagtgaaagctttagatgtagaatatgcaacttttctctgctgccctccttccctaaaccatcttgccttaacggaggctcagtcagggggacaatgggactgatctgtaaatgatctaacttgtcattgcagaaaatatacttactccgtggccacaaaatttcagcccttcagccaagcttcatccatcacatcataaagaataacttgccaaagaggggtttgaaaatccaaaccagatccctctccactcctagagaggccagttccatgacactgcaccggagccaagtgtttccagcaagccctgatcagttgcatgttagtccttgtttgtatgataaacgggacctagtagattaacatcatctcctcagcccaagggctgaccccagtggtgctgctcaagaggaaggaggaggctgggagcggtggctcccgcttgtcatcccagcactttgaggggctgaggagggcaaatctcttgagcccagcattcaagagcagcctggaaaatgtagagattctgtctctaccaaaaaaaaaaaaaaaaaaaaagaagcaggtggaggaaggaggagctgcagaaaggctccgggagccagtgtctagtaagcagaggcctagcccaggctgagtggtcccagcccaggagggcctctctcggcacctgtctttagatgcacgtctgcctctggcctttgagatgcacacattcatcaagcaggaggatctgtagtcattaaaccaaggtgccagtctggggcccagccttcaatgaagcatcagtggctttttcattcccatagagcaactgcgaggaagaccccatgctcccaggggcccaattctccaggccaggaccagatcatttgttccttctcagaatctgagatcttttgctgatggttccaaaattgaatgctgaaatctaaaaagaaaattatacttactctggtcaatgggatatgttggagacctgagagtgaaaaaatcaaactgaagaccagtttccttctttaatggaagaaaagtaagaaagttaacttagaagaatatttagagttctgaaaatcccactctgagaccactctgccatctcacattgttctcttgagccttatctcaatggataaaggtcactagagtttattagacacaggaaaacatcgtttacagacttcttcattgtgtagggattctgccttcaggcctgttcaccagccaggagaattgtgctttttgatccagggctcttggccagaacagccttctcgctcattaactcagtcaaccaaatgcttcctgtgtttccactggtggttcagaacgtagtctctgccctctgatacctcacggtctaacgggggagaaacaagaaagtcagaacttacaatacaagataataaggaataagagcagagcctttggaaccagacagacttagatccaaatgtcagctctgcatttactagcaagtggtctatcttggtaagatgcaactcttttctctaagtcttaatttctccctctgtaaagtatgacctcatggggttattgtgaagattaaatggcatatcgtatataaggcccttggcacgatctttggaaaataataaccattcagtgaatgtaatctactagtatagtagcgattgaggtgtttatagggtgctatgagggcccagagaaaggagatgagatgaacaggagagaggaagggatactgttgaggaaggatttcaggatggaatcccaccacaggctgtattttgaagaaatggttgaagtcaataagaagagtgaagggaaggtgagaatgtttcaggcaggaagaataaaatctgaataagtgcagagtcctgacagaacatagggtgtttgaggaacttggtatggaaatagattaatatggcttaacatggagcaaaatgaaacagaactgagactagaggatgaccaggaccaggtcatgaaggacattaaaggtgggtaaaactcataccatgaaggagagaagagttacagtttttaaaagaaaataaatagccttcaggagctcaaatttgaaatcaatacgagatagatgatcaagtgaatgttctgtcttcttgatgagcctgactgagaaaaccttataatctaacccaaggcaacaaactgagaaattagaaaataaaacttagagattagaaaacaaaaactgaaacccaaactttttacttggaaatttaaaaacatgcttctatataactcttaggttaaaaatgaaatcaaaattgtaagacaagctgtttagaaaagaactatgagagtaccgtttatcaaagcccatgggatgaaaccaaagtggcactaagaagaaaatgtggaggcttcaatgcatttattagaatacaaagaataccaaatcaaatgaattaagcattcaactcaagaaaactagaaaaagagaagaaagtaaacctaaagaaagttttaaaaaggaattcaataaattaaaaacaaaacacacaatttttaaaaacagacttgattaataaaaccaaaagctatgtcttttttaaaaaagcaaaaaatagataaacctttgacaaatcagatttttttaatgagagaatgcacaaataaagagctctaagagctgggcatggtgactcatgcctatattcccagcactttgggaggctgaggcaggaggattggttgaggccaggagtttaagaccagcctgggctacgtagcaagaccccacctctacaaaaaatttcgaaattagttgggtgtggcggctcatgcctatagtcccagctacttgggaggctaaagcaggaggatcacctgaacccaggagttggaggctgcagtgagccatgatcatgccactgcactgggcaacagattaagactctgtcacaaaaaaaaaagcgttaagttaaggagcgtgaataaaaataatacatttcatattctaagacaatatcatctacaactttattccaatataaattactaaaactttaccatataagtagtagaaagcctgaatagataaaagctatggaagaaaaattaaagatagtgatagatttatcaccaagctcagatggttctgcaaacaaattctaagaaaccgtcagggaacagatcattactgcgttgacacagaaggcaaacctctcaacttggtgtataaggctagttaacattgttactaaaacaggcaaagaatggcccccaaaataactctaaaccagtatcacctacaaatacaaaaactctatataaaatattagcaagtgagtacaagagtataaggaactctattaatgtaattcactgtgctaggttaagataaaaccataactcttcagatatcatagctctttagatagaaaaatgtaaaagtatttgataaaaattcaacaacattcctgactaaaacaaattaaaattgtaaaacccctggaaagccaggagtaaaacatgttctccataatctatagcaaacatcatagttgctgataaaccattagaagcatttccttcaaagttaggaataaaacaagaattgctactattgctactattatttaatcccatattggaggttttagccaacacactatggcaagaagaggaaatgagaaaggttaatgctgcaaaagaagaaataaataaagctaccattgctgatataattatctatccaaaaaaagtagaaatccatgattaaaagctatttgaactgataaaagttcagaaaattggaattgtttcaatatactaaaatcaattagttttctgcacatcagtggggatatattagatgtaatgaaaatgaagggtccattcacaatagaagctataaagtatttgagaataaatctaacaagatctacataaagaaaaaagtaaactgcttaaaagtaatttaagttcaccatttgcaaattgaactaaagaaaaatctaaagaagaactagtgaaaattgcttgcaatcttaccactgaaaagaaacctctgttaaaatgtatcagtattttaaaactgtgttttgtcctttggaaatatgccatattaagcaaacatagcataagcaaattaagcaaaaagacaaacctttttttaaaagcatatttgtgaaaaaagcatatttgaagctatgataagaaactgagtagaagctataaaacgtagattcatcaggaaggagcagaagttgaaaaggagatttctggctgggcacagtggctcatgcctgtaatcccagcactttgggaggccaaggcgggtggatcacttgaggtcaggagtttgagacaagcctggccaacatggtgaaaccctatctctactaaaaatacaaaaattagaaaggcgtggtggtgagcacctatcatcccagctactcaggaggctgaggcaggagaatagcttgatcccgggaggcataggttgtagtgagccgacgtcatgccactgcactccagcctggatgacagagcaagactccatctcaaaaaaaaaaaaaaagaaaagaaaagaaaaggagatttctgagtagaaacacgttagcagaggaaacttcatttggggaacaggattgttttgatgccatgctccctcagctgaccacacagattacatcctggccagaaaaaggccctgcaaagagctctgatcattttggttctgattccatccttagttcttacccattatctgcttacccttcctccccacctatttaagatacaaagcaaaacaaaccaaaaatacagatgagttgcttggtagagctgcctaggcctccaaggcggggcccagaggattttttgactgaaccccctgttgtgttttccatatgtgcttccccagaccgcccaggtttgctgaatgtgaagcccattgaagacattcaagacaacctgctacaagccctggagctccagctgaagctgaaccaccctgagtcctcacagctgtttgccaagctgctccagaaaatgacagacctcagacagattgtcacggaacacgtgcagctactgcaggtgatcaagaagacggagacagacatgagtcttcacccgctcctgcaggagatctacaaggacttgtactagcagagagtcctgagccactgccaacatttcccttcttccagttgcactattctgagggaaaatctgacacctaagaaatttactgtgaaaaagcattttaaaaagaaaaggttttagaatatgatctattttatgcatattgtttataaagacacatttacaatttacttttaatattaaaaattaccatattatgaaattgctgatagtatttgaagactgagtcttgtgtgtttcccaccctagcccccaggctttcttttttaccccttttccttctcccctccctccctccatccctctcactcttcctccctcccttccctcctttccttcttcctttatttttcttttctttcttagacattttaaaatatgtgagtggaactgctgatacactttcattctcagtaaattaattttttactcaatttacaacttttcggaactctgcatctgctttaacaatcagaactaagaagggaaggggaacttcagaatcagaaactgctcagagcatgtgttttgtagcctggatgtgctgatatgcagcatatccctgggattacccagaattcagtcttcttccacaatcctaaccgagattttcacgcaccaccagcagcctactcgtatactacctactaatcaatgccactgcgcacccacagagccagtggccagcaactgagcactgctagaaactctggggaacacagaacttttttaagatttggtatctgcgccaggcatggtgtctcaagcctttaatccacgcacgttaggaggccaaggtggatggatcgattgagctggtctcttgttcgagaccctgtctccacaacagttttaaatattagccatgtgtggtggcacacacctgtagtcccagctactcgcaggctgaggcgggaggattgcttgagcctgggagttgaggctgcagtgagctgtgatgatgccactgtattccagcctgggccacagagtgagaccctgtctctaaaaaaagataaaaaagatttgacacctgccaaaaagaatttaccgattataaactgaggagaaaagattaatcttttttcatacagattcaaatacgcagatgaaatcacatgccaggtgaatggtaagagtttgtaggaagtaagatgagtgaagattggaatcccagagactgaatctgtggatttgctgaagagggcctcagggaagtgttagactggaataggtagagaggaggagaaaagacattccagagaagcaaaataacaggaacacaatgaaagaaaaaaaaaactgagggagaagagctactttctgttttctccttctgcaaggcagttttgctgtgattattcctgtcctcctccttgggaccactctgtccagagatctcttttctgaactgagaggctaactatccgcatcattaatggaatgcttgcctcccaagcagatagattctaagttccctgaaggcgtgacaatctattcattcttggcacagtgaatagattcgttgattcaatccaccaaattcacttgcattggctactcatgaactcatcatactatgtctttgaagaatgccttacggggtgtctaagggagagaatagagtcatgggttctccatttctgtttctgactgggccaataaagccccttcctcatccctcttttccacttaccactagggacagaaattaaaaaccatggcttcaggctactaaaagcctaaaccaaaccaaatcaaaccaaacaacaacaacaaaataaggcaggttggacaagcttacgagtgtaaccaaactatctggaggtgtctgttgtgcgggacgcttatttccactgacctaaatttccctgccacttctcccttaatttatcttgccttaggatatttacactcaggagacataactgcagacttgaggttttcaagccaaaatatcaagaaagacctgttcatcttttgcttaaaaataactatatctccaaagaatcaggttatagaagtgagtactgaccccagccctaaaaatgtaggattcctaacccttcaggagagacctttctgagctcaaacctttaggatgacagatagacaaagactgaagccattgtctaagtaacaccaaaacatttggaaggaaagtgacaaattcagtcagtcatatggctctttttttttcttccttgatgccaa

SEQ ID NO: 2 - protein, 475 aa, Homo sapiens
MVDTEMPFWPTNFGISSVDLSVMEDHSHSFDIKPFTTVDFSSISTPHYEDIPFTRTDPVVADYKYDLKLQEYQSAIKVEPASPPYYSEKTQLYNKPHEEPSNSLMAIECRVCGDKASGFHYGVHACEGCKGFFRRTIRLKLIYDRCDLNCRIHKKSRNKCQYCRFQKCLAVGMSHNAIRFGRMPQAEKEKLLAEISSDIDQLNPESADLRALAKHLYDSYIKSFPLTKAKARAILTGKTTDKSPFVIYDMNSLMMGEDKIKFKHITPLQEQSKEVAIRIFQGCQFRSVEAVQEITEYAKSIPGFVNLDLNDQVTLLKYGVHEIIYTMLASLMNKDGVLISEGQGFMTREFLKSLRKPFGDFMEPKFEFAVKFNALELDDSDLAIFIAVIILSGDRPGLLNVKPIEDIQDNLLQALELQLKLNHPESSQLFAKLLQKMTDLRQIVTEHVQLLQVIKKTETDMSLHPLLQEIYKDLY

SEQ ID NO: 3 - protein, 505 aa, Homo sapiens
MGETLGDSPIDPESDSFTDTLSANISQEMTMVDTEMPFWPTNFGISSVDLSVMEDHSHSFDIKPFTTVDFSSISTPHYEDIPFTRTDPVVADYKYDLKLQEYQSAIKVEPASPPYYSEKTQLYNKPHEEPSNSLMAIECRVCGDKASGFHYGVHACEGCKGFFRRTIRLKLIYDRCDLNCRIHKKSRNKCQYCRFQKCLAVGMSHNAIRFGRMPQAEKEKLLAEISSDIDQLNPESADLRALAKHLYDSYIKSFPLTKAKARAILTGKTTDKSPFVIYDMNSLMMGEDKIKFKHITPLQEQSKEVAIRIFQGCQFRSVEAVQEITEYAKSIPGFVNLDLNDQVTLLKYGVHEIIYTMLASLMNKDGVLISEGQGFMTREFLKSLRKPFGDFMEPKFEFAVKFNALELDDSDLAIFIAVIILSGDRPGLLNVKPIEDIQDNLLQALELQLKLNHPESSQLFAKLLQKMTDLRQIVTEHVQLLQVIKKTETDMSLHPLLQEIYKDLY